European Patent Application EP 4 434 534 A1, published September 25, 2024. Title: Klotho mRNA. Applicant: ADvantage Therapeutics, Inc. The sequence listing filed with the application follows.

SEQUENCE LISTING (78 sequences)

SEQ ID NO: 1 - RNA, 1353 nt, synthetic construct
  source 1..1353: mol_type = other RNA
ctgttccagggcaccttccccgacggatttctgtgggccgtgggaagcgctgcctaccagaccgagggcggctggcaacagcacggcaagggcgccagcatctgggacaccttcacccaccatcctctggctcctcccggagacagcagaaacgccagcctgcctctgggagcccccagccccctgcagcccgccactggagacgtggccagcgactcctacaacaacgtgttccgcgacaccgaggccctgcgcgagctgggcgtgacccactaccgctttagcatcagctgggccagagtgctgcccaacggcagcgccggcgtgcccaaccgggaaggcctgagatactatcgccgcctgctggagaggctgagagagttgggcgtgcagcccgtggtgaccctgtaccactgggacctgccccagcgcctgcaggacgcctacggcggctgggccaacagggcactcgccgaccacttccgcgactacgccgagctgtgcttccgccacttcggcgggcaggtgaagtactggatcaccatcgacaacccctacgtggtggcctggcacggctacgctacaggaaggctggcccccgggatccgcggcagccccaggctgggctacctggtggcccacaacctgctgctggcacacgccaaagtgtggcacctgtataacaccagctttcgccccacccagggtggacaggtgagcattgccctgagttctcattggatcaaccccaggcgcatgaccgatcacagcatcaaggaatgccagaagagcctggacttcgtgctgggctggttcgccaagcccgtgtttatcgacggcgactaccccgagtctatgaagaacaacctcagcagcatcctgcctgacttcaccgagagcgagaagaagttcatcaagggcaccgccgacttcttcgccctgtgcttcggccccaccctgagcttccagctgctggatccccatatgaagttcagacaactcgagagtcctaacctgcgccagctgctgagctggatcgacctggaattcaaccacccacagatcttcatcgtggagaacggctggtttgtgagcggcaccactaagcgcgacgacgcaaagtatatgtattatctgaagaaattcatcatggaaaccctgaaggccatcaagctggacggcgtggacgtgatcggatacaccgcatggagcctgatggacggcttcgagtggcaccgcggttacagcatccgccggggcctgttctacgttgacttcctgagccaggacaagatgttgctgcccaagagctccgccctgttctaccagaagttgatcgagaagaacggcttc

SEQ ID NO: 2 - RNA, 1353 nt, synthetic construct
  source 1..1353: mol_type = other RNA
ttgtttcagggaacctttcctgacggtttcctgtgggctgtgggcagcgccgcctatcagaccgagggcggctggcaacagcacggaaaaggagccagcatctgggataccttcacccaccaccccctggccccccccggcgattcccgcaatgccagcctccctctgggagcccctagccccctgcaacctgccacaggagacgtggcctcagacagctataacaacgtgttccgcgacaccgaggcactgcgcgagctgggcgtgacccattaccgctttagcatcagctgggccagagtgctgcccaatggctctgccggcgtgcccaaccgggagggcctgaggtactaccgccgcctgctggagaggctgcgggagctgggcgtgcagcccgtggtaaccctgtaccactgggacctgccccagcgcctgcaggacgcttacggcggctgggccaaccgcgctctcgcagaccacttccgcgactacgccgagctgtgctttcgccactttggcggccaggtgaagtattggatcaccatcgataacccttacgtggtggcctggcacggatacgctacaggccgcctggcccccggcatccgcggcagccccagactgggctacctggtggcccacaacctgctgctggcccacgccaaggtgtggcacctgtacaacaccagcttccgccccacccagggtggacaggtctctattgccctgagctctcactggattaaccccaggaggatgaccgatcacagcatcaaggaatgccagaagagcctggacttcgttctgggctggttcgccaagcccgtgtttatcgacggcgactaccccgagagcatgaagaacaacctgtctagcatcctgcccgacttcaccgagagcgaaaaaaaattcatcaagggcaccgccgatttcttcgccctgtgtttcggcccaaccctgagcttccaactgctggatccccacatgaagttcagacaactcgagagtcccaacctgcgccagctgctgagctggatcgatctggaattcaaccacccccagatattcatagtggagaacggctggtttgtaagcggcactactaagcgcgatgatgcaaagtacatgtactatctgaagaagttcatcatggaaaccctgaaggccatcaagctggatggcgtggacgtgatcggatacaccgcatggagcctgatggacggcttcgagtggcaccgcggttactcaatccgcagggggttgttctacgtcgacttcctgagtcaggacaagatgttgctgccaaagagtagcgcccttttctaccagaagttgattgagaagaacggcttc

SEQ ID NO: 3 - RNA, 1353 nt, synthetic construct
  source 1..1353: mol_type = other RNA
ctgttccagggcaccttccccgacggatttctgtgggccgtgggaagcgctgcctaccagaccgagggcggctggcaacagcacggcaagggcgccagcatctgggacaccttcacccaccatcctctggctcctcccggagacagcagaaacgccagcctgcctctgggagcccccagccccctgcagcccgccactggagacgtggccagcgactcctacaacaacgtgttccgcgacaccgaggccctgcgcgagctgggcgtgacccactaccgctttagcatcagctgggccagagtgctgcccaacggcagcgccggcgtgcccaaccgggaaggcctgagatactatcgccgcctgctggagaggctgagagagttgggcgtgcagcccgtggtgaccctgtaccactgggacctgccccagcgcctgcaggacgcctacggcggctgggccaacagggcactcgccgaccacttccgcgactacgccgagctgtgcttccgccacttcggcgggcaggtgaagtactggatcaccatcgacaacccctacgtggtggcctggcacggctacgctacaggaaggctggcccccgggatccgcggcagccccaggctgggctacctggtggcccacaacctgctgctggcacacgccaaagtgtggcacctgtataacaccagctttcgccccacccagggtggacaggtgagcattgccctgagttctcattggatcaaccccaggcgcatgaccgatcacagcatcaaggaatgccagaagagcctggacttcgtgctgggctggttcgccaagcccgtgtttatcgacggcgactaccccgagtctatgaagaacaacctcagcagcatcctgcctgacgtcaccgagagcgagaagaagttcatcaagggcaccgccgacttcttcgccctgagcttcggccccaccctgagcttccagctgctggatccccatatgaagttcagacaactcgagagtcctaacctgcgccagctgctgagctggatcgacctggaattcaaccacccacagatcttcatcgtggagaacggctggtttgtgagcggcaccactaagcgcgacgacgcaaagtatatgtattatctgaagaaattcatcatggaaaccctgaaggccatcaagctggacggcgtggacgtgatcggatacaccgcatggagcctgatggacggcttcgagtggcaccgcggttacagcatccgccggggcctgttctacgttgacttcctgagccaggacaagatgttgctgcccaagagctccgccctgttctaccagaagttgatcgagaagaacggcttc

SEQ ID NO: 4 - RNA, 1353 nt, synthetic construct
  source 1..1353: mol_type = other RNA
ttgtttcagggaacctttcctgacggtttcctgtgggctgtgggcagcgccgcctatcagaccgagggcggctggcaacagcacggaaaaggagccagcatctgggataccttcacccaccaccccctggccccccccggcgattcccgcaatgccagcctccctctgggagcccctagccccctgcaacctgccacaggagacgtggcctcagacagctataacaacgtgttccgcgacaccgaggcactgcgcgagctgggcgtgacccattaccgctttagcatcagctgggccagagtgctgcccaatggctctgccggcgtgcccaaccgggagggcctgaggtactaccgccgcctgctggagaggctgcgggagctgggcgtgcagcccgtggtaaccctgtaccactgggacctgccccagcgcctgcaggacgcttacggcggctgggccaaccgcgctctcgcagaccacttccgcgactacgccgagctgtgctttcgccactttggcggccaggtgaagtattggatcaccatcgataacccttacgtggtggcctggcacggatacgctacaggccgcctggcccccggcatccgcggcagccccagactgggctacctggtggcccacaacctgctgctggcccacgccaaggtgtggcacctgtacaacaccagcttccgccccacccagggtggacaggtctctattgccctgagctctcactggattaaccccaggaggatgaccgatcacagcatcaaggaatgccagaagagcctggacttcgttctgggctggttcgccaagcccgtgtttatcgacggcgactaccccgagagcatgaagaacaacctgtctagcatcctgcccgacgtcaccgagagcgaaaaaaaattcatcaagggcaccgccgatttcttcgccctgagcttcggcccaaccctgagcttccaactgctggatccccacatgaagttcagacaactcgagagtcccaacctgcgccagctgctgagctggatcgatctggaattcaaccacccccagatattcatagtggagaacggctggtttgtaagcggcactactaagcgcgatgatgcaaagtacatgtactatctgaagaagttcatcatggaaaccctgaaggccatcaagctggatggcgtggacgtgatcggatacaccgcatggagcctgatggacggcttcgagtggcaccgcggttactcaatccgcagggggttgttctacgtcgacttcctgagtcaggacaagatgttgctgccaaagagtagcgcccttttctaccagaagttgattgagaagaacggcttc

SEQ ID NO: 5 - RNA, 1521 nt, synthetic construct
  source 1..1521: mol_type = other RNA
atgcccgctagcgccccaccgagaagaccgcggccgccaccgccatcgctgtcgctgctgctggtgctgctgggactgggcggaagaagactgcgtgcggagcctggcgacggggcccagacctgggccagattcagcagaccccccgcacccgaggccgccggcctgttccagggcaccttccccgacggatttctgtgggccgtgggaagcgctgcctaccagaccgagggcggctggcaacagcacggcaagggcgccagcatctgggacaccttcacccaccatcctctggctcctcccggagacagcagaaacgccagcctgcctctgggagcccccagccccctgcagcccgccactggagacgtggccagcgactcctacaacaacgtgttccgcgacaccgaggccctgcgcgagctgggcgtgacccactaccgctttagcatcagctgggccagagtgctgcccaacggcagcgccggcgtgcccaaccgggaaggcctgagatactatcgccgcctgctggagaggctgagagagttgggcgtgcagcccgtggtgaccctgtaccactgggacctgccccagcgcctgcaggacgcctacggcggctgggccaacagggcactcgccgaccacttccgcgactacgccgagctgtgcttccgccacttcggcgggcaggtgaagtactggatcaccatcgacaacccctacgtggtggcctggcacggctacgctacaggaaggctggcccccgggatccgcggcagccccaggctgggctacctggtggcccacaacctgctgctggcacacgccaaagtgtggcacctgtataacaccagctttcgccccacccagggtggacaggtgagcattgccctgagttctcattggatcaaccccaggcgcatgaccgatcacagcatcaaggaatgccagaagagcctggacttcgtgctgggctggttcgccaagcccgtgtttatcgacggcgactaccccgagtctatgaagaacaacctcagcagcatcctgcctgacttcaccgagagcgagaagaagttcatcaagggcaccgccgacttcttcgccctgtgcttcggccccaccctgagcttccagctgctggatccccatatgaagttcagacaactcgagagtcctaacctgcgccagctgctgagctggatcgacctggaattcaaccacccacagatcttcatcgtggagaacggctggtttgtgagcggcaccactaagcgcgacgacgcaaagtatatgtattatctgaagaaattcatcatggaaaccctgaaggccatcaagctggacggcgtggacgtgatcggatacaccgcatggagcctgatggacggcttcgagtggcaccgcggttacagcatccgccggggcctgttctacgttgacttcctgagccaggacaagatgttgctgcccaagagctccgccctgttctaccagaagttgatcgagaagaacggcttctga

SEQ ID NO: 6 - RNA, 1521 nt, synthetic construct
  source 1..1521: mol_type = other RNA
atgcccgctagcgccccaccgagaagaccgcggccgccaccgccatcgctgtcgctgctgctggtgctgctgggactgggcggaagaagactgcgtgcggagcctggagatggagcccaaacatgggccagattcagcagacctcccgctcctgaagccgccggcttgtttcagggaacctttcctgacggtttcctgtgggctgtgggcagcgccgcctatcagaccgagggcggctggcaacagcacggaaaaggagccagcatctgggataccttcacccaccaccccctggccccccccggcgattcccgcaatgccagcctccctctgggagcccctagccccctgcaacctgccacaggagacgtggcctcagacagctataacaacgtgttccgcgacaccgaggcactgcgcgagctgggcgtgacccattaccgctttagcatcagctgggccagagtgctgcccaatggctctgccggcgtgcccaaccgggagggcctgaggtactaccgccgcctgctggagaggctgcgggagctgggcgtgcagcccgtggtaaccctgtaccactgggacctgccccagcgcctgcaggacgcttacggcggctgggccaaccgcgctctcgcagaccacttccgcgactacgccgagctgtgctttcgccactttggcggccaggtgaagtattggatcaccatcgataacccttacgtggtggcctggcacggatacgctacaggccgcctggcccccggcatccgcggcagccccagactgggctacctggtggcccacaacctgctgctggcccacgccaaggtgtggcacctgtacaacaccagcttccgccccacccagggtggacaggtctctattgccctgagctctcactggattaaccccaggaggatgaccgatcacagcatcaaggaatgccagaagagcctggacttcgttctgggctggttcgccaagcccgtgtttatcgacggcgactaccccgagagcatgaagaacaacctgtctagcatcctgcccgacttcaccgagagcgaaaaaaaattcatcaagggcaccgccgatttcttcgccctgtgtttcggcccaaccctgagcttccaactgctggatccccacatgaagttcagacaactcgagagtcccaacctgcgccagctgctgagctggatcgatctggaattcaaccacccccagatattcatagtggagaacggctggtttgtaagcggcactactaagcgcgatgatgcaaagtacatgtactatctgaagaagttcatcatggaaaccctgaaggccatcaagctggatggcgtggacgtgatcggatacaccgcatggagcctgatggacggcttcgagtggcaccgcggttactcaatccgcagggggttgttctacgtcgacttcctgagtcaggacaagatgttgctgccaaagagtagcgcccttttctaccagaagttgattgagaagaacggcttctga

SEQ ID NO: 7 - RNA, 1521 nt, synthetic construct
  source 1..1521: mol_type = other RNA
atgcccgctagcgccccaccgagaagaccgcggccgccaccgccatcgctgtcgctgctgctggtgctgctgggactgggcggaagaagactgcgtgcggagcctggcgacggggcccagacctgggccagattcagcagaccccccgcacccgaggccgccggcctgttccagggcaccttccccgacggatttctgtgggccgtgggaagcgctgcctaccagaccgagggcggctggcaacagcacggcaagggcgccagcatctgggacaccttcacccaccatcctctggctcctcccggagacagcagaaacgccagcctgcctctgggagcccccagccccctgcagcccgccactggagacgtggccagcgactcctacaacaacgtgttccgcgacaccgaggccctgcgcgagctgggcgtgacccactaccgctttagcatcagctgggccagagtgctgcccaacggcagcgccggcgtgcccaaccgggaaggcctgagatactatcgccgcctgctggagaggctgagagagttgggcgtgcagcccgtggtgaccctgtaccactgggacctgccccagcgcctgcaggacgcctacggcggctgggccaacagggcactcgccgaccacttccgcgactacgccgagctgtgcttccgccacttcggcgggcaggtgaagtactggatcaccatcgacaacccctacgtggtggcctggcacggctacgctacaggaaggctggcccccgggatccgcggcagccccaggctgggctacctggtggcccacaacctgctgctggcacacgccaaagtgtggcacctgtataacaccagctttcgccccacccagggtggacaggtgagcattgccctgagttctcattggatcaaccccaggcgcatgaccgatcacagcatcaaggaatgccagaagagcctggacttcgtgctgggctggttcgccaagcccgtgtttatcgacggcgactaccccgagtctatgaagaacaacctcagcagcatcctgcctgacgtcaccgagagcgagaagaagttcatcaagggcaccgccgacttcttcgccctgagcttcggccccaccctgagcttccagctgctggatccccatatgaagttcagacaactcgagagtcctaacctgcgccagctgctgagctggatcgacctggaattcaaccacccacagatcttcatcgtggagaacggctggtttgtgagcggcaccactaagcgcgacgacgcaaagtatatgtattatctgaagaaattcatcatggaaaccctgaaggccatcaagctggacggcgtggacgtgatcggatacaccgcatggagcctgatggacggcttcgagtggcaccgcggttacagcatccgccggggcctgttctacgttgacttcctgagccaggacaagatgttgctgcccaagagctccgccctgttctaccagaagttgatcgagaagaacggcttctga

SEQ ID NO: 8 - RNA, 1521 nt, synthetic construct
  source 1..1521: mol_type = other RNA
atgcccgctagcgccccaccgagaagaccgcggccgccaccgccatcgctgtcgctgctgctggtgctgctgggactgggcggaagaagactgcgtgcggagcctggagatggagcccaaacatgggccagattcagcagacctcccgctcctgaagccgccggcttgtttcagggaacctttcctgacggtttcctgtgggctgtgggcagcgccgcctatcagaccgagggcggctggcaacagcacggaaaaggagccagcatctgggataccttcacccaccaccccctggccccccccggcgattcccgcaatgccagcctccctctgggagcccctagccccctgcaacctgccacaggagacgtggcctcagacagctataacaacgtgttccgcgacaccgaggcactgcgcgagctgggcgtgacccattaccgctttagcatcagctgggccagagtgctgcccaatggctctgccggcgtgcccaaccgggagggcctgaggtactaccgccgcctgctggagaggctgcgggagctgggcgtgcagcccgtggtaaccctgtaccactgggacctgccccagcgcctgcaggacgcttacggcggctgggccaaccgcgctctcgcagaccacttccgcgactacgccgagctgtgctttcgccactttggcggccaggtgaagtattggatcaccatcgataacccttacgtggtggcctggcacggatacgctacaggccgcctggcccccggcatccgcggcagccccagactgggctacctggtggcccacaacctgctgctggcccacgccaaggtgtggcacctgtacaacaccagcttccgccccacccagggtggacaggtctctattgccctgagctctcactggattaaccccaggaggatgaccgatcacagcatcaaggaatgccagaagagcctggacttcgttctgggctggttcgccaagcccgtgtttatcgacggcgactaccccgagagcatgaagaacaacctgtctagcatcctgcccgacgtcaccgagagcgaaaaaaaattcatcaagggcaccgccgatttcttcgccctgagcttcggcccaaccctgagcttccaactgctggatccccacatgaagttcagacaactcgagagtcccaacctgcgccagctgctgagctggatcgatctggaattcaaccacccccagatattcatagtggagaacggctggtttgtaagcggcactactaagcgcgatgatgcaaagtacatgtactatctgaagaagttcatcatggaaaccctgaaggccatcaagctggatggcgtggacgtgatcggatacaccgcatggagcctgatggacggcttcgagtggcaccgcggttactcaatccgcagggggttgttctacgtcgacttcctgagtcaggacaagatgttgctgccaaagagtagcgcccttttctaccagaagttgattgagaagaacggcttctga

SEQ ID NO: 9 - RNA, 2691 nt, synthetic construct
  source 1..2691: mol_type = other RNA
ctgttccagggcaccttccccgacggatttctgtgggccgtgggaagcgctgcctaccagaccgagggcggctggcaacagcacggcaagggcgccagcatctgggacaccttcacccaccatcctctggctcctcccggagacagcagaaacgccagcctgcctctgggagcccccagccccctgcagcccgccactggagacgtggccagcgactcctacaacaacgtgttccgcgacaccgaggccctgcgcgagctgggcgtgacccactaccgctttagcatcagctgggccagagtgctgcccaacggcagcgccggcgtgcccaaccgggaaggcctgagatactatcgccgcctgctggagaggctgagagagttgggcgtgcagcccgtggtgaccctgtaccactgggacctgccccagcgcctgcaggacgcctacggcggctgggccaacagggcactcgccgaccacttccgcgactacgccgagctgtgcttccgccacttcggcgggcaggtgaagtactggatcaccatcgacaacccctacgtggtggcctggcacggctacgctacaggaaggctggcccccgggatccgcggcagccccaggctgggctacctggtggcccacaacctgctgctggcacacgccaaagtgtggcacctgtataacaccagctttcgccccacccagggtggacaggtgagcattgccctgagttctcattggatcaaccccaggcgcatgaccgatcacagcatcaaggaatgccagaagagcctggacttcgtgctgggctggttcgccaagcccgtgtttatcgacggcgactaccccgagtctatgaagaacaacctcagcagcatcctgcctgacttcaccgagagcgagaagaagttcatcaagggcaccgccgacttcttcgccctgtgcttcggccccaccctgagcttccagctgctggatccccatatgaagttcagacaactcgagagtcctaacctgcgccagctgctgagctggatcgacctggaattcaaccacccacagatcttcatcgtggagaacggctggtttgtgagcggcaccactaagcgcgacgacgcaaagtatatgtattatctgaagaaattcatcatggaaaccctgaaggccatcaagctggacggcgtggacgtgatcggatacaccgcatggagcctgatggacggcttcgagtggcaccgcggttacagcatccgccggggcctgttctacgttgacttcctgagccaggacaagatgttgctgcccaagagctccgccctgttctaccagaagttgatcgagaagaacggcttcccaccactccccgagaaccagcccctggagggcaccttcccctgcgatttcgcctggggcgtggtggacaactacatccaggtggacaccaccctgagtcagttcactgacctgaacgtgtacctttgggacgtgcaccacagcaagcgcctgataaaggtcgacggcgtggtgaccaagaagcgcaaaagctactgcgtggactttgccgccatccagccccagatcgccctgctgcaggagatgcacgtgactcacttccgcttcagcctcgactgggccctgattctgcccctgggcaaccagtcacaagtgaaccacaccattctgcagtactaccgctgtatggccagcgagctggtacgcgtgaacatcacccccgttgtggccctttggcagcccatggcccccaaccagggcctgcctcgcctgctggcccgccagggagcctgggagaatccctacaccgcactggccttcgctgaatacgcccgcctgtgcttccaggagctggggcaccacgtgaaactctggatcaccatgaacgagccctacaccagaaacatgacctacagcgccggacacaatctgctgaaggcccacgctctggcctggcacgtgtacaacgagaagtttcgccacgcccagaacggcaagatcagcatcgccctgcaggccgattggatcgagcccgcctgccccttcagccagaaggacaaggaggtggctgagcgggtgctggagttcgacatcgggtggctggctgagcctatcttcggcagcggagactacccctgggtgatgcgcgattggcttaaccagaggaacaatttcctgctgccctacttcaccgaggacgagaagaagctgatccagggcacctttgacttcctggctttgagccactataccactatcctggtggacagcgagaaggaggaccccatcaagtacaacgactacttggaggtgcaggagatgaccgacatcacctggctgaacagccctagccaggtggctgtggtgccttggggcctgcgcaaggtgctgaactggctgaagttcaagtacggcgacctgcccatgtatatcatcagcaacggcatcgacgacggcctgcacgccgaggacgaccagctgagagtgtactacatgcagaactacatcaacgaggccctcaaggcccacatcctggacggcatcaacctgtgtggctactttgcctacagcttcaacgacagaaccgccccccgcttcggcctgtacaggtacgccgccgaccagttcgaacccaaggccagcatgaagcactaccgcaaaatcatcgacagcaacgga

SEQ ID NO: 10 - RNA, 2691 nt, synthetic construct
  source 1..2691: mol_type = other RNA
ttgtttcagggaacctttcctgacggtttcctgtgggctgtgggcagcgccgcctatcagaccgagggcggctggcaacagcacggaaaaggagccagcatctgggataccttcacccaccaccccctggccccccccggcgattcccgcaatgccagcctccctctgggagcccctagccccctgcaacctgccacaggagacgtggcctcagacagctataacaacgtgttccgcgacaccgaggcactgcgcgagctgggcgtgacccattaccgctttagcatcagctgggccagagtgctgcccaatggctctgccggcgtgcccaaccgggagggcctgaggtactaccgccgcctgctggagaggctgcgggagctgggcgtgcagcccgtggtaaccctgtaccactgggacctgccccagcgcctgcaggacgcttacggcggctgggccaaccgcgctctcgcagaccacttccgcgactacgccgagctgtgctttcgccactttggcggccaggtgaagtattggatcaccatcgataacccttacgtggtggcctggcacggatacgctacaggccgcctggcccccggcatccgcggcagccccagactgggctacctggtggcccacaacctgctgctggcccacgccaaggtgtggcacctgtacaacaccagcttccgccccacccagggtggacaggtctctattgccctgagctctcactggattaaccccaggaggatgaccgatcacagcatcaaggaatgccagaagagcctggacttcgttctgggctggttcgccaagcccgtgtttatcgacggcgactaccccgagagcatgaagaacaacctgtctagcatcctgcccgacttcaccgagagcgaaaaaaaattcatcaagggcaccgccgatttcttcgccctgtgtttcggcccaaccctgagcttccaactgctggatccccacatgaagttcagacaactcgagagtcccaacctgcgccagctgctgagctggatcgatctggaattcaaccacccccagatattcatagtggagaacggctggtttgtaagcggcactactaagcgcgatgatgcaaagtacatgtactatctgaagaagttcatcatggaaaccctgaaggccatcaagctggatggcgtggacgtgatcggatacaccgcatggagcctgatggacggcttcgagtggcaccgcggttactcaatccgcagggggttgttctacgtcgacttcctgagtcaggacaagatgttgctgccaaagagtagcgcccttttctaccagaagttgattgagaagaacggcttcccaccactccccgagaaccagcccctggagggcacctttccctgcgatttcgcttggggcgtggtggataattatattcaggtggacaccaccctgtcacagttcactgacctgaacgtgtacctgtgggacgtgcaccattccaagcgcctgatcaaggtggacggcgtggtgaccaagaagcgcaaatcctactgcgttgactttgccgccattcagccacagatcgccctgctgcaggagatgcacgtcacccacttccgcttcagcctggactgggccctcatcctgccactgggcaaccagtcccaggtgaaccacaccattctgcagtactaccgctgtatggccagcgagctggtacgcgtgaacatcacccccgtggtggccctgtggcagcccatggcccccaaccagggcctgccacgcctgctggccaggcagggggcctgggagaacccctacaccgcactcgctttcgccgaatatgccaggctgtgcttccaggagctggggcaccacgtgaagctctggatcaccatgaacgaaccctacaccagaaacatgacctactctgccggacacaatctgctgaaggcccacgccctggcctggcacgtctacaacgagaagttccgccacgcccaaaatggaaagatctctatagccctgcaggccgattggatcgagcccgcctgccccttctcacagaaggacaaggaggtggccgagcgcgtgctggagttcgacatcggctggctggccgagcccatcttcggcagcggagactacccctgggtgatgcgcgattggcttaaccagcgcaacaactttctgctgccctacttcaccgaggacgagaagaagctgatccagggcaccttcgacttcctggccctgagccactatactaccatcctggtcgacagcgagaaggaggacccaatcaagtacaacgactacctggaggtgcaggagatgaccgacatcacctggctgaacagccctagccaggtcgccgtggtgccttggggcctgcgcaaggtgctgaactggctgaagttcaagtatggcgacctgccaatgtacatcatcagcaacggcattgatgacggcctgcacgccgaggacgatcagctgagagtgtactatatgcagaactacatcaacgaggcactgaaggcccacatcctggacggcatcaacctgtgtggctactttgcatactccttcaacgacagaaccgccccccgcttcggcctgtacaggtacgctgccgatcagttcgagcccaaggccagcatgaagcactacagaaaaatcattgatagcaacggg

SEQ ID NO: 11 - RNA, 2691 nt, synthetic construct
  source 1..2691: mol_type = other RNA
ctgttccagggcaccttccccgacggatttctgtgggccgtgggaagcgctgcctaccagaccgagggcggctggcaacagcacggcaagggcgccagcatctgggacaccttcacccaccatcctctggctcctcccggagacagcagaaacgccagcctgcctctgggagcccccagccccctgcagcccgccactggagacgtggccagcgactcctacaacaacgtgttccgcgacaccgaggccctgcgcgagctgggcgtgacccactaccgctttagcatcagctgggccagagtgctgcccaacggcagcgccggcgtgcccaaccgggaaggcctgagatactatcgccgcctgctggagaggctgagagagttgggcgtgcagcccgtggtgaccctgtaccactgggacctgccccagcgcctgcaggacgcctacggcggctgggccaacagggcactcgccgaccacttccgcgactacgccgagctgtgcttccgccacttcggcgggcaggtgaagtactggatcaccatcgacaacccctacgtggtggcctggcacggctacgctacaggaaggctggcccccgggatccgcggcagccccaggctgggctacctggtggcccacaacctgctgctggcacacgccaaagtgtggcacctgtataacaccagctttcgccccacccagggtggacaggtgagcattgccctgagttctcattggatcaaccccaggcgcatgaccgatcacagcatcaaggaatgccagaagagcctggacttcgtgctgggctggttcgccaagcccgtgtttatcgacggcgactaccccgagtctatgaagaacaacctcagcagcatcctgcctgacgtcaccgagagcgagaagaagttcatcaagggcaccgccgacttcttcgccctgagcttcggccccaccctgagcttccagctgctggatccccatatgaagttcagacaactcgagagtcctaacctgcgccagctgctgagctggatcgacctggaattcaaccacccacagatcttcatcgtggagaacggctggtttgtgagcggcaccactaagcgcgacgacgcaaagtatatgtattatctgaagaaattcatcatggaaaccctgaaggccatcaagctggacggcgtggacgtgatcggatacaccgcatggagcctgatggacggcttcgagtggcaccgcggttacagcatccgccggggcctgttctacgttgacttcctgagccaggacaagatgttgctgcccaagagctccgccctgttctaccagaagttgatcgagaagaacggcttcccaccactccccgagaaccagcccctggagggcaccttcccctgcgatttcgcctggggcgtggtggacaactacatccaggtggacaccaccctgagtcagttcactgacctgaacgtgtacctttgggacgtgcaccacagcaagcgcctgataaaggtcgacggcgtggtgaccaagaagcgcaaaagctactgcgtggactttgccgccatccagccccagatcgccctgctgcaggagatgcacgtgactcacttccgcttcagcctcgactgggccctgattctgcccctgggcaaccagtcacaagtgaaccacaccattctgcagtactaccgctgtatggccagcgagctggtacgcgtgaacatcacccccgttgtggccctttggcagcccatggcccccaaccagggcctgcctcgcctgctggcccgccagggagcctgggagaatccctacaccgcactggccttcgctgaatacgcccgcctgtgcttccaggagctggggcaccacgtgaaactctggatcaccatgaacgagccctacaccagaaacatgacctacagcgccggacacaatctgctgaaggcccacgctctggcctggcacgtgtacaacgagaagtttcgccacgcccagaacggcaagatcagcatcgccctgcaggccgattggatcgagcccgcctgccccttcagccagaaggacaaggaggtggctgagcgggtgctggagttcgacatcgggtggctggctgagcctatcttcggcagcggagactacccctgggtgatgcgcgattggcttaaccagaggaacaatttcctgctgccctacttcaccgaggacgagaagaagctgatccagggcacctttgacttcctggctttgagccactataccactatcctggtggacagcgagaaggaggaccccatcaagtacaacgactacttggaggtgcaggagatgaccgacatcacctggctgaacagccctagccaggtggctgtggtgccttggggcctgcgcaaggtgctgaactggctgaagttcaagtacggcgacctgcccatgtatatcatcagcaacggcatcgacgacggcctgcacgccgaggacgaccagctgagagtgtactacatgcagaactacatcaacgaggccctcaaggcccacatcctggacggcatcaacctgtgtggctactttgcctacagcttcaacgacagaaccgccccccgcttcggcctgtacaggtacgccgccgaccagttcgaacccaaggccagcatgaagcactaccgcaaaatcatcgacagcaacgga

SEQ ID NO: 12 - RNA, 2691 nt, synthetic construct
  source 1..2691: mol_type = other RNA
ttgtttcagggaacctttcctgacggtttcctgtgggctgtgggcagcgccgcctatcagaccgagggcggctggcaacagcacggaaaaggagccagcatctgggataccttcacccaccaccccctggccccccccggcgattcccgcaatgccagcctccctctgggagcccctagccccctgcaacctgccacaggagacgtggcctcagacagctataacaacgtgttccgcgacaccgaggcactgcgcgagctgggcgtgacccattaccgctttagcatcagctgggccagagtgctgcccaatggctctgccggcgtgcccaaccgggagggcctgaggtactaccgccgcctgctggagaggctgcgggagctgggcgtgcagcccgtggtaaccctgtaccactgggacctgccccagcgcctgcaggacgcttacggcggctgggccaaccgcgctctcgcagaccacttccgcgactacgccgagctgtgctttcgccactttggcggccaggtgaagtattggatcaccatcgataacccttacgtggtggcctggcacggatacgctacaggccgcctggcccccggcatccgcggcagccccagactgggctacctggtggcccacaacctgctgctggcccacgccaaggtgtggcacctgtacaacaccagcttccgccccacccagggtggacaggtctctattgccctgagctctcactggattaaccccaggaggatgaccgatcacagcatcaaggaatgccagaagagcctggacttcgttctgggctggttcgccaagcccgtgtttatcgacggcgactaccccgagagcatgaagaacaacctgtctagcatcctgcccgacgtcaccgagagcgaaaaaaaattcatcaagggcaccgccgatttcttcgccctgagcttcggcccaaccctgagcttccaactgctggatccccacatgaagttcagacaactcgagagtcccaacctgcgccagctgctgagctggatcgatctggaattcaaccacccccagatattcatagtggagaacggctggtttgtaagcggcactactaagcgcgatgatgcaaagtacatgtactatctgaagaagttcatcatggaaaccctgaaggccatcaagctggatggcgtggacgtgatcggatacaccgcatggagcctgatggacggcttcgagtggcaccgcggttactcaatccgcagggggttgttctacgtcgacttcctgagtcaggacaagatgttgctgccaaagagtagcgcccttttctaccagaagttgattgagaagaacggcttcccaccactccccgagaaccagcccctggagggcacctttccctgcgatttcgcttggggcgtggtggataattatattcaggtggacaccaccctgtcacagttcactgacctgaacgtgtacctgtgggacgtgcaccattccaagcgcctgatcaaggtggacggcgtggtgaccaagaagcgcaaatcctactgcgttgactttgccgccattcagccacagatcgccctgctgcaggagatgcacgtcacccacttccgcttcagcctggactgggccctcatcctgccactgggcaaccagtcccaggtgaaccacaccattctgcagtactaccgctgtatggccagcgagctggtacgcgtgaacatcacccccgtggtggccctgtggcagcccatggcccccaaccagggcctgccacgcctgctggccaggcagggggcctgggagaacccctacaccgcactcgctttcgccgaatatgccaggctgtgcttccaggagctggggcaccacgtgaagctctggatcaccatgaacgaaccctacaccagaaacatgacctactctgccggacacaatctgctgaaggcccacgccctggcctggcacgtctacaacgagaagttccgccacgcccaaaatggaaagatctctatagccctgcaggccgattggatcgagcccgcctgccccttctcacagaaggacaaggaggtggccgagcgcgtgctggagttcgacatcggctggctggccgagcccatcttcggcagcggagactacccctgggtgatgcgcgattggcttaaccagcgcaacaactttctgctgccctacttcaccgaggacgagaagaagctgatccagggcaccttcgacttcctggccctgagccactatactaccatcctggtcgacagcgagaaggaggacccaatcaagtacaacgactacctggaggtgcaggagatgaccgacatcacctggctgaacagccctagccaggtcgccgtggtgccttggggcctgcgcaaggtgctgaactggctgaagttcaagtatggcgacctgccaatgtacatcatcagcaacggcattgatgacggcctgcacgccgaggacgatcagctgagagtgtactatatgcagaactacatcaacgaggcactgaaggcccacatcctggacggcatcaacctgtgtggctactttgcatactccttcaacgacagaaccgccccccgcttcggcctgtacaggtacgctgccgatcagttcgagcccaaggccagcatgaagcactacagaaaaatcattgatagcaacggg

SEQ ID NO: 13 - RNA, 2844 nt, synthetic construct
  source 1..2844: mol_type = other RNA
gagcctggcgacggggcccagacctgggccagattcagcagaccccccgcacccgaggccgccggcctgttccagggcaccttccccgacggatttctgtgggccgtgggaagcgctgcctaccagaccgagggcggctggcaacagcacggcaagggcgccagcatctgggacaccttcacccaccatcctctggctcctcccggagacagcagaaacgccagcctgcctctgggagcccccagccccctgcagcccgccactggagacgtggccagcgactcctacaacaacgtgttccgcgacaccgaggccctgcgcgagctgggcgtgacccactaccgctttagcatcagctgggccagagtgctgcccaacggcagcgccggcgtgcccaaccgggaaggcctgagatactatcgccgcctgctggagaggctgagagagttgggcgtgcagcccgtggtgaccctgtaccactgggacctgccccagcgcctgcaggacgcctacggcggctgggccaacagggcactcgccgaccacttccgcgactacgccgagctgtgcttccgccacttcggcgggcaggtgaagtactggatcaccatcgacaacccctacgtggtggcctggcacggctacgctacaggaaggctggcccccgggatccgcggcagccccaggctgggctacctggtggcccacaacctgctgctggcacacgccaaagtgtggcacctgtataacaccagctttcgccccacccagggtggacaggtgagcattgccctgagttctcattggatcaaccccaggcgcatgaccgatcacagcatcaaggaatgccagaagagcctggacttcgtgctgggctggttcgccaagcccgtgtttatcgacggcgactaccccgagtctatgaagaacaacctcagcagcatcctgcctgacttcaccgagagcgagaagaagttcatcaagggcaccgccgacttcttcgccctgtgcttcggccccaccctgagcttccagctgctggatccccatatgaagttcagacaactcgagagtcctaacctgcgccagctgctgagctggatcgacctggaattcaaccacccacagatcttcatcgtggagaacggctggtttgtgagcggcaccactaagcgcgacgacgcaaagtatatgtattatctgaagaaattcatcatggaaaccctgaaggccatcaagctggacggcgtggacgtgatcggatacaccgcatggagcctgatggacggcttcgagtggcaccgcggttacagcatccgccggggcctgttctacgttgacttcctgagccaggacaagatgttgctgcccaagagctccgccctgttctaccagaagttgatcgagaagaacggcttcccaccactccccgagaaccagcccctggagggcaccttcccctgcgatttcgcctggggcgtggtggacaactacatccaggtggacaccaccctgagtcagttcactgacctgaacgtgtacctttgggacgtgcaccacagcaagcgcctgataaaggtcgacggcgtggtgaccaagaagcgcaaaagctactgcgtggactttgccgccatccagccccagatcgccctgctgcaggagatgcacgtgactcacttccgcttcagcctcgactgggccctgattctgcccctgggcaaccagtcacaagtgaaccacaccattctgcagtactaccgctgtatggccagcgagctggtacgcgtgaacatcacccccgttgtggccctttggcagcccatggcccccaaccagggcctgcctcgcctgctggcccgccagggagcctgggagaatccctacaccgcactggccttcgctgaatacgcccgcctgtgcttccaggagctggggcaccacgtgaaactctggatcaccatgaacgagccctacaccagaaacatgacctacagcgccggacacaatctgctgaaggcccacgctctggcctggcacgtgtacaacgagaagtttcgccacgcccagaacggcaagatcagcatcgccctgcaggccgattggatcgagcccgcctgccccttcagccagaaggacaaggaggtggctgagcgggtgctggagttcgacatcgggtggctggctgagcctatcttcggcagcggagactacccctgggtgatgcgcgattggcttaaccagaggaacaatttcctgctgccctacttcaccgaggacgagaagaagctgatccagggcacctttgacttcctggctttgagccactataccactatcctggtggacagcgagaaggaggaccccatcaagtacaacgactacttggaggtgcaggagatgaccgacatcacctggctgaacagccctagccaggtggctgtggtgccttggggcctgcgcaaggtgctgaactggctgaagttcaagtacggcgacctgcccatgtatatcatcagcaacggcatcgacgacggcctgcacgccgaggacgaccagctgagagtgtactacatgcagaactacatcaacgaggccctcaaggcccacatcctggacggcatcaacctgtgtggctactttgcctacagcttcaacgacagaaccgccccccgcttcggcctgtacaggtacgccgccgaccagttcgaacccaaggccagcatgaagcactaccgcaaaatcatcgacagcaacggattccctggacccgagacactggagcgcttctgcccagaggagttcaccgtgtgcaccgagtgcagtttcttccacacccgcaagagc

SEQ ID NO: 14 - RNA, 2844 nt, synthetic construct
  source 1..2844: mol_type = other RNA
gagcctggagatggagcccaaacatgggccagattcagcagacctcccgctcctgaagccgccggcttgtttcagggaacctttcctgacggtttcctgtgggctgtgggcagcgccgcctatcagaccgagggcggctggcaacagcacggaaaaggagccagcatctgggataccttcacccaccaccccctggccccccccggcgattcccgcaatgccagcctccctctgggagcccctagccccctgcaacctgccacaggagacgtggcctcagacagctataacaacgtgttccgcgacaccgaggcactgcgcgagctgggcgtgacccattaccgctttagcatcagctgggccagagtgctgcccaatggctctgccggcgtgcccaaccgggagggcctgaggtactaccgccgcctgctggagaggctgcgggagctgggcgtgcagcccgtggtaaccctgtaccactgggacctgccccagcgcctgcaggacgcttacggcggctgggccaaccgcgctctcgcagaccacttccgcgactacgccgagctgtgctttcgccactttggcggccaggtgaagtattggatcaccatcgataacccttacgtggtggcctggcacggatacgctacaggccgcctggcccccggcatccgcggcagccccagactgggctacctggtggcccacaacctgctgctggcccacgccaaggtgtggcacctgtacaacaccagcttccgccccacccagggtggacaggtctctattgccctgagctctcactggattaaccccaggaggatgaccgatcacagcatcaaggaatgccagaagagcctggacttcgttctgggctggttcgccaagcccgtgtttatcgacggcgactaccccgagagcatgaagaacaacctgtctagcatcctgcccgacttcaccgagagcgaaaaaaaattcatcaagggcaccgccgatttcttcgccctgtgtttcggcccaaccctgagcttccaactgctggatccccacatgaagttcagacaactcgagagtcccaacctgcgccagctgctgagctggatcgatctggaattcaaccacccccagatattcatagtggagaacggctggtttgtaagcggcactactaagcgcgatgatgcaaagtacatgtactatctgaagaagttcatcatggaaaccctgaaggccatcaagctggatggcgtggacgtgatcggatacaccgcatggagcctgatggacggcttcgagtggcaccgcggttactcaatccgcagggggttgttctacgtcgacttcctgagtcaggacaagatgttgctgccaaagagtagcgcccttttctaccagaagttgattgagaagaacggcttcccaccactccccgagaaccagcccctggagggcacctttccctgcgatttcgcttggggcgtggtggataattatattcaggtggacaccaccctgtcacagttcactgacctgaacgtgtacctgtgggacgtgcaccattccaagcgcctgatcaaggtggacggcgtggtgaccaagaagcgcaaatcctactgcgttgactttgccgccattcagccacagatcgccctgctgcaggagatgcacgtcacccacttccgcttcagcctggactgggccctcatcctgccactgggcaaccagtcccaggtgaaccacaccattctgcagtactaccgctgtatggccagcgagctggtacgcgtgaacatcacccccgtggtggccctgtggcagcccatggcccccaaccagggcctgccacgcctgctggccaggcagggggcctgggagaacccctacaccgcactcgctttcgccgaatatgccaggctgtgcttccaggagctggggcaccacgtgaagctctggatcaccatgaacgaaccctacaccagaaacatgacctactctgccggacacaatctgctgaaggcccacgccctggcctggcacgtctacaacgagaagttccgccacgcccaaaatggaaagatctctatagccctgcaggccgattggatcgagcccgcctgccccttctcacagaaggacaaggaggtggccgagcgcgtgctggagttcgacatcggctggctggccgagcccatcttcggcagcggagactacccctgggtgatgcgcgattggcttaaccagcgcaacaactttctgctgccctacttcaccgaggacgagaagaagctgatccagggcaccttcgacttcctggccctgagccactatactaccatcctggtcgacagcgagaaggaggacccaatcaagtacaacgactacctggaggtgcaggagatgaccgacatcacctggctgaacagccctagccaggtcgccgtggtgccttggggcctgcgcaaggtgctgaactggctgaagttcaagtatggcgacctgccaatgtacatcatcagcaacggcattgatgacggcctgcacgccgaggacgatcagctgagagtgtactatatgcagaactacatcaacgaggcactgaaggcccacatcctggacggcatcaacctgtgtggctactttgcatactccttcaacgacagaaccgccccccgcttcggcctgtacaggtacgctgccgatcagttcgagcccaaggccagcatgaagcactacagaaaaatcattgatagcaacgggttcccaggccccgagaccctggagcgcttctgccccgaggagttcaccgtgtgcaccgagtgcagttttttccacacccgcaagagc

SEQ ID NO: 15 - RNA, 2844 nt, synthetic construct
  source 1..2844: mol_type = other RNA
gagcctggcgacggggcccagacctgggccagattcagcagaccccccgcacccgaggccgccggcctgttccagggcaccttccccgacggatttctgtgggccgtgggaagcgctgcctaccagaccgagggcggctggcaacagcacggcaagggcgccagcatctgggacaccttcacccaccatcctctggctcctcccggagacagcagaaacgccagcctgcctctgggagcccccagccccctgcagcccgccactggagacgtggccagcgactcctacaacaacgtgttccgcgacaccgaggccctgcgcgagctgggcgtgacccactaccgctttagcatcagctgggccagagtgctgcccaacggcagcgccggcgtgcccaaccgggaaggcctgagatactatcgccgcctgctggagaggctgagagagttgggcgtgcagcccgtggtgaccctgtaccactgggacctgccccagcgcctgcaggacgcctacggcggctgggccaacagggcactcgccgaccacttccgcgactacgccgagctgtgcttccgccacttcggcgggcaggtgaagtactggatcaccatcgacaacccctacgtggtggcctggcacggctacgctacaggaaggctggcccccgggatccgcggcagccccaggctgggctacctggtggcccacaacctgctgctggcacacgccaaagtgtggcacctgtataacaccagctttcgccccacccagggtggacaggtgagcattgccctgagttctcattggatcaaccccaggcgcatgaccgatcacagcatcaaggaatgccagaagagcctggacttcgtgctgggctggttcgccaagcccgtgtttatcgacggcgactaccccgagtctatgaagaacaacctcagcagcatcctgcctgacgtcaccgagagcgagaagaagttcatcaagggcaccgccgacttcttcgccctgagcttcggccccaccctgagcttccagctgctggatccccatatgaagttcagacaactcgagagtcctaacctgcgccagctgctgagctggatcgacctggaattcaaccacccacagatcttcatcgtggagaacggctggtttgtgagcggcaccactaagcgcgacgacgcaaagtatatgtattatctgaagaaattcatcatggaaaccctgaaggccatcaagctggacggcgtggacgtgatcggatacaccgcatggagcctgatggacggcttcgagtggcaccgcggttacagcatccgccggggcctgttctacgttgacttcctgagccaggacaagatgttgctgcccaagagctccgccctgttctaccagaagttgatcgagaagaacggcttcccaccactccccgagaaccagcccctggagggcaccttcccctgcgatttcgcctggggcgtggtggacaactacatccaggtggacaccaccctgagtcagttcactgacctgaacgtgtacctttgggacgtgcaccacagcaagcgcctgataaaggtcgacggcgtggtgaccaagaagcgcaaaagctactgcgtggactttgccgccatccagccccagatcgccctgctgcaggagatgcacgtgactcacttccgcttcagcctcgactgggccctgattctgcccctgggcaaccagtcacaagtgaaccacaccattctgcagtactaccgctgtatggccagcgagctggtacgcgtgaacatcacccccgttgtggccctttggcagcccatggcccccaaccagggcctgcctcgcctgctggcccgccagggagcctgggagaatccctacaccgcactggccttcgctgaatacgcccgcctgtgcttccaggagctggggcaccacgtgaaactctggatcaccatgaacgagccctacaccagaaacatgacctacagcgccggacacaatctgctgaaggcccacgctctggcctggcacgtgtacaacgagaagtttcgccacgcccagaacggcaagatcagcatcgccctgcaggccgattggatcgagcccgcctgccccttcagccagaaggacaaggaggtggctgagcgggtgctggagttcgacatcgggtggctggctgagcctatcttcggcagcggagactacccctgggtgatgcgcgattggcttaaccagaggaacaatttcctgctgccctacttcaccgaggacgagaagaagctgatccagggcacctttgacttcctggctttgagccactataccactatcctggtggacagcgagaaggaggaccccatcaagtacaacgactacttggaggtgcaggagatgaccgacatcacctggctgaacagccctagccaggtggctgtggtgccttggggcctgcgcaaggtgctgaactggctgaagttcaagtacggcgacctgcccatgtatatcatcagcaacggcatcgacgacggcctgcacgccgaggacgaccagctgagagtgtactacatgcagaactacatcaacgaggccctcaaggcccacatcctggacggcatcaacctgtgtggctactttgcctacagcttcaacgacagaaccgccccccgcttcggcctgtacaggtacgccgccgaccagttcgaacccaaggccagcatgaagcactaccgcaaaatcatcgacagcaacggattccctggacccgagacactggagcgcttctgcccagaggagttcaccgtgtgcaccgagtgcagtttcttccacacccgcaagagc

SEQ ID NO: 16 - RNA, 2844 nt, synthetic construct
  source 1..2844: mol_type = other RNA
gagcctggagatggagcccaaacatgggccagattcagcagacctcccgctcctgaagccgccggcttgtttcagggaacctttcctgacggtttcctgtgggctgtgggcagcgccgcctatcagaccgagggcggctggcaacagcacggaaaaggagccagcatctgggataccttcacccaccaccccctggccccccccggcgattcccgcaatgccagcctccctctgggagcccctagccccctgcaacctgccacaggagacgtggcctcagacagctataacaacgtgttccgcgacaccgaggcactgcgcgagctgggcgtgacccattaccgctttagcatcagctgggccagagtgctgcccaatggctctgccggcgtgcccaaccgggagggcctgaggtactaccgccgcctgctggagaggctgcgggagctgggcgtgcagcccgtggtaaccctgtaccactgggacctgccccagcgcctgcaggacgcttacggcggctgggccaaccgcgctctcgcagaccacttccgcgactacgccgagctgtgctttcgccactttggcggccaggtgaagtattggatcaccatcgataacccttacgtggtggcctggcacggatacgctacaggccgcctggcccccggcatccgcggcagccccagactgggctacctggtggcccacaacctgctgctggcccacgccaaggtgtggcacctgtacaacaccagcttccgccccacccagggtggacaggtctctattgccctgagctctcactggattaaccccaggaggatgaccgatcacagcatcaaggaatgccagaagagcctggacttcgttctgggctggttcgccaagcccgtgtttatcgacggcgactaccccgagagcatgaagaacaacctgtctagcatcctgcccgacgtcaccgagagcgaaaaaaaattcatcaagggcaccgccgatttcttcgccctgagcttcggcccaaccctgagcttccaactgctggatccccacatgaagttcagacaactcgagagtcccaacctgcgccagctgctgagctggatcgatctggaattcaaccacccccagatattcatagtggagaacggctggtttgtaagcggcactactaagcgcgatgatgcaaagtacatgtactatctgaagaagttcatcatggaaaccctgaaggccatcaagctggatggcgtggacgtgatcggatacaccgcatggagcctgatggacggcttcgagtggcaccgcggttactcaatccgcagggggttgttctacgtcgacttcctgagtcaggacaagatgttgctgccaaagagtagcgcccttttctaccagaagttgattgagaagaacggcttcccaccactccccgagaaccagcccctggagggcacctttccctgcgatttcgcttggggcgtggtggataattatattcaggtggacaccaccctgtcacagttcactgacctgaacgtgtacctgtgggacgtgcaccattccaagcgcctgatcaaggtggacggcgtggtgaccaagaagcgcaaatcctactgcgttgactttgccgccattcagccacagatcgccctgctgcaggagatgcacgtcacccacttccgcttcagcctggactgggccctcatcctgccactgggcaaccagtcccaggtgaaccacaccattctgcagtactaccgctgtatggccagcgagctggtacgcgtgaacatcacccccgtggtggccctgtggcagcccatggcccccaaccagggcctgccacgcctgctggccaggcagggggcctgggagaacccctacaccgcactcgctttcgccgaatatgccaggctgtgcttccaggagctggggcaccacgtgaagctctggatcaccatgaacgaaccctacaccagaaacatgacctactctgccggacacaatctgctgaaggcccacgccctggcctggcacgtctacaacgagaagttccgccacgcccaaaatggaaagatctctatagccctgcaggccgattggatcgagcccgcctgccccttctcacagaaggacaaggaggtggccgagcgcgtgctggagttcgacatcggctggctggccgagcccatcttcggcagcggagactacccctgggtgatgcgcgattggcttaaccagcgcaacaactttctgctgccctacttcaccgaggacgagaagaagctgatccagggcaccttcgacttcctggccctgagccactatactaccatcctggtcgacagcgagaaggaggacccaatcaagtacaacgactacctggaggtgcaggagatgaccgacatcacctggctgaacagccctagccaggtcgccgtggtgccttggggcctgcgcaaggtgctgaactggctgaagttcaagtatggcgacctgccaatgtacatcatcagcaacggcattgatgacggcctgcacgccgaggacgatcagctgagagtgtactatatgcagaactacatcaacgaggcactgaaggcccacatcctggacggcatcaacctgtgtggctactttgcatactccttcaacgacagaaccgccccccgcttcggcctgtacaggtacgctgccgatcagttcgagcccaaggccagcatgaagcactacagaaaaatcattgatagcaacgggttcccaggccccgagaccctggagcgcttctgccccgaggagttcaccgtgtgcaccgagtgcagttttttccacacccgcaagagc

SEQ ID NO: 17 - RNA, 2946 nt, Homo sapiens
  source 1..2946: mol_type = other RNA
atgcccgccagcgccccgccgcgccgcccgcggccgccgccgccgtcgctgtcgctgctgctggtgctgctgggcctgggcggccgccgcctgcgtgcggagccgggcgacggcgcgcagacctgggcccgtttctcgcggcctcctgcccccgaggccgcgggcctcttccagggcaccttccccgacggcttcctctgggccgtgggcagcgccgcctaccagaccgagggcggctggcagcagcacggcaagggtgcgtccatctgggatacgttcacccaccaccccctggcacccccgggagactcccggaacgccagtctgccgttgggcgccccgtcgccgctgcagcccgccaccggggacgtagccagcgacagctacaacaacgtcttccgcgacacggaggcgctgcgcgagctcggggtcactcactaccgcttctccatctcgtgggcgcgagtgctccccaatggcagcgcgggcgtccccaaccgcgaggggctgcgctactaccggcgcctgctggagcggctgcgggagctgggcgtgcagcccgtggtcaccctgtaccactgggacctgccccagcgcctgcaggacgcctacggcggctgggccaaccgcgccctggccgaccacttcagggattacgcggagctctgcttccgccacttcggcggtcaggtcaagtactggatcaccatcgacaacccctacgtggtggcctggcacggctacgccaccgggcgcctggcccccggcatccggggcagcccgcggctcgggtacctggtggcgcacaacctcctcctggctcatgccaaagtctggcatctctacaatacttctttccgtcccactcagggaggtcaggtgtccattgccctaagctctcactggatcaatcctcgaagaatgaccgaccacagcatcaaagaatgtcaaaaatctctggactttgtactaggttggtttgccaaacccgtatttattgatggtgactatcccgagagcatgaagaataacctttcatctattctgcctgattttactgaatctgagaaaaagttcatcaaaggaactgctgacttttttgctctttgctttggacccaccttgagttttcaacttttggaccctcacatgaagttccgccaattggaatctcccaacctgaggcaactgctttcctggattgaccttgaatttaaccatcctcaaatatttattgtggaaaatggctggtttgtctcagggaccaccaagagagatgatgccaaatatatgtattacctcaaaaagttcatcatggaaaccttaaaagccatcaagctggatggggtggatgtcatcgggtataccgcatggtccctcatggatggtttcgagtggcacagaggttacagcatcaggcgtggactcttctatgttgactttctaagccaggacaagatgttgttgccaaagtcttcagccttgttctaccaaaagctgatagagaaaaatggcttccctcctttacctgaaaatcagcccctagaagggacatttccctgtgactttgcttggggagttgttgacaactacattcaagtagataccactctgtctcagtttaccgacctgaatgtttacctgtgggatgtccaccacagtaaaaggcttattaaagtggatggggttgtgaccaagaagaggaaatcctactgtgttgactttgctgccatccagccccagatcgctttactccaggaaatgcacgttacacattttcgcttctccctggactgggccctgattctccctctgggtaaccagtcccaggtgaaccacaccatcctgcagtactatcgctgcatggccagcgagcttgtccgtgtcaacatcaccccagtggtggccctgtggcagcctatggccccgaaccaaggactgccgcgcctcctggccaggcagggcgcctgggagaacccctacactgccctggcctttgcagagtatgcccgactgtgctttcaagagctcggccatcacgtcaagctttggataacgatgaatgagccgtatacaaggaatatgacatacagtgctggccacaaccttctgaaggcccatgccctggcttggcatgtgtacaatgaaaagtttaggcatgctcagaatgggaaaatatccatagccttgcaggctgattggatagaacctgcctgccctttctcccaaaaggacaaagaggtggctgagagagttttggaatttgacattggctggctggctgagcccattttcggctctggagattatccatgggtgatgagggactggctgaaccaaagaaacaattttcttcttccttatttcactgaagatgaaaaaaagctaatccagggtacctttgactttttggctttaagccattataccaccatccttgtagactcagaaaaagaagatccaataaaatacaatgattacctagaagtgcaagaaatgaccgacatcacgtggctcaactcccccagtcaggtggcggtagtgccctgggggttgcgcaaagtgctgaactggctgaagttcaagtacggagacctccccatgtacataatatccaatggaatcgatgacgggctgcatgctgaggacgaccagctgagggtgtattatatgcagaattacataaacgaagctctcaaagcccacatactggatggtatcaatctttgcggatactttgcttattcgtttaacgaccgcacagctccgaggtttggcctctatcgttatgctgcagatcagtttgagcccaaggcatccatgaaacattacaggaaaattattgacagcaatggtttcccgggcccagaaactctggaaagattttgtccagaagaattcaccgtgtgtactgagtgcagtttttttcacacccgaaagtcttga

SEQ ID NO: 18 - RNA, 2946 nt, synthetic construct
  source 1..2946: mol_type = other RNA
atgcccgctagcgccccaccgagaagaccgcggccgccaccgccatcgctgtcgctgctgctggtgctgctgggactgggcggaagaagactgcgtgcggagcctggcgacggggcccagacctgggccagattcagcagaccccccgcacccgaggccgccggcctgttccagggcaccttccccgacggatttctgtgggccgtgggaagcgctgcctaccagaccgagggcggctggcaacagcacggcaagggcgccagcatctgggacaccttcacccaccatcctctggctcctcccggagacagcagaaacgccagcctgcctctgggagcccccagccccctgcagcccgccactggagacgtggccagcgactcctacaacaacgtgttccgcgacaccgaggccctgcgcgagctgggcgtgacccactaccgctttagcatcagctgggccagagtgctgcccaacggcagcgccggcgtgcccaaccgggaaggcctgagatactatcgccgcctgctggagaggctgagagagttgggcgtgcagcccgtggtgaccctgtaccactgggacctgccccagcgcctgcaggacgcctacggcggctgggccaacagggcactcgccgaccacttccgcgactacgccgagctgtgcttccgccacttcggcgggcaggtgaagtactggatcaccatcgacaacccctacgtggtggcctggcacggctacgctacaggaaggctggcccccgggatccgcggcagccccaggctgggctacctggtggcccacaacctgctgctggcacacgccaaagtgtggcacctgtataacaccagctttcgccccacccagggtggacaggtgagcattgccctgagttctcattggatcaaccccaggcgcatgaccgatcacagcatcaaggaatgccagaagagcctggacttcgtgctgggctggttcgccaagcccgtgtttatcgacggcgactaccccgagtctatgaagaacaacctcagcagcatcctgcctgacttcaccgagagcgagaagaagttcatcaagggcaccgccgacttcttcgccctgtgcttcggccccaccctgagcttccagctgctggatccccatatgaagttcagacaactcgagagtcctaacctgcgccagctgctgagctggatcgacctggaattcaaccacccacagatcttcatcgtggagaacggctggtttgtgagcggcaccactaagcgcgacgacgcaaagtatatgtattatctgaagaaattcatcatggaaaccctgaaggccatcaagctggacggcgtggacgtgatcggatacaccgcatggagcctgatggacggcttcgagtggcaccgcggttacagcatccgccggggcctgttctacgttgacttcctgagccaggacaagatgttgctgcccaagagctccgccctgttctaccagaagttgatcgagaagaacggcttcccaccactccccgagaaccagcccctggagggcaccttcccctgcgatttcgcctggggcgtggtggacaactacatccaggtggacaccaccctgagtcagttcactgacctgaacgtgtacctttgggacgtgcaccacagcaagcgcctgataaaggtcgacggcgtggtgaccaagaagcgcaaaagctactgcgtggactttgccgccatccagccccagatcgccctgctgcaggagatgcacgtgactcacttccgcttcagcctcgactgggccctgattctgcccctgggcaaccagtcacaagtgaaccacaccattctgcagtactaccgctgtatggccagcgagctggtacgcgtgaacatcacccccgttgtggccctttggcagcccatggcccccaaccagggcctgcctcgcctgctggcccgccagggagcctgggagaatccctacaccgcactggccttcgctgaatacgcccgcctgtgcttccaggagctggggcaccacgtgaaactctggatcaccatgaacgagccctacaccagaaacatgacctacagcgccggacacaatctgctgaaggcccacgctctggcctggcacgtgtacaacgagaagtttcgccacgcccagaacggcaagatcagcatcgccctgcaggccgattggatcgagcccgcctgccccttcagccagaaggacaaggaggtggctgagcgggtgctggagttcgacatcgggtggctggctgagcctatcttcggcagcggagactacccctgggtgatgcgcgattggcttaaccagaggaacaatttcctgctgccctacttcaccgaggacgagaagaagctgatccagggcacctttgacttcctggctttgagccactataccactatcctggtggacagcgagaaggaggaccccatcaagtacaacgactacttggaggtgcaggagatgaccgacatcacctggctgaacagccctagccaggtggctgtggtgccttggggcctgcgcaaggtgctgaactggctgaagttcaagtacggcgacctgcccatgtatatcatcagcaacggcatcgacgacggcctgcacgccgaggacgaccagctgagagtgtactacatgcagaactacatcaacgaggccctcaaggcccacatcctggacggcatcaacctgtgtggctactttgcctacagcttcaacgacagaaccgccccccgcttcggcctgtacaggtacgccgccgaccagttcgaacccaaggccagcatgaagcactaccgcaaaatcatcgacagcaacggattccctggacccgagacactggagcgcttctgcccagaggagttcaccgtgtgcaccgagtgcagtttcttccacacccgcaagagctga

SEQ ID NO: 19 - RNA, 2946 nt, synthetic construct
  source 1..2946: mol_type = other RNA
atgcccgctagcgccccaccgagaagaccgcggccgccaccgccatcgctgtcgctgctgctggtgctgctgggactgggcggaagaagactgcgtgcggagcctggagatggagcccaaacatgggccagattcagcagacctcccgctcctgaagccgccggcttgtttcagggaacctttcctgacggtttcctgtgggctgtgggcagcgccgcctatcagaccgagggcggctggcaacagcacggaaaaggagccagcatctgggataccttcacccaccaccccctggccccccccggcgattcccgcaatgccagcctccctctgggagcccctagccccctgcaacctgccacaggagacgtggcctcagacagctataacaacgtgttccgcgacaccgaggcactgcgcgagctgggcgtgacccattaccgctttagcatcagctgggccagagtgctgcccaatggctctgccggcgtgcccaaccgggagggcctgaggtactaccgccgcctgctggagaggctgcgggagctgggcgtgcagcccgtggtaaccctgtaccactgggacctgccccagcgcctgcaggacgcttacggcggctgggccaaccgcgctctcgcagaccacttccgcgactacgccgagctgtgctttcgccactttggcggccaggtgaagtattggatcaccatcgataacccttacgtggtggcctggcacggatacgctacaggccgcctggcccccggcatccgcggcagccccagactgggctacctggtggcccacaacctgctgctggcccacgccaaggtgtggcacctgtacaacaccagcttccgccccacccagggtggacaggtctctattgccctgagctctcactggattaaccccaggaggatgaccgatcacagcatcaaggaatgccagaagagcctggacttcgttctgggctggttcgccaagcccgtgtttatcgacggcgactaccccgagagcatgaagaacaacctgtctagcatcctgcccgacttcaccgagagcgaaaaaaaattcatcaagggcaccgccgatttcttcgccctgtgtttcggcccaaccctgagcttccaactgctggatccccacatgaagttcagacaactcgagagtcccaacctgcgccagctgctgagctggatcgatctggaattcaaccacccccagatattcatagtggagaacggctggtttgtaagcggcactactaagcgcgatgatgcaaagtacatgtactatctgaagaagttcatcatggaaaccctgaaggccatcaagctggatggcgtggacgtgatcggatacaccgcatggagcctgatggacggcttcgagtggcaccgcggttactcaatccgcagggggttgttctacgtcgacttcctgagtcaggacaagatgttgctgccaaagagtagcgcccttttctaccagaagttgattgagaagaacggcttcccaccactccccgagaaccagcccctggagggcacctttccctgcgatttcgcttggggcgtggtggataattatattcaggtggacaccaccctgtcacagttcactgacctgaacgtgtacctgtgggacgtgcaccattccaagcgcctgatcaaggtggacggcgtggtgaccaagaagcgcaaatcctactgcgttgactttgccgccattcagccacagatcgccctgctgcaggagatgcacgtcacccacttccgcttcagcctggactgggccctcatcctgccactgggcaaccagtcccaggtgaaccacaccattctgcagtactaccgctgtatggccagcgagctggtacgcgtgaacatcacccccgtggtggccctgtggcagcccatggcccccaaccagggcctgccacgcctgctggccaggcagggggcctgggagaacccctacaccgcactcgctttcgccgaatatgccaggctgtgcttccaggagctggggcaccacgtgaagctctggatcaccatgaacgaaccctacaccagaaacatgacctactctgccggacacaatctgctgaaggcccacgccctggcctggcacgtctacaacgagaagttccgccacgcccaaaatggaaagatctctatagccctgcaggccgattggatcgagcccgcctgccccttctcacagaaggacaaggaggtggccgagcgcgtgctggagttcgacatcggctggctggccgagcccatcttcggcagcggagactacccctgggtgatgcgcgattggcttaaccagcgcaacaactttctgctgccctacttcaccgaggacgagaagaagctgatccagggcaccttcgacttcctggccctgagccactatactaccatcctggtcgacagcgagaaggaggacccaatcaagtacaacgactacctggaggtgcaggagatgaccgacatcacctggctgaacagccctagccaggtcgccgtggtgccttggggcctgcgcaaggtgctgaactggctgaagttcaagtatggcgacctgccaatgtacatcatcagcaacggcattgatgacggcctgcacgccgaggacgatcagctgagagtgtactatatgcagaactacatcaacgaggcactgaaggcccacatcctggacggcatcaacctgtgtggctactttgcatactccttcaacgacagaaccgccccccgcttcggcctgtacaggtacgctgccgatcagttcgagcccaaggccagcatgaagcactacagaaaaatcattgatagcaacgggttcccaggccccgagaccctggagcgcttctgccccgaggagttcaccgtgtgcaccgagtgcagttttttccacacccgcaagagctga

SEQ ID NO: 20 - RNA, 2946 nt, synthetic construct
  source 1..2946: mol_type = other RNA
atgcccgctagcgccccaccgagaagaccgcggccgccaccgccatcgctgtcgctgctgctggtgctgctgggactgggcggaagaagactgcgtgcggagcctggcgacggggcccagacctgggccagattcagcagaccccccgcacccgaggccgccggcctgttccagggcaccttccccgacggatttctgtgggccgtgggaagcgctgcctaccagaccgagggcggctggcaacagcacggcaagggcgccagcatctgggacaccttcacccaccatcctctggctcctcccggagacagcagaaacgccagcctgcctctgggagcccccagccccctgcagcccgccactggagacgtggccagcgactcctacaacaacgtgttccgcgacaccgaggccctgcgcgagctgggcgtgacccactaccgctttagcatcagctgggccagagtgctgcccaacggcagcgccggcgtgcccaaccgggaaggcctgagatactatcgccgcctgctggagaggctgagagagttgggcgtgcagcccgtggtgaccctgtaccactgggacctgccccagcgcctgcaggacgcctacggcggctgggccaacagggcactcgccgaccacttccgcgactacgccgagctgtgcttccgccacttcggcgggcaggtgaagtactggatcaccatcgacaacccctacgtggtggcctggcacggctacgctacaggaaggctggcccccgggatccgcggcagccccaggctgggctacctggtggcccacaacctgctgctggcacacgccaaagtgtggcacctgtataacaccagctttcgccccacccagggtggacaggtgagcattgccctgagttctcattggatcaaccccaggcgcatgaccgatcacagcatcaaggaatgccagaagagcctggacttcgtgctgggctggttcgccaagcccgtgtttatcgacggcgactaccccgagtctatgaagaacaacctcagcagcatcctgcctgacgtcaccgagagcgagaagaagttcatcaagggcaccgccgacttcttcgccctgagcttcggccccaccctgagcttccagctgctggatccccatatgaagttcagacaactcgagagtcctaacctgcgccagctgctgagctggatcgacctggaattcaaccacccacagatcttcatcgtggagaacggctggtttgtgagcggcaccactaagcgcgacgacgcaaagtatatgtattatctgaagaaattcatcatggaaaccctgaaggccatcaagctggacggcgtggacgtgatcggatacaccgcatggagcctgatggacggcttcgagtggcaccgcggttacagcatccgccggggcctgttctacgttgacttcctgagccaggacaagatgttgctgcccaagagctccgccctgttctaccagaagttgatcgagaagaacggcttcccaccactccccgagaaccagcccctggagggcaccttcccctgcgatttcgcctggggcgtggtggacaactacatccaggtggacaccaccctgagtcagttcactgacctgaacgtgtacctttgggacgtgcaccacagcaagcgcctgataaaggtcgacggcgtggtgaccaagaagcgcaaaagctactgcgtggactttgccgccatccagccccagatcgccctgctgcaggagatgcacgtgactcacttccgcttcagcctcgactgggccctgattctgcccctgggcaaccagtcacaagtgaaccacaccattctgcagtactaccgctgtatggccagcgagctggtacgcgtgaacatcacccccgttgtggccctttggcagcccatggcccccaaccagggcctgcctcgcctgctggcccgccagggagcctgggagaatccctacaccgcactggccttcgctgaatacgcccgcctgtgcttccaggagctggggcaccacgtgaaactctggatcaccatgaacgagccctacaccagaaacatgacctacagcgccggacacaatctgctgaaggcccacgctctggcctggcacgtgtacaacgagaagtttcgccacgcccagaacggcaagatcagcatcgccctgcaggccgattggatcgagcccgcctgccccttcagccagaaggacaaggaggtggctgagcgggtgctggagttcgacatcgggtggctggctgagcctatcttcggcagcggagactacccctgggtgatgcgcgattggcttaaccagaggaacaatttcctgctgccctacttcaccgaggacgagaagaagctgatccagggcacctttgacttcctggctttgagccactataccactatcctggtggacagcgagaaggaggaccccatcaagtacaacgactacttggaggtgcaggagatgaccgacatcacctggctgaacagccctagccaggtggctgtggtgccttggggcctgcgcaaggtgctgaactggctgaagttcaagtacggcgacctgcccatgtatatcatcagcaacggcatcgacgacggcctgcacgccgaggacgaccagctgagagtgtactacatgcagaactacatcaacgaggccctcaaggcccacatcctggacggcatcaacctgtgtggctactttgcctacagcttcaacgacagaaccgccccccgcttcggcctgtacaggtacgccgccgaccagttcgaacccaaggccagcatgaagcactaccgcaaaatcatcgacagcaacggattccctggacccgagacactggagcgcttctgcccagaggagttcaccgtgtgcaccgagtgcagtttcttccacacccgcaagagctga

SEQ ID NO: 21 - RNA, 2946 nt, synthetic construct
  source 1..2946: mol_type = other RNA
atgcccgctagcgccccaccgagaagaccgcggccgccaccgccatcgctgtcgctgctgctggtgctgctgggactgggcggaagaagactgcgtgcggagcctggagatggagcccaaacatgggccagattcagcagacctcccgctcctgaagccgccggcttgtttcagggaacctttcctgacggtttcctgtgggctgtgggcagcgccgcctatcagaccgagggcggctggcaacagcacggaaaaggagccagcatctgggataccttcacccaccaccccctggccccccccggcgattcccgcaatgccagcctccctctgggagcccctagccccctgcaacctgccacaggagacgtggcctcagacagctataacaacgtgttccgcgacaccgaggcactgcgcgagctgggcgtgacccattaccgctttagcatcagctgggccagagtgctgcccaatggctctgccggcgtgcccaaccgggagggcctgaggtactaccgccgcctgctggagaggctgcgggagctgggcgtgcagcccgtggtaaccctgtaccactgggacctgccccagcgcctgcaggacgcttacggcggctgggccaaccgcgctctcgcagaccacttccgcgactacgccgagctgtgctttcgccactttggcggccaggtgaagtattggatcaccatcgataacccttacgtggtggcctggcacggatacgctacaggccgcctggcccccggcatccgcggcagccccagactgggctacctggtggcccacaacctgctgctggcccacgccaaggtgtggcacctgtacaacaccagcttccgccccacccagggtggacaggtctctattgccctgagctctcactggattaaccccaggaggatgaccgatcacagcatcaaggaatgccagaagagcctggacttcgttctgggctggttcgccaagcccgtgtttatcgacggcgactaccccgagagcatgaagaacaacctgtctagcatcctgcccgacgtcaccgagagcgaaaaaaaattcatcaagggcaccgccgatttcttcgccctgagcttcggcccaaccctgagcttccaactgctggatccccacatgaagttcagacaactcgagagtcccaacctgcgccagctgctgagctggatcgatctggaattcaaccacccccagatattcatagtggagaacggctggtttgtaagcggcactactaagcgcgatgatgcaaagtacatgtactatctgaagaagttcatcatggaaaccctgaaggccatcaagctggatggcgtggacgtgatcggatacaccgcatggagcctgatggacggcttcgagtggcaccgcggttactcaatccgcagggggttgttctacgtcgacttcctgagtcaggacaagatgttgctgccaaagagtagcgcccttttctaccagaagttgattgagaagaacggcttcccaccactccccgagaaccagcccctggagggcacctttccctgcgatttcgcttggggcgtggtggataattatattcaggtggacaccaccctgtcacagttcactgacctgaacgtgtacctgtgggacgtgcaccattccaagcgcctgatcaaggtggacggcgtggtgaccaagaagcgcaaatcctactgcgttgactttgccgccattcagccacagatcgccctgctgcaggagatgcacgtcacccacttccgcttcagcctggactgggccctcatcctgccactgggcaaccagtcccaggtgaaccacaccattctgcagtactaccgctgtatggccagcgagctggtacgcgtgaacatcacccccgtggtggccctgtggcagcccatggcccccaaccagggcctgccacgcctgctggccaggcagggggcctgggagaacccctacaccgcactcgctttcgccgaatatgccaggctgtgcttccaggagctggggcaccacgtgaagctctggatcaccatgaacgaaccctacaccagaaacatgacctactctgccggacacaatctgctgaaggcccacgccctggcctggcacgtctacaacgagaagttccgccacgcccaaaatggaaagatctctatagccctgcaggccgattggatcgagcccgcctgccccttctcacagaaggacaaggaggtggccgagcgcgtgctggagttcgacatcggctggctggccgagcccatcttcggcagcggagactacccctgggtgatgcgcgattggcttaaccagcgcaacaactttctgctgccctacttcaccgaggacgagaagaagctgatccagggcaccttcgacttcctggccctgagccactatactaccatcctggtcgacagcgagaaggaggacccaatcaagtacaacgactacctggaggtgcaggagatgaccgacatcacctggctgaacagccctagccaggtcgccgtggtgccttggggcctgcgcaaggtgctgaactggctgaagttcaagtatggcgacctgccaatgtacatcatcagcaacggcattgatgacggcctgcacgccgaggacgatcagctgagagtgtactatatgcagaactacatcaacgaggcactgaaggcccacatcctggacggcatcaacctgtgtggctactttgcatactccttcaacgacagaaccgccccccgcttcggcctgtacaggtacgctgccgatcagttcgagcccaaggccagcatgaagcactacagaaaaatcattgatagcaacgggttcccaggccccgagaccctggagcgcttctgccccgaggagttcaccgtgtgcaccgagtgcagttttttccacacccgcaagagctga

SEQ ID NO: 22 - RNA, 2946 nt, synthetic construct
  source 1..2946: mol_type = other RNA
atgcccgctagcgccccaccgagaagaccgcggccgccaccgccatcgctgtcgctgctgctggtgctgctgggactgggcggaagaagactgcgtgcggagccaggcgatggcgcccagacttgggcccgcttcagcagacctcccgcccccgaggccgccggattgttccagggaaccttccctgacggtttcctgtgggccgtgggtagcgccgcctaccagaccgagggcggctggcagcagcacggcaagggcgcaagcatctgggacacctttacccaccaccccctggccccccccggcgacagtagaaatgctagtctccccctgggcgcccccagcccccttcagcccgccaccggagacgtggcctcagacagctacaacaacgtgttcagagacaccgaagctctgagggagctcggcgtgacccactatcggtttagcattagctgggccagagtgctgcccaacggcagcgccggcgtgcccaaccgcgaaggcctcagatactatcgcagactgctggagaggctgcgggagctgggcgtgcagcccgtggtaactctgtaccactgggatctgccccagagattgcaagacgcttacggcggatgggccaaccgcgctctcgccgaccacttccgggactacgcagagctgtgcttccgccacttcggcggtcaggtgaaatattggattacaatcgacaacccctacgttgtggcctggcacgggtacgctactgggcgcctggcacccggcatccgcggcagccccagactgggctaccttgttgctcacaacctcctgctggctcatgcaaaggtgtggcacttgtacaacacaagtttccgccccacccagggtggacaggtgtcaatcgcactgtcttcacactggattaacccccggcgcatgactgaccactcaattaaggaatgccagaagagcctggacttcgttctgggctggttcgccaagcccgtgtttatcgacggggactaccccgagagcatgaagaataatctgagcagcatcttgcccgactttaccgagagcgaaaagaaattcatcaagggcaccgccgactttttcgcactgtgtttcggccccactctgagctttcaactgctcgatccccacatgaagtttagacaactggagtcccctaatctgcgccagcttctgagctggattgatctggaatttaaccatccccagatttttatagttgagaatgggtggtttgttagcggcaccactaagcgcgatgacgcaaagtacatgtattatctgaagaaatttatcatggaaactctgaaggccataaaactcgacggcgttgacgtgatcggttataccgcatggagccttatggacgggttcgagtggcaccgcgggtactccatcaggaggggcttgttctacgtcgacttcctcagtcaggacaagatgttgctgcctaagagcagcgccttgttctaccagaagttgatcgaaaagaacggctttccaccactccccgagaaccaacccctggagggcacctttccctgcgatttcgcttggggcgtggtggacaactacatccaggtggataccactctgtctcagttcactgatctcaacgtgtatctgtgggacgtccaccactccaagaggctgatcaaggtggacggcgtcgtgaccaagaagagaaagtcctactgcgtggactttgccgccattcagccccagatcgccctgctgcaggagatgcatgtcacacacttccgcttttctctggactgggccctgattctgcccctggggaaccagtcccaggtcaaccacaccattctccagtactaccgctgtatggccagtgagctggtacgcgtgaacatcacccccgtcgtggccctctggcagcccatggcccccaatcagggcctgccacgcctgctcgcccggcagggagcctgggaaaatccatacactgcactcgccttcgctgagtacgccaggctgtgcttccaggagctgggacatcacgtgaagctgtggattaccatgaacgaaccatacactagaaatatgacctactccgccggacacaatctcctgaaggcccacgcactggcttggcacgtgtacaacgagaagttcaggcacgcccagaatggaaagattagcatcgccctgcaggccgactggatcgagcccgcctgtcccttcagccagaaagacaaagaggtggctgagcgcgtgctggagtttgatattggctggcttgctgagccaatattcggcagtggagactacccctgggtgatgagagattggcttaaccagagaaacaactttctcctgccctacttcaccgaggacgaaaagaaactgatccagggtaccttcgatttccttgctctgagccactatactaccatcctggtcgacagcgagaaggaggaccccatcaaatataacgactacctggaggtgcaagagatgactgacatcacatggctgaatagccctagccaggtcgccgtggtgccttggggcctgcgcaaggtgctcaactggctgaagttcaagtatggcgacctgcccatgtacatcatcagcaacggcattgatgacggactgcacgccgaggatgatcaactcagagtatactatatgcagaactatatcaacgaggcattgaaggcccacatcctggacggcatcaacctgtgtgggtactttgcatactccttcaacgacagaaccgctccccgctttggtctgtataggtacgctgccgaccagttcgagcccaaggccagcatgaagcactaccgcaagattatcgatagcaatggcttccctggccccgagacccttgagcgcttttgccccgaggagttcaccgtgtgtaccgaatgttccttcttccacacacgcaagtcatga

SEQ ID NO: 23 - RNA, 2946 nt, synthetic construct
  source 1..2946: mol_type = other RNA
atgcccgctagcgccccaccgagaagaccgcggccgccaccgccatcgctgtcgctgctgctggtgctgctgggactgggcggaagaagactgcgtgcggagcctggcgatggcgctcagacttgggctcgcttcagcagacccccagcccccgaagcagccggattgttccagggaaccttccccgatggtttcctgtgggccgtaggtagcgccgcctaccagactgagggcggatggcagcagcacggcaagggcgcaagcatctgggacaccttcacccaccaccccctggccccccctggcgactcccgcaatgctagtctccccctgggcgcccctagcccccttcagcccgccactggcgacgtggcctcagacagctacaacaatgtgttccgggacacagaagctctgagggagcttggcgtgacccattataggtttagcatctcatgggcccgcgtgctgccaaatggcagcgccggcgtgcctaaccgcgaaggacttcgctactatcgcagactgctggagaggctgcgggaactgggggtgcaacctgtggtgacattgtaccactgggatctgcctcagcgcttgcaagacgcttacggtggatgggccaaccgcgctctggccgaccatttccgggactacgcagagctttgcttccgccacttcgggggtcaagtgaaatattggattacaatcgataacccctacgtggttgcatggcatggctacgccacagggcgccttgctcccggcatcagaggaagccccaggctgggttatcttgtggcacacaacctcctgctggcacacgcaaaagtgtggcacttgtataacacaagtttccgccccacccagggtggacaggtgtcaatagcactgtcttcacactggattaatcctcggaggatgacagatcactccatcaaggaatgccagaagagcctggacttcgtcctgggctggtttgctaagcccgtgtttatcgacggggactaccccgagagcatgaagaataatctgagcagcatattgccagattttaccgagtccgagaagaaatttatcaaagggaccgctgactttttcgctctgtgtttcggccccactctgagctttcaattgctggatccacacatgaagtttagacaactggaaagtcccaatctgcggcagttgctgagctggattgatctggaattcaaccatccccagatttttattgttgagaatgggtggtttgttagtggcactacaaagagggatgacgccaagtacatgtactatctgaagaaattcatcatggagaccctgaaggccataaagctcgacggagttgacgtgatcggttataccgcatggagcctgatggacgggttcgagtggcaccgcgggtacagcatcaggagaggcttgttctacgtcgacttcttgtcacaggacaaaatgttgttgcctaagtcaagtgccttgttttaccagaaactgattgaaaaaaacggctttcctcctttgcccgagaaccaacctctggagggaacctttccctgcgattttgcttggggcgtggtggacaactacatccaggtggacacaaccctgtctcagttcaccgatttgaatgtgtatctctgggatgtccaccactccaagcgcctgatcaaggtggatggcgtcgtgaccaagaaaagaaagagctactgcgtggactttgccgccattcagccccagattgccctgctccaggagatgcacgtcacacactttaggttctccctggactgggccctgatactgcccctgggtaaccagtcacaagtgaaccataccattttgcagtactaccgctgtatggcttcagagctggtacgcgtgaacatcacccccgtagttgccctctggcagcccatggcccccaatcagggcctgcctcgcctgctcgcccggcagggagcctgggaaaacccatacaccgcacttgccttcgctgagtacgccaggttgtgcttccaggagctgggacatcacgtgaagctttggattaccatgaacgagccatacaccaggaacatgacatactccgccggacataatctgctgaaggctcacgcactggcctggcacgtgtacaacgagaagtttcggcatgcccagaatggaaagatcagcatcgctctgcaggcagactggatcgagcctgcctgtcctttcagtcagaaagataaagaggtggccgagcgggtgctggaattcgatatcggatggctggctgaaccaatcttcggcagtggggactacccctgggtgatgagagattggctgaaccagcgcaacaattttctgctgccctactttaccgaggacgaaaagaagcttatccagggtaccttcgatttccttgccctgtcccactatactaccatacttgtcgactctgagaaagaggaccccatcaaatacaatgactacctggaggtgcaagaaatgacagacataacctggctgaatagccctagtcaggtcgctgtggtgccttggggcctccgcaaagtgttgaactggctgaagtttaagtatggcgacctgcccatgtacatcattagcaacgggattgatgacggactgcacgctgaggatgatcaactgagagtatactatatgcagaattacatcaatgaggctttgaaggcccacatcctggatggaattaacctgtgcgggtactttgcatactccttcaacgatagaaccgctccccgctttggtctgtataggtacgctgccgatcagttcgagcccaaagccagcatgaagcactaccgcaagatcatcgatagcaacggcttccctgggcccgagactctcgagaggttttgccccgaggagttcaccgtgtgtaccgaatgcagttttttccacacaaggaaatcatga

SEQ ID NO: 24 - RNA, 2946 nt, synthetic construct
  source 1..2946: mol_type = other RNA
atgcccgctagcgccccaccgagaagaccgcggccgccaccgccatcgctgtcgctgctgctggtgctgctgggactgggcggaagaagactgcgtgcggagcctggagacggcgctcagacatgggcccggttcagccggccaccagcccccgaagctgctggattgttccagggaacctttcctgacgggttcctgtgggcagtaggctctgctgcctatcagactgagggtggatggcagcagcacggtaaaggcgcaagcatttgggatacattcacccaccacccactggcacccccaggcgacagccgcaacgcttctcttccactgggagcccccagtcctcttcagcccgccacaggcgacgttgcatcagatagctataacaatgtgttccgggacaccgaagctctgagggagctcggcgtgacacactatcggttcagcatcagttgggccagggtgctgccaaacggcagtgctggtgtgcccaaccgcgaaggtctcagatactatcgccgccttctggagaggctgagagaactgggcgtgcagccagtggtgactctgtatcactgggatctgccacagagactgcaagatgcttatggtggttgggccaaccgcgccctggcagatcatttccgggactatgcagaactgtgcttccggcactttggaggacaggttaaatattggattactatcgacaacccctatgttgtggcctggcacgggtacgccactgggcgcctcgctcccggcataaggggctcccccaggctgggttaccttgtcgcccacaacctcttgctcgctcacgccaaggtctggcatctgtacaatacttctttccgccccacccagggtggtcaggtgtcaatcgcactgagcagccactggattaaccccaggcgcatgaccgatcattctattaaggagtgccagaagagccttgatttcgttctgggctggtttgctaaaccagtctttattgacggtgactaccctgagagcatgaaaaataatctgtccagcatcttgccagattttaccgagagcgaaaagaaatttatcaagggtaccgctgattttttcgctttgtgtttcggccccacattgagcttccagctgctggacccacacatgaagtttcgccagctggagtcacccaacttgcggcagctgctgtcatggatcgacctggaatttaatcacccccagatctttattgttgagaatgggtggtttgtttctggcactactaagagggatgacgcaaagtatatgtattatctgaagaagtttattatggagaccctgaaagcaatcaagctcgatggagtggatgtgatcggttataccgcttggagccttatggatggatttgagtggcacagggggtattcaataaggagaggcttgttctacgtggactttctgtcacaggataaaatgttgctgcccaaatcaagcgcccttttttaccagaaattgatagaaaagaacggcttccctcctctcccagagaaccagccactggagggaacatttccttgcgatttcgcatggggagtggtggataactacatacaggtggacaccactctgtctcagtttaccgatctcaatgtgtatctgtgggacgttcaccattccaagcgcctcattaaagtggatggcgttgtcactaagaaaagaaagagctactgtgtggactttgctgccattcagccacagatcgctctgctccaggagatgcacgtgacccacttccggttctccctggactgggccttgatactgcccttgggcaaccagagtcaggtcaatcataccatcctgcagtactatcgctgtatggcctcagagctggttcgcgtgaacataacccccgtggtggcactgtggcagcccatggcaccaaatcagggcctgcccagactgctggctagacagggcgcctgggaaaatccctacactgcactggcatttgctgagtacgccaggttgtgttttcaggagctgggacatcacgttaagctttggattaccatgaacgaaccatatactagaaacatgacctattccgccggacacaatctgctgaaagcccacgccctggcatggcatgtgtataacgagaaattcaggcacgcccagaacggaaagatcagcattgccctgcaagcagactggattgagccagcctgtcctttctcacaaaaagacaaagaggtggccgaacgggtcctggagttcgacatcggctggctcgctgaaccaatctttggcagtggcgactacccttgggttatgagggactggctcaaccagagaaacaactttcttcttccctattttacagaggatgagaagaaactgattcagggcaccttcgattttcttgctctcagccattatactactatccttgtggatagtgaaaaagaggacccaattaagtacaatgactatctcgaagtgcaagagatgaccgacatcacctggctgaatagcccatcccaggtcgcagtggtgccttggggcctgcggaaggtgctgaactggctgaagtttaagtatggcgacctgcccatgtacattattagcaacgggatagacgatggactgcacgcagaagatgatcagctgcgcgtgtattatatgcaaaattatatcaacgaagccttgaaggcccacatcctggatggaatcaacctgtgtggctattttgcatactcattcaacgaccgcaccgcaccacggtttggtctgtataggtacgctgccgaccagtttgagccaaaagccagtatgaagcactaccggaaaatcatcgattctaatggcttccctggccctgagaccctggagagattttgccccgaggaattcaccgtgtgtacagaatgttcattttttcacacccggaaaagttga

SEQ ID NO: 25 - RNA, 2946 nt, synthetic construct
  source 1..2946: mol_type = other RNA
atgcccgctagcgccccaccgagaagaccgcggccgccaccgccatcgctgtcgctgctgctggtgctgctgggactgggcggaagaagactgcgtgcggaacccggcgatggagcccaaacatgggccagattcagcagacctcccgctccagaagctgctggtctgtttcagggtacgtttcctgacggttttctctgggcagtcggctctgctgcctatcagactgagggaggttggcaacaacatggcaaaggtgctagcatatgggacactttcacgcatcacccactggccccgcctggggatagtcgcaacgcaagtctgccactgggagcaccctctcctctgcaaccggctaccggggatgtggcttccgactcttacaacaacgtgttcagggatactgaagcgcttagggaattgggcgtgacgcattaccgctttagcattagctgggccagagtcttgcctaatggatcagccggtgtgccaaatcgcgaagggctgcgatactataggcggctgttggagaggctccgggaactgggtgttcagcctgtggtgacactctatcactgggacctcccacagagacttcaagacgcgtacggaggctgggcaaatcgggccttggctgatcatttccgggactatgcagagctgtgtttccgtcactttggcggccaggtaaagtattggattaccatagataacccttatgtcgtagcttggcatggctatgcgacagggagacttgctcctgggattcgcggatctcccaggctgggatatctggtcgctcacaatctgttgctggcccatgccaaagtatggcacctgtacaacacctcattccggccgacccaaggcggccaggtgtcaattgcccttagcagccactggattaatccccgccgaatgaccgatcacagcattaaggagtgccagaaatccctggactttgttttggggtggtttgcgaaaccggtgttcatcgatggggactaccccgagtccatgaagaacaatctgagttctatcctgccagacttcacagaatccgagaagaagttcatcaaggggactgccgacttcttcgcactgtgctttggccccacactctcctttcagctgctcgatcctcacatgaaatttcgccagcttgagagcccaaatctccgtcagctgctttcatggatagacctggagttcaaccatccccagatctttatcgtcgaaaacggttggttcgtgagtggaaccacaaagagggacgatgccaaatacatgtattacctcaagaagttcattatggagactctgaaggccatcaaactcgacggagttgacgtgatcggctatactgcatggtccttgatggatggattcgaatggcatagagggtacagcatccgaagaggcctgttttacgtggactttctgagccaggacaagatgctgctccccaaaagctcagccctcttctaccagaaactgatcgagaagaacggctttccacccttgcccgagaatcagcctctggagggcacattcccctgtgactttgcctggggcgttgtggacaattacattcaggtggataccaccctgtctcagttcaccgatctgaacgtgtacctctgggatgttcaccacagtaaacgtctgatcaaggtcgatggggtggttacaaagaaacgcaagagttattgcgtcgattttgcagccatccagccgcagattgccctgctccaagagatgcacgtgacacacttcagattttccctggattgggccctgattctccctctgggaaaccagagccaggtaaaccacaccattctgcagtactaccgttgcatggcaagtgaactggtgagagtgaacattactccagtggtagctttgtggcagcctatggcccctaatcaaggactgccaagactgctcgcccgtcaaggcgcatgggaaaatccctatacggctcttgcctttgctgagtatgcaaggctgtgctttcaggaactgggacatcacgtgaagttgtggattaccatgaatgagccttatactcgaaacatgacctattcagctggccataatctcctcaaagcccatgcattggcttggcacgtctacaacgagaagtttcgccatgcccaaaatggcaagatcagcattgccctccaagcagactggatcgagccagcatgtcccttttctcagaaagacaaggaagtcgccgaacgggtgctggagtttgacatcggatggctggctgagcccatatttgggagtggcgattacccctgggtgatgagggactggttgaaccagaggaacaactttcttctcccgtatttcacagaggacgagaagaagctgatccagggtacatttgacttcctggctctgtcccattacaccaccattctggttgattctgagaaggaggatcccatcaagtacaatgactacctggaagtacaggagatgacggacattacctggctgaattccccatcacaggttgctgtggttccatggggtttgcgcaaagtgctgaactggctcaagttcaaatatggggatctcccgatgtatattatctctaatggcatagacgatgggcttcatgcagaagatgatcagctgagagtctactatatgcagaactacatcaacgaagcgcttaaagcgcacatattggacggaattaatctgtgtgggtacttcgcctatagcttcaatgatcggactgctccccggtttggcctgtatcgctatgccgcggaccagttcgagcctaaagcgagcatgaagcactacaggaaaatcatcgactcaaacggcttcccaggtcctgaaactcttgaacggttttgtcccgaggaattcaccgtctgcactgagtgtagcttcttccacacacgaaaatcctga

SEQ ID NO: 26 - RNA, 2946 nt, synthetic construct
  source 1..2946: mol_type = other RNA
atgcccgctagcgccccaccgagaagaccgcggccgccaccgccatcgctgtcgctgctgctggtgctgctgggactgggcggaagaagactgcgtgcggagcccggcgatggggcccaaacctgggctcggttcagtagaccgcctgcacctgaagctgcagggttgttccagggcacttttccggatgggtttctctgggcggtagggtccgcggcatatcagaccgagggggggtggcaacaacacgggaagggtgcgtcaatatgggacacttttactcatcacccacttgcgcctcccggagattcaaggaatgcctctctgcctctgggagcacccagtcctctccaacccgcaactggcgatgtcgcatcagacagttacaacaacgtttttagggacacagaagcgctccgagaactgggggttactcattatcggttttccatttcatgggcccgagtactcccaaatgggtccgctggagtaccgaaccgcgagggcctccgctattatagaagactcctcgagcgcctgcgcgaactcggtgttcaaccggttgtcaccctgtaccattgggatctcccgcaacgcctgcaagatgcttacgggggctgggcaaaccgcgcactggcggatcattttcgagattacgccgagctgtgcttccggcattttggtgggcaagtcaagtattggatcaccattgacaacccatatgtcgttgcatggcatggatatgcaaccgggaggcttgcaccggggattagggggagccctagacttggatacctggtcgcccataatctgttgctcgctcatgcgaaggtctggcatctgtataacactagcttccggccgacgcaagggggccaagtatccattgcactgtcttcccactggattaatcccagacgcatgaccgatcacagcataaaggagtgtcaaaagtccctggattttgtcctgggctggtttgcaaagcccgtcttcatagacggcgactaccctgagagcatgaagaataacctgtcttctattcttccggatttcacggagtcagaaaaaaagtttatcaagggcaccgccgacttcttcgcactgtgtttcggaccgacattgtcctttcagcttttggaccctcatatgaaattcaggcagctcgagtcccccaatctgcgacagctgttgtcatggattgatttggaatttaaccacccacaaatttttattgtcgaaaatggttggtttgttagtgggactaccaaacgcgacgatgcgaagtacatgtactatttgaagaagtttataatggagacccttaaagccatcaaattggatggcgtggatgtgataggttatactgcatggagcttgatggacggcttcgagtggcatcgagggtacagcataaggaggggtcttttctacgttgatttcttgtctcaggataagatgcttctgccaaaaagttcagcgcttttttatcagaaattgatagaaaagaatggttttccgccgcttccagaaaatcagcccctcgaaggtacgtttccgtgcgactttgcctggggcgtggtcgacaactacatacaggtagacactactttgtcccaattcactgatctcaatgtgtatctctgggatgttcatcacagcaagcgactgataaaggtagatggggtcgttactaaaaagaggaagtcatactgcgtcgattttgcagccatccagcctcagatagcgttgctccaggagatgcacgtgacacattttcggttttcactggactgggcccttattctgccgctcgggaaccaatctcaagttaatcatactattctgcaatattacaggtgcatggcgagcgagcttgttcgagtaaatattacgcctgtggttgcactctggcagccgatggcgcctaatcaggggcttccgagacttcttgctcgacaaggtgcttgggagaacccatatacagcattggcctttgcagaatacgcgcgcttgtgtttccaagagctgggccatcatgtgaaactttggataaccatgaatgagccttatacacggaacatgacatactcagcagggcacaacttgctgaaggctcatgctcttgcatggcatgtttataatgaaaaatttcgacacgcacaaaacgggaaaatcagcattgctctgcaggctgattggatagaacccgcatgtccattttcacaaaaagacaaggaagtagcggagcgcgtacttgagttcgacataggctggcttgccgagcccatatttggttccggtgattatccgtgggtaatgcgggattggcttaatcaacgcaacaacttcctcctgccttactttacagaggacgagaaaaaactcattcagggcacctttgatttcctcgctcttagccattatacaactatactcgttgacagtgaaaaggaagaccctatcaagtacaacgattatcttgaagtccaggaaatgacagatataacctggcttaacagcccgtcccaggtagctgttgttccttgggggttgcggaaagttttgaattggctgaaattcaagtatggggatcttcccatgtatattatttcaaacggcatcgatgatggtttgcatgccgaagatgaccaacttagggtatattacatgcaaaactacatcaacgaggcgctcaaggcccatatccttgacggtatcaacttgtgcggttattttgcctattcctttaatgatagaacagcccctaggttcggtttgtaccgctacgcagcggaccaatttgagccgaaagcgtcaatgaaacactataggaagataatagatagcaatggatttcctgggcccgagactctcgagaggttctgtccagaggaattcacagtctgcacagaatgtagcttttttcatacgagaaagtcctga

SEQ ID NO: 27 - RNA, 2946 nt, synthetic construct
  source 1..2946: mol_type = other RNA
atgcccgctagcgccccaccgagaagaccgcggccgccaccgccatcgctgtcgctgctgctggtgctgctgggactgggcggaagaagactgcgtgcggaaccgggggatggagctcagacttgggctaggttctctagacctccagctcccgaagctgcaggactgtttcagggaactttccccgatgggtttctgtgggccgtgggatctgctgcctaccaaaccgagggcggatggcaacagcatggaaaaggtgcatccatttgggataccttcacccaccatcctctggcaccccccggagattcaagaaatgcttctctccctctcggtgctccatcaccactgcagcctgctacaggagatgttgccagtgattcatacaacaatgtgtttagggacaccgaagctttgcgagagctcggggtcactcattaccgcttttctatttcatgggcccgcgtacttccaaatggatctgcgggagtcccaaatagagagggcttgagatattaccgaaggttgctggaacgcctgagggaacttggagtgcaacccgtagtgacattgtaccactgggatctcccccagaggcttcaggatgcttacggtggttgggctaacagagctctcgcagaccacttcagagattatgcagaactgtgctttcgacatttcggcggccaggtaaaatactggatcaccatagacaatccctatgtggttgcgtggcatggttatgccacaggaagactggctcccggtatccgggggagtcctagacttggctacctcgtggcccacaatctgctgttggcgcacgctaaggtgtggcatctgtataatactagctttagaccgacccagggaggtcaagtgagcatcgccctgtcctctcactggataaatccccgcagaatgaccgaccactccattaaggagtgtcaaaagtctctcgacttcgtgctcggatggtttgctaagccggttttcattgatggagactaccccgagagcatgaaaaacaacttgagctccattctgcctgactttacagaaagcgaaaaaaaatttatcaagggtactgccgactttttcgcactctgctttggccccactcttagctttcagttgctcgatccacacatgaagttccgccaactggagagtcctaatctgcgccaactcctttcttggattgacttggagttcaatcacccgcagatcttcatcgtggaaaacggctggttcgtgtcaggaaccacgaagcgcgacgatgccaagtacatgtactacctcaaaaagttcatcatggaaactctcaaagcaattaaactggacggcgtcgacgtgatcggctataccgcgtggtctctgatggacggtttcgagtggcataggggctattccataaggcgagggttgttttacgttgattttctcagccaagataaaatgctgctgcccaagtcttcagccttgttttatcagaaattgattgagaagaatggcttcccgccactccccgagaatcaacccctcgaggggacatttccatgtgacttcgcctggggggtagtcgataattacatccaagtggatacaaccctcagccagtttaccgacctgaacgtttacttgtgggacgtgcaccacagtaagagactgattaaagtggatggagtggttactaaaaagcggaagagttattgtgtagattttgccgcaatccagccacaaatcgccctgctgcaggagatgcacgtgacccatttcagatttagtctcgactgggctctgattttgcccttgggcaatcagagccaggtgaatcatacaatcctccagtactatcggtgtatggccagtgaattggtccgagtcaacatcaccccagtggtggcactctggcagccaatggctcctaaccaagggctgccaagactgctggcaaggcagggtgcctgggagaatccttacactgctctggcctttgccgagtacgctcgcctttgttttcaggagctcgggcatcatgtgaaactgtggattacaatgaatgaaccatatactcgcaacatgacctattccgcaggtcacaatctcctcaaggctcatgcactcgcatggcacgtctacaatgaaaaattccgacacgcccagaatgggaagattagtatcgccctgcaggctgattggatcgagcccgcatgtccattttcacaaaaggacaaagaggtagccgagagagtgctggagttcgatatcggctggcttgccgaacctattttcggctctggcgattacccctgggtgatgagggattggttgaaccagaggaacaatttcctcctgccgtattttaccgaggacgaaaagaagttgatccaaggcacattcgatttcctcgccctttctcactacacaaccatacttgtggatagcgagaaggaggacccaattaaatataatgactatctggaagttcaggagatgactgatatcacatggctgaattcccccagccaagtagcagtcgtgccctggggtctgagaaaggtgcttaattggttgaagtttaagtacggtgatctgcctatgtatataatttctaacggcatagatgatgggctgcacgctgaggacgatcaactgcgagtgtactacatgcagaattatatcaacgaagccttgaaagcccacattctggacggcatcaatctttgtggctacttcgcttattcattcaatgatagaacagccccccgctttggattgtatcggtatgccgccgaccaattcgagccaaaggcttctatgaagcactaccggaagattatcgactccaacgggtttccagggccagagacactggaaaggttttgcccagaggagttcaccgtgtgtacagagtgcagctttttccacacccggaaatcatga

SEQ ID NO: 28 - RNA, 2946 nt, synthetic construct
  source 1..2946: mol_type = other RNA
atgcccgctagcgccccaccgagaagaccgcggccgccaccgccatcgctgtcgctgctgctggtgctgctgggactgggcggaagaagactgcgtgcggaaccaggagatggtgcccaaacttgggctaggttctctcgtccacccgcacctgaagctgctgggctgtttcaaggtacttttcctgatggatttctttgggctgtcgggtccgctgcttatcaaactgaaggtggatggcaacaacatgggaaaggcgcttcaatttgggacacctttacacatcatcctctcgccccacctggtgatagtcgcaatgcgagcttacctctcggagcaccatctcccttgcaaccagcaacaggcgatgtggcttcagattcctataataatgtgtttagagatactgaagctctcagagaattgggagtgacccattatagattttctatttcttgggcccgggtcctgcctaacgggtccgccggggttcctaatcgagaaggtttgcggtattatagaaggcttctcgaaaggttgcgagaacttggagtacaacctgtcgtgactttgtatcattgggatcttccgcaaagacttcaagatgcatatggtggatgggcaaatcgtgcactcgctgatcattttcgggactatgccgaactttgttttaggcattttggcggccaagttaaatattggattacaatagataatccttatgtagttgcatggcatggttatgcaacaggccggttggcaccagggattcgaggttcaccacgacttggatatttagtcgcccataatcttcttttggcccacgcgaaggtatggcacttatataacacctcttttaggccgacgcaaggtggacaagtctctatcgcattgtcctcacattggattaaccccaggcgtatgacagatcattctattaaggaatgccagaagagtctcgatttcgtgttaggctggttcgcaaagccagtcttcatcgacggagattacccggaatcaatgaagaacaatctgagcagtatccttcccgacttcaccgagagtgaaaagaaatttattaagggcaccgcagatttcttcgccctgtgtttcggcccgactctctccttccagctgctcgatccacatatgaaatttcggcagctcgagtcacctaatttaagacagctcctgagttggatcgatctggagttcaatcacccacagatcttcatcgttgagaacgggtggttcgtgtctggcacgactaaacgcgacgacgctaagtacatgtactatctgaagaaatttataatggagacacttaaggctataaaattggacggcgtagacgtgattggttacactgcttggagcctgatggacggctttgaatggcatcgtgggtattcaatacggcggggcttattttacgtggatttcttgtctcaagataaaatgctgctgcccaaaagcagtgcacttttctatcagaaactcatcgaaaagaacggatttccacccttgccagagaaccaacctctggaaggaaccttcccatgcgatttcgcgtggggtgtggtggataattatatccaggtggacactaccttaagtcaattcacagatctcaacgtgtatttatgggacgtgcatcatagcaagagactgatcaaggtcgacggtgtggttactaagaagcgcaagagctattgcgtcgatttcgcagcaattcaaccacaaattgccctgctgcaagagatgcatgtgacccacttcagatttagtctcgattgggcattgatcctgcccctcggaaatcaatcacaagtaaatcatactatactccaatattacaggtgtatggcttccgaactggttcgagtaaatattacacctgtcgttgctttgtggcaaccgatggcacctaatcaggggcttccaaggctgctcgcaagacaaggagcgtgggaaaatccatatacagcgttagctttcgctgaatacgctaggctctgtttccaggaattgggtcaccatgtgaaattgtggatcactatgaacgaaccttacactcggaacatgacctattctgcaggacataatctcctcaaagctcacgcattagcctggcacgtttataacgagaaattccgacacgcccaaaacggtaagatttctattgcgcttcaagccgactggattgagcccgcttgtccctttagccagaaagataaggaagtagcagaacgagtactggagttcgatataggatggctcgcggaaccgatatttggatccggcgactacccgtgggtcatgcgagattggctcaatcagcgcaataacttcctgctcccatactttacagaggacgagaagaaactcattcaaggcacgttcgatttccttgccctgtcccactacacgacgattctcgtggattccgagaaagaggaccctatcaagtataacgactatttggaagtccaggagatgactgatataacttggctgaattcaccttcccaagtcgccgttgtcccgtggggtctgagaaaggtacttaattggttgaaatttaaatatggcgatcttcctatgtatatcattagcaacgggattgacgatggcttgcacgcagaagatgatcaattgcgtgtctactacatgcaaaactatatcaatgaggccctgaaggctcatatcctcgacggcattaacttgtgtgggtatttcgcatactcattcaatgatagaaccgcacctcgcttcgggctttaccgctacgccgctgaccaattcgaacctaaagcctcaatgaagcactatagaaagatcatcgattccaacgggtttcccgggcctgagacacttgagaggttctgccccgaggagtttacggtctgcacagaatgtagcttcttccatacacggaaatcctga

SEQ ID NO: 29 - RNA, 3249 nt, synthetic construct
  source 1..3249: mol_type = other RNA
gggagacataaaccctggcgcgctcgcggcccggcactcttctggtccccacagactcagagagaacccaccatgcccgctagcgccccaccgagaagaccgcggccgccaccgccatcgctgtcgctgctgctggtgctgctgggactgggcggaagaagactgcgtgcggagcctggcgacggggcccagacctgggccagattcagcagaccccccgcacccgaggccgccggcctgttccagggcaccttccccgacggatttctgtgggccgtgggaagcgctgcctaccagaccgagggcggctggcaacagcacggcaagggcgccagcatctgggacaccttcacccaccatcctctggctcctcccggagacagcagaaacgccagcctgcctctgggagcccccagccccctgcagcccgccactggagacgtggccagcgactcctacaacaacgtgttccgcgacaccgaggccctgcgcgagctgggcgtgacccactaccgctttagcatcagctgggccagagtgctgcccaacggcagcgccggcgtgcccaaccgggaaggcctgagatactatcgccgcctgctggagaggctgagagagttgggcgtgcagcccgtggtgaccctgtaccactgggacctgccccagcgcctgcaggacgcctacggcggctgggccaacagggcactcgccgaccacttccgcgactacgccgagctgtgcttccgccacttcggcgggcaggtgaagtactggatcaccatcgacaacccctacgtggtggcctggcacggctacgctacaggaaggctggcccccgggatccgcggcagccccaggctgggctacctggtggcccacaacctgctgctggcacacgccaaagtgtggcacctgtataacaccagctttcgccccacccagggtggacaggtgagcattgccctgagttctcattggatcaaccccaggcgcatgaccgatcacagcatcaaggaatgccagaagagcctggacttcgtgctgggctggttcgccaagcccgtgtttatcgacggcgactaccccgagtctatgaagaacaacctcagcagcatcctgcctgacttcaccgagagcgagaagaagttcatcaagggcaccgccgacttcttcgccctgtgcttcggccccaccctgagcttccagctgctggatccccatatgaagttcagacaactcgagagtcctaacctgcgccagctgctgagctggatcgacctggaattcaaccacccacagatcttcatcgtggagaacggctggtttgtgagcggcaccactaagcgcgacgacgcaaagtatatgtattatctgaagaaattcatcatggaaaccctgaaggccatcaagctggacggcgtggacgtgatcggatacaccgcatggagcctgatggacggcttcgagtggcaccgcggttacagcatccgccggggcctgttctacgttgacttcctgagccaggacaagatgttgctgcccaagagctccgccctgttctaccagaagttgatcgagaagaacggcttcccaccactccccgagaaccagcccctggagggcaccttcccctgcgatttcgcctggggcgtggtggacaactacatccaggtggacaccaccctgagtcagttcactgacctgaacgtgtacctttgggacgtgcaccacagcaagcgcctgataaaggtcgacggcgtggtgaccaagaagcgcaaaagctactgcgtggactttgccgccatccagccccagatcgccctgctgcaggagatgcacgtgactcacttccgcttcagcctcgactgggccctgattctgcccctgggcaaccagtcacaagtgaaccacaccattctgcagtactaccgctgtatggccagcgagctggtacgcgtgaacatcacccccgttgtggccctttggcagcccatggcccccaaccagggcctgcctcgcctgctggcccgccagggagcctgggagaatccctacaccgcactggccttcgctgaatacgcccgcctgtgcttccaggagctggggcaccacgtgaaactctggatcaccatgaacgagccctacaccagaaacatgacctacagcgccggacacaatctgctgaaggcccacgctctggcctggcacgtgtacaacgagaagtttcgccacgcccagaacggcaagatcagcatcgccctgcaggccgattggatcgagcccgcctgccccttcagccagaaggacaaggaggtggctgagcgggtgctggagttcgacatcgggtggctggctgagcctatcttcggcagcggagactacccctgggtgatgcgcgattggcttaaccagaggaacaatttcctgctgccctacttcaccgaggacgagaagaagctgatccagggcacctttgacttcctggctttgagccactataccactatcctggtggacagcgagaaggaggaccccatcaagtacaacgactacttggaggtgcaggagatgaccgacatcacctggctgaacagccctagccaggtggctgtggtgccttggggcctgcgcaaggtgctgaactggctgaagttcaagtacggcgacctgcccatgtatatcatcagcaacggcatcgacgacggcctgcacgccgaggacgaccagctgagagtgtactacatgcagaactacatcaacgaggccctcaaggcccacatcctggacggcatcaacctgtgtggctactttgcctacagcttcaacgacagaaccgccccccgcttcggcctgtacaggtacgccgccgaccagttcgaacccaaggccagcatgaagcactaccgcaaaatcatcgacagcaacggattccctggacccgagacactggagcgcttctgcccagaggagttcaccgtgtgcaccgagtgcagtttcttccacacccgcaagagctgagctggagcctcggtggccatgcttcttgccccttgggcctccccccagcccctcctccccttcctgcacccgtacccccgtggtctttgaataaagtctgagtgggcggcaaaaaaaaaaaaaaaaaaaaaaaaaaaaaaaaaaaaaaaaaaaaaaaaaaaaaaaaaaaaaaaaaaaaaaaaaaaaaaaaaaaaaaaaaaaaaaaaaaaaaaaaaaaaaaaaaaaaaaaaa

SEQ ID NO: 30 - RNA, 3249 nt, synthetic construct
  source 1..3249: mol_type = other RNA
gggagacataaaccctggcgcgctcgcggcccggcactcttctggtccccacagactcagagagaacccaccatgcccgctagcgccccaccgagaagaccgcggccgccaccgccatcgctgtcgctgctgctggtgctgctgggactgggcggaagaagactgcgtgcggagcctggagatggagcccaaacatgggccagattcagcagacctcccgctcctgaagccgccggcttgtttcagggaacctttcctgacggtttcctgtgggctgtgggcagcgccgcctatcagaccgagggcggctggcaacagcacggaaaaggagccagcatctgggataccttcacccaccaccccctggccccccccggcgattcccgcaatgccagcctccctctgggagcccctagccccctgcaacctgccacaggagacgtggcctcagacagctataacaacgtgttccgcgacaccgaggcactgcgcgagctgggcgtgacccattaccgctttagcatcagctgggccagagtgctgcccaatggctctgccggcgtgcccaaccgggagggcctgaggtactaccgccgcctgctggagaggctgcgggagctgggcgtgcagcccgtggtaaccctgtaccactgggacctgccccagcgcctgcaggacgcttacggcggctgggccaaccgcgctctcgcagaccacttccgcgactacgccgagctgtgctttcgccactttggcggccaggtgaagtattggatcaccatcgataacccttacgtggtggcctggcacggatacgctacaggccgcctggcccccggcatccgcggcagccccagactgggctacctggtggcccacaacctgctgctggcccacgccaaggtgtggcacctgtacaacaccagcttccgccccacccagggtggacaggtctctattgccctgagctctcactggattaaccccaggaggatgaccgatcacagcatcaaggaatgccagaagagcctggacttcgttctgggctggttcgccaagcccgtgtttatcgacggcgactaccccgagagcatgaagaacaacctgtctagcatcctgcccgacttcaccgagagcgaaaaaaaattcatcaagggcaccgccgatttcttcgccctgtgtttcggcccaaccctgagcttccaactgctggatccccacatgaagttcagacaactcgagagtcccaacctgcgccagctgctgagctggatcgatctggaattcaaccacccccagatattcatagtggagaacggctggtttgtaagcggcactactaagcgcgatgatgcaaagtacatgtactatctgaagaagttcatcatggaaaccctgaaggccatcaagctggatggcgtggacgtgatcggatacaccgcatggagcctgatggacggcttcgagtggcaccgcggttactcaatccgcagggggttgttctacgtcgacttcctgagtcaggacaagatgttgctgccaaagagtagcgcccttttctaccagaagttgattgagaagaacggcttcccaccactccccgagaaccagcccctggagggcacctttccctgcgatttcgcttggggcgtggtggataattatattcaggtggacaccaccctgtcacagttcactgacctgaacgtgtacctgtgggacgtgcaccattccaagcgcctgatcaaggtggacggcgtggtgaccaagaagcgcaaatcctactgcgttgactttgccgccattcagccacagatcgccctgctgcaggagatgcacgtcacccacttccgcttcagcctggactgggccctcatcctgccactgggcaaccagtcccaggtgaaccacaccattctgcagtactaccgctgtatggccagcgagctggtacgcgtgaacatcacccccgtggtggccctgtggcagcccatggcccccaaccagggcctgccacgcctgctggccaggcagggggcctgggagaacccctacaccgcactcgctttcgccgaatatgccaggctgtgcttccaggagctggggcaccacgtgaagctctggatcaccatgaacgaaccctacaccagaaacatgacctactctgccggacacaatctgctgaaggcccacgccctggcctggcacgtctacaacgagaagttccgccacgcccaaaatggaaagatctctatagccctgcaggccgattggatcgagcccgcctgccccttctcacagaaggacaaggaggtggccgagcgcgtgctggagttcgacatcggctggctggccgagcccatcttcggcagcggagactacccctgggtgatgcgcgattggcttaaccagcgcaacaactttctgctgccctacttcaccgaggacgagaagaagctgatccagggcaccttcgacttcctggccctgagccactatactaccatcctggtcgacagcgagaaggaggacccaatcaagtacaacgactacctggaggtgcaggagatgaccgacatcacctggctgaacagccctagccaggtcgccgtggtgccttggggcctgcgcaaggtgctgaactggctgaagttcaagtatggcgacctgccaatgtacatcatcagcaacggcattgatgacggcctgcacgccgaggacgatcagctgagagtgtactatatgcagaactacatcaacgaggcactgaaggcccacatcctggacggcatcaacctgtgtggctactttgcatactccttcaacgacagaaccgccccccgcttcggcctgtacaggtacgctgccgatcagttcgagcccaaggccagcatgaagcactacagaaaaatcattgatagcaacgggttcccaggccccgagaccctggagcgcttctgccccgaggagttcaccgtgtgcaccgagtgcagttttttccacacccgcaagagctgagctggagcctcggtggccatgcttcttgccccttgggcctccccccagcccctcctccccttcctgcacccgtacccccgtggtctttgaataaagtctgagtgggcggcaaaaaaaaaaaaaaaaaaaaaaaaaaaaaaaaaaaaaaaaaaaaaaaaaaaaaaaaaaaaaaaaaaaaaaaaaaaaaaaaaaaaaaaaaaaaaaaaaaaaaaaaaaaaaaaaaaaaaaaaa

SEQ ID NO: 31 - RNA, 3249 nt, synthetic construct
  source 1..3249: mol_type = other RNA
gggagacataaaccctggcgcgctcgcggcccggcactcttctggtccccacagactcagagagaacccaccatgcccgctagcgccccaccgagaagaccgcggccgccaccgccatcgctgtcgctgctgctggtgctgctgggactgggcggaagaagactgcgtgcggagcctggcgacggggcccagacctgggccagattcagcagaccccccgcacccgaggccgccggcctgttccagggcaccttccccgacggatttctgtgggccgtgggaagcgctgcctaccagaccgagggcggctggcaacagcacggcaagggcgccagcatctgggacaccttcacccaccatcctctggctcctcccggagacagcagaaacgccagcctgcctctgggagcccccagccccctgcagcccgccactggagacgtggccagcgactcctacaacaacgtgttccgcgacaccgaggccctgcgcgagctgggcgtgacccactaccgctttagcatcagctgggccagagtgctgcccaacggcagcgccggcgtgcccaaccgggaaggcctgagatactatcgccgcctgctggagaggctgagagagttgggcgtgcagcccgtggtgaccctgtaccactgggacctgccccagcgcctgcaggacgcctacggcggctgggccaacagggcactcgccgaccacttccgcgactacgccgagctgtgcttccgccacttcggcgggcaggtgaagtactggatcaccatcgacaacccctacgtggtggcctggcacggctacgctacaggaaggctggcccccgggatccgcggcagccccaggctgggctacctggtggcccacaacctgctgctggcacacgccaaagtgtggcacctgtataacaccagctttcgccccacccagggtggacaggtgagcattgccctgagttctcattggatcaaccccaggcgcatgaccgatcacagcatcaaggaatgccagaagagcctggacttcgtgctgggctggttcgccaagcccgtgtttatcgacggcgactaccccgagtctatgaagaacaacctcagcagcatcctgcctgacgtcaccgagagcgagaagaagttcatcaagggcaccgccgacttcttcgccctgagcttcggccccaccctgagcttccagctgctggatccccatatgaagttcagacaactcgagagtcctaacctgcgccagctgctgagctggatcgacctggaattcaaccacccacagatcttcatcgtggagaacggctggtttgtgagcggcaccactaagcgcgacgacgcaaagtatatgtattatctgaagaaattcatcatggaaaccctgaaggccatcaagctggacggcgtggacgtgatcggatacaccgcatggagcctgatggacggcttcgagtggcaccgcggttacagcatccgccggggcctgttctacgttgacttcctgagccaggacaagatgttgctgcccaagagctccgccctgttctaccagaagttgatcgagaagaacggcttcccaccactccccgagaaccagcccctggagggcaccttcccctgcgatttcgcctggggcgtggtggacaactacatccaggtggacaccaccctgagtcagttcactgacctgaacgtgtacctttgggacgtgcaccacagcaagcgcctgataaaggtcgacggcgtggtgaccaagaagcgcaaaagctactgcgtggactttgccgccatccagccccagatcgccctgctgcaggagatgcacgtgactcacttccgcttcagcctcgactgggccctgattctgcccctgggcaaccagtcacaagtgaaccacaccattctgcagtactaccgctgtatggccagcgagctggtacgcgtgaacatcacccccgttgtggccctttggcagcccatggcccccaaccagggcctgcctcgcctgctggcccgccagggagcctgggagaatccctacaccgcactggccttcgctgaatacgcccgcctgtgcttccaggagctggggcaccacgtgaaactctggatcaccatgaacgagccctacaccagaaacatgacctacagcgccggacacaatctgctgaaggcccacgctctggcctggcacgtgtacaacgagaagtttcgccacgcccagaacggcaagatcagcatcgccctgcaggccgattggatcgagcccgcctgccccttcagccagaaggacaaggaggtggctgagcgggtgctggagttcgacatcgggtggctggctgagcctatcttcggcagcggagactacccctgggtgatgcgcgattggcttaaccagaggaacaatttcctgctgccctacttcaccgaggacgagaagaagctgatccagggcacctttgacttcctggctttgagccactataccactatcctggtggacagcgagaaggaggaccccatcaagtacaacgactacttggaggtgcaggagatgaccgacatcacctggctgaacagccctagccaggtggctgtggtgccttggggcctgcgcaaggtgctgaactggctgaagttcaagtacggcgacctgcccatgtatatcatcagcaacggcatcgacgacggcctgcacgccgaggacgaccagctgagagtgtactacatgcagaactacatcaacgaggccctcaaggcccacatcctggacggcatcaacctgtgtggctactttgcctacagcttcaacgacagaaccgccccccgcttcggcctgtacaggtacgccgccgaccagttcgaacccaaggccagcatgaagcactaccgcaaaatcatcgacagcaacggattccctggacccgagacactggagcgcttctgcccagaggagttcaccgtgtgcaccgagtgcagtttcttccacacccgcaagagctgagctggagcctcggtggccatgcttcttgccccttgggcctccccccagcccctcctccccttcctgcacccgtacccccgtggtctttgaataaagtctgagtgggcggcaaaaaaaaaaaaaaaaaaaaaaaaaaaaaaaaaaaaaaaaaaaaaaaaaaaaaaaaaaaaaaaaaaaaaaaaaaaaaaaaaaaaaaaaaaaaaaaaaaaaaaaaaaaaaaaaaaaaaaaaa

SEQ ID NO: 32 - RNA, 3249 nt, synthetic construct
  source 1..3249: mol_type = other RNA
gggagacataaaccctggcgcgctcgcggcccggcactcttctggtccccacagactcagagagaacccaccatgcccgctagcgccccaccgagaagaccgcggccgccaccgccatcgctgtcgctgctgctggtgctgctgggactgggcggaagaagactgcgtgcggagcctggagatggagcccaaacatgggccagattcagcagacctcccgctcctgaagccgccggcttgtttcagggaacctttcctgacggtttcctgtgggctgtgggcagcgccgcctatcagaccgagggcggctggcaacagcacggaaaaggagccagcatctgggataccttcacccaccaccccctggccccccccggcgattcccgcaatgccagcctccctctgggagcccctagccccctgcaacctgccacaggagacgtggcctcagacagctataacaacgtgttccgcgacaccgaggcactgcgcgagctgggcgtgacccattaccgctttagcatcagctgggccagagtgctgcccaatggctctgccggcgtgcccaaccgggagggcctgaggtactaccgccgcctgctggagaggctgcgggagctgggcgtgcagcccgtggtaaccctgtaccactgggacctgccccagcgcctgcaggacgcttacggcggctgggccaaccgcgctctcgcagaccacttccgcgactacgccgagctgtgctttcgccactttggcggccaggtgaagtattggatcaccatcgataacccttacgtggtggcctggcacggatacgctacaggccgcctggcccccggcatccgcggcagccccagactgggctacctggtggcccacaacctgctgctggcccacgccaaggtgtggcacctgtacaacaccagcttccgccccacccagggtggacaggtctctattgccctgagctctcactggattaaccccaggaggatgaccgatcacagcatcaaggaatgccagaagagcctggacttcgttctgggctggttcgccaagcccgtgtttatcgacggcgactaccccgagagcatgaagaacaacctgtctagcatcctgcccgacgtcaccgagagcgaaaaaaaattcatcaagggcaccgccgatttcttcgccctgagcttcggcccaaccctgagcttccaactgctggatccccacatgaagttcagacaactcgagagtcccaacctgcgccagctgctgagctggatcgatctggaattcaaccacccccagatattcatagtggagaacggctggtttgtaagcggcactactaagcgcgatgatgcaaagtacatgtactatctgaagaagttcatcatggaaaccctgaaggccatcaagctggatggcgtggacgtgatcggatacaccgcatggagcctgatggacggcttcgagtggcaccgcggttactcaatccgcagggggttgttctacgtcgacttcctgagtcaggacaagatgttgctgccaaagagtagcgcccttttctaccagaagttgattgagaagaacggcttcccaccactccccgagaaccagcccctggagggcacctttccctgcgatttcgcttggggcgtggtggataattatattcaggtggacaccaccctgtcacagttcactgacctgaacgtgtacctgtgggacgtgcaccattccaagcgcctgatcaaggtggacggcgtggtgaccaagaagcgcaaatcctactgcgttgactttgccgccattcagccacagatcgccctgctgcaggagatgcacgtcacccacttccgcttcagcctggactgggccctcatcctgccactgggcaaccagtcccaggtgaaccacaccattctgcagtactaccgctgtatggccagcgagctggtacgcgtgaacatcacccccgtggtggccctgtggcagcccatggcccccaaccagggcctgccacgcctgctggccaggcagggggcctgggagaacccctacaccgcactcgctttcgccgaatatgccaggctgtgcttccaggagctggggcaccacgtgaagctctggatcaccatgaacgaaccctacaccagaaacatgacctactctgccggacacaatctgctgaaggcccacgccctggcctggcacgtctacaacgagaagttccgccacgcccaaaatggaaagatctctatagccctgcaggccgattggatcgagcccgcctgccccttctcacagaaggacaaggaggtggccgagcgcgtgctggagttcgacatcggctggctggccgagcccatcttcggcagcggagactacccctgggtgatgcgcgattggcttaaccagcgcaacaactttctgctgccctacttcaccgaggacgagaagaagctgatccagggcaccttcgacttcctggccctgagccactatactaccatcctggtcgacagcgagaaggaggacccaatcaagtacaacgactacctggaggtgcaggagatgaccgacatcacctggctgaacagccctagccaggtcgccgtggtgccttggggcctgcgcaaggtgctgaactggctgaagttcaagtatggcgacctgccaatgtacatcatcagcaacggcattgatgacggcctgcacgccgaggacgatcagctgagagtgtactatatgcagaactacatcaacgaggcactgaaggcccacatcctggacggcatcaacctgtgtggctactttgcatactccttcaacgacagaaccgccccccgcttcggcctgtacaggtacgctgccgatcagttcgagcccaaggccagcatgaagcactacagaaaaatcattgatagcaacgggttcccaggccccgagaccctggagcgcttctgccccgaggagttcaccgtgtgcaccgagtgcagttttttccacacccgcaagagctgagctggagcctcggtggccatgcttcttgccccttgggcctccccccagcccctcctccccttcctgcacccgtacccccgtggtctttgaataaagtctgagtgggcggcaaaaaaaaaaaaaaaaaaaaaaaaaaaaaaaaaaaaaaaaaaaaaaaaaaaaaaaaaaaaaaaaaaaaaaaaaaaaaaaaaaaaaaaaaaaaaaaaaaaaaaaaaaaaaaaaaaaaaaaaa

SEQ ID NO: 33 - RNA, 1482 nt, synthetic construct
  source 1..1482: mol_type = other RNA
ctgttccagggcaccttccccgacggatttctgtgggccgtgggaagcgctgcctaccagaccgagggcggctggcaacagcacggcaagggcgccagcatctgggacaccttcacccaccatcctctggctcctcccggagacagcagaaacgccagcctgcctctgggagcccccagccccctgcagcccgccactggagacgtggccagcgactcctacaacaacgtgttccgcgacaccgaggccctgcgcgagctgggcgtgacccactaccgctttagcatcagctgggccagagtgctgcccaacggcagcgccggcgtgcccaaccgggaaggcctgagatactatcgccgcctgctggagaggctgagagagttgggcgtgcagcccgtggtgaccctgtaccactgggacctgccccagcgcctgcaggacgcctacggcggctgggccaacagggcactcgccgaccacttccgcgactacgccgagctgtgcttccgccacttcggcgggcaggtgaagtactggatcaccatcgacaacccctacgtggtggcctggcacggctacgctacaggaaggctggcccccgggatccgcggcagccccaggctgggctacctggtggcccacaacctgctgctggcacacgccaaagtgtggcacctgtataacaccagctttcgccccacccagggtggacaggtgagcattgccctgagttctcattggatcaaccccaggcgcatgaccgatcacagcatcaaggaatgccagaagagcctggacttcgtgctgggctggttcgccaagcccgtgtttatcgacggcgactaccccgagtctatgaagaacaacctcagcagcatcctgcctgacttcaccgagagcgagaagaagttcatcaagggcaccgccgacttcttcgccctgtgcttcggccccaccctgagcttccagctgctggatccccatatgaagttcagacaactcgagagtcctaacctgcgccagctgctgagctggatcgacctggaattcaaccacccacagatcttcatcgtggagaacggctggtttgtgagcggcaccactaagcgcgacgacgcaaagtatatgtattatctgaagaaattcatcatggaaaccctgaaggccatcaagctggacggcgtggacgtgatcggatacaccgcatggagcctgatggacggcttcgagtggcaccgcggttacagcatccgccggggcctgttctacgttgacttcctgagccaggacaagatgttgctgcccaagagctccgccctgttctaccagaagttgatcgagaagaacggcttcccaccactccccgagaaccagcccctggagggcaccttcccctgcgatttcgcctggggcgtggtggacaactacatccaggtgagccagctgacaaaacctatcagcagcctgacaaagccttaccat

SEQ ID NO: 34 - RNA, 1482 nt, synthetic construct
  source 1..1482: mol_type = other RNA
ttgtttcagggaacctttcctgacggtttcctgtgggctgtgggcagcgccgcctatcagaccgagggcggctggcaacagcacggaaaaggagccagcatctgggataccttcacccaccaccccctggccccccccggcgattcccgcaatgccagcctccctctgggagcccctagccccctgcaacctgccacaggagacgtggcctcagacagctataacaacgtgttccgcgacaccgaggcactgcgcgagctgggcgtgacccattaccgctttagcatcagctgggccagagtgctgcccaatggctctgccggcgtgcccaaccgggagggcctgaggtactaccgccgcctgctggagaggctgcgggagctgggcgtgcagcccgtggtaaccctgtaccactgggacctgccccagcgcctgcaggacgcttacggcggctgggccaaccgcgctctcgcagaccacttccgcgactacgccgagctgtgctttcgccactttggcggccaggtgaagtattggatcaccatcgataacccttacgtggtggcctggcacggatacgctacaggccgcctggcccccggcatccgcggcagccccagactgggctacctggtggcccacaacctgctgctggcccacgccaaggtgtggcacctgtacaacaccagcttccgccccacccagggtggacaggtctctattgccctgagctctcactggattaaccccaggaggatgaccgatcacagcatcaaggaatgccagaagagcctggacttcgttctgggctggttcgccaagcccgtgtttatcgacggcgactaccccgagagcatgaagaacaacctgtctagcatcctgcccgacttcaccgagagcgaaaaaaaattcatcaagggcaccgccgatttcttcgccctgtgtttcggcccaaccctgagcttccaactgctggatccccacatgaagttcagacaactcgagagtcccaacctgcgccagctgctgagctggatcgatctggaattcaaccacccccagatattcatagtggagaacggctggtttgtaagcggcactactaagcgcgatgatgcaaagtacatgtactatctgaagaagttcatcatggaaaccctgaaggccatcaagctggatggcgtggacgtgatcggatacaccgcatggagcctgatggacggcttcgagtggcaccgcggttactcaatccgcagggggttgttctacgtcgacttcctgagtcaggacaagatgttgctgccaaagagtagcgcccttttctaccagaagttgattgagaagaacggcttcccaccactccccgagaaccagcccctggagggcacctttccctgcgatttcgcttggggcgtggtggataattatattcaggtgagccagctgacaaaacctatcagcagcctgacaaagccttaccat

SEQ ID NO: 35 - RNA, 1482 nt, synthetic construct
  source 1..1482: mol_type = other RNA
ctgttccagggcaccttccccgacggatttctgtgggccgtgggaagcgctgcctaccagaccgagggcggctggcaacagcacggcaagggcgccagcatctgggacaccttcacccaccatcctctggctcctcccggagacagcagaaacgccagcctgcctctgggagcccccagccccctgcagcccgccactggagacgtggccagcgactcctacaacaacgtgttccgcgacaccgaggccctgcgcgagctgggcgtgacccactaccgctttagcatcagctgggccagagtgctgcccaacggcagcgccggcgtgcccaaccgggaaggcctgagatactatcgccgcctgctggagaggctgagagagttgggcgtgcagcccgtggtgaccctgtaccactgggacctgccccagcgcctgcaggacgcctacggcggctgggccaacagggcactcgccgaccacttccgcgactacgccgagctgtgcttccgccacttcggcgggcaggtgaagtactggatcaccatcgacaacccctacgtggtggcctggcacggctacgctacaggaaggctggcccccgggatccgcggcagccccaggctgggctacctggtggcccacaacctgctgctggcacacgccaaagtgtggcacctgtataacaccagctttcgccccacccagggtggacaggtgagcattgccctgagttctcattggatcaaccccaggcgcatgaccgatcacagcatcaaggaatgccagaagagcctggacttcgtgctgggctggttcgccaagcccgtgtttatcgacggcgactaccccgagtctatgaagaacaacctcagcagcatcctgcctgacgtcaccgagagcgagaagaagttcatcaagggcaccgccgacttcttcgccctgagcttcggccccaccctgagcttccagctgctggatccccatatgaagttcagacaactcgagagtcctaacctgcgccagctgctgagctggatcgacctggaattcaaccacccacagatcttcatcgtggagaacggctggtttgtgagcggcaccactaagcgcgacgacgcaaagtatatgtattatctgaagaaattcatcatggaaaccctgaaggccatcaagctggacggcgtggacgtgatcggatacaccgcatggagcctgatggacggcttcgagtggcaccgcggttacagcatccgccggggcctgttctacgttgacttcctgagccaggacaagatgttgctgcccaagagctccgccctgttctaccagaagttgatcgagaagaacggcttcccaccactccccgagaaccagcccctggagggcaccttcccctgcgatttcgcctggggcgtggtggacaactacatccaggtgagccagctgacaaaacctatcagcagcctgacaaagccttaccat

SEQ ID NO: 36 - RNA, 1482 nt, synthetic construct
  source 1..1482: mol_type = other RNA
ttgtttcagggaacctttcctgacggtttcctgtgggctgtgggcagcgccgcctatcagaccgagggcggctggcaacagcacggaaaaggagccagcatctgggataccttcacccaccaccccctggccccccccggcgattcccgcaatgccagcctccctctgggagcccctagccccctgcaacctgccacaggagacgtggcctcagacagctataacaacgtgttccgcgacaccgaggcactgcgcgagctgggcgtgacccattaccgctttagcatcagctgggccagagtgctgcccaatggctctgccggcgtgcccaaccgggagggcctgaggtactaccgccgcctgctggagaggctgcgggagctgggcgtgcagcccgtggtaaccctgtaccactgggacctgccccagcgcctgcaggacgcttacggcggctgggccaaccgcgctctcgcagaccacttccgcgactacgccgagctgtgctttcgccactttggcggccaggtgaagtattggatcaccatcgataacccttacgtggtggcctggcacggatacgctacaggccgcctggcccccggcatccgcggcagccccagactgggctacctggtggcccacaacctgctgctggcccacgccaaggtgtggcacctgtacaacaccagcttccgccccacccagggtggacaggtctctattgccctgagctctcactggattaaccccaggaggatgaccgatcacagcatcaaggaatgccagaagagcctggacttcgttctgggctggttcgccaagcccgtgtttatcgacggcgactaccccgagagcatgaagaacaacctgtctagcatcctgcccgacgtcaccgagagcgaaaaaaaattcatcaagggcaccgccgatttcttcgccctgagcttcggcccaaccctgagcttccaactgctggatccccacatgaagttcagacaactcgagagtcccaacctgcgccagctgctgagctggatcgatctggaattcaaccacccccagatattcatagtggagaacggctggtttgtaagcggcactactaagcgcgatgatgcaaagtacatgtactatctgaagaagttcatcatggaaaccctgaaggccatcaagctggatggcgtggacgtgatcggatacaccgcatggagcctgatggacggcttcgagtggcaccgcggttactcaatccgcagggggttgttctacgtcgacttcctgagtcaggacaagatgttgctgccaaagagtagcgcccttttctaccagaagttgattgagaagaacggcttcccaccactccccgagaaccagcccctggagggcacctttccctgcgatttcgcttggggcgtggtggataattatattcaggtgagccagctgacaaaacctatcagcagcctgacaaagccttaccat

SEQ ID NO: 37 - RNA, 1548 nt, synthetic construct
  source 1..1548: mol_type = other RNA
gagcctggcgacggggcccagacctgggccagattcagcagaccccccgcacccgaggccgccggcctgttccagggcaccttccccgacggatttctgtgggccgtgggaagcgctgcctaccagaccgagggcggctggcaacagcacggcaagggcgccagcatctgggacaccttcacccaccatcctctggctcctcccggagacagcagaaacgccagcctgcctctgggagcccccagccccctgcagcccgccactggagacgtggccagcgactcctacaacaacgtgttccgcgacaccgaggccctgcgcgagctgggcgtgacccactaccgctttagcatcagctgggccagagtgctgcccaacggcagcgccggcgtgcccaaccgggaaggcctgagatactatcgccgcctgctggagaggctgagagagttgggcgtgcagcccgtggtgaccctgtaccactgggacctgccccagcgcctgcaggacgcctacggcggctgggccaacagggcactcgccgaccacttccgcgactacgccgagctgtgcttccgccacttcggcgggcaggtgaagtactggatcaccatcgacaacccctacgtggtggcctggcacggctacgctacaggaaggctggcccccgggatccgcggcagccccaggctgggctacctggtggcccacaacctgctgctggcacacgccaaagtgtggcacctgtataacaccagctttcgccccacccagggtggacaggtgagcattgccctgagttctcattggatcaaccccaggcgcatgaccgatcacagcatcaaggaatgccagaagagcctggacttcgtgctgggctggttcgccaagcccgtgtttatcgacggcgactaccccgagtctatgaagaacaacctcagcagcatcctgcctgacttcaccgagagcgagaagaagttcatcaagggcaccgccgacttcttcgccctgtgcttcggccccaccctgagcttccagctgctggatccccatatgaagttcagacaactcgagagtcctaacctgcgccagctgctgagctggatcgacctggaattcaaccacccacagatcttcatcgtggagaacggctggtttgtgagcggcaccactaagcgcgacgacgcaaagtatatgtattatctgaagaaattcatcatggaaaccctgaaggccatcaagctggacggcgtggacgtgatcggatacaccgcatggagcctgatggacggcttcgagtggcaccgcggttacagcatccgccggggcctgttctacgttgacttcctgagccaggacaagatgttgctgcccaagagctccgccctgttctaccagaagttgatcgagaagaacggcttcccaccactccccgagaaccagcccctggagggcaccttcccctgcgatttcgcctggggcgtggtggacaactacatccaggtgagccagctgacaaaacctatcagcagcctgacaaagccttaccat

SEQ ID NO: 38 - RNA, 1548 nt, synthetic construct
  source 1..1548: mol_type = other RNA
gagcctggagatggagcccaaacatgggccagattcagcagacctcccgctcctgaagccgccggcttgtttcagggaacctttcctgacggtttcctgtgggctgtgggcagcgccgcctatcagaccgagggcggctggcaacagcacggaaaaggagccagcatctgggataccttcacccaccaccccctggccccccccggcgattcccgcaatgccagcctccctctgggagcccctagccccctgcaacctgccacaggagacgtggcctcagacagctataacaacgtgttccgcgacaccgaggcactgcgcgagctgggcgtgacccattaccgctttagcatcagctgggccagagtgctgcccaatggctctgccggcgtgcccaaccgggagggcctgaggtactaccgccgcctgctggagaggctgcgggagctgggcgtgcagcccgtggtaaccctgtaccactgggacctgccccagcgcctgcaggacgcttacggcggctgggccaaccgcgctctcgcagaccacttccgcgactacgccgagctgtgctttcgccactttggcggccaggtgaagtattggatcaccatcgataacccttacgtggtggcctggcacggatacgctacaggccgcctggcccccggcatccgcggcagccccagactgggctacctggtggcccacaacctgctgctggcccacgccaaggtgtggcacctgtacaacaccagcttccgccccacccagggtggacaggtctctattgccctgagctctcactggattaaccccaggaggatgaccgatcacagcatcaaggaatgccagaagagcctggacttcgttctgggctggttcgccaagcccgtgtttatcgacggcgactaccccgagagcatgaagaacaacctgtctagcatcctgcccgacttcaccgagagcgaaaaaaaattcatcaagggcaccgccgatttcttcgccctgtgtttcggcccaaccctgagcttccaactgctggatccccacatgaagttcagacaactcgagagtcccaacctgcgccagctgctgagctggatcgatctggaattcaaccacccccagatattcatagtggagaacggctggtttgtaagcggcactactaagcgcgatgatgcaaagtacatgtactatctgaagaagttcatcatggaaaccctgaaggccatcaagctggatggcgtggacgtgatcggatacaccgcatggagcctgatggacggcttcgagtggcaccgcggttactcaatccgcagggggttgttctacgtcgacttcctgagtcaggacaagatgttgctgccaaagagtagcgcccttttctaccagaagttgattgagaagaacggcttcccaccactccccgagaaccagcccctggagggcacctttccctgcgatttcgcttggggcgtggtggataattatattcaggtgagccagctgacaaaacctatcagcagcctgacaaagccttaccat

SEQ ID NO: 39 - RNA, 1548 nt, synthetic construct
  source 1..1548: mol_type = other RNA
gagcctggcgacggggcccagacctgggccagattcagcagaccccccgcacccgaggccgccggcctgttccagggcaccttccccgacggatttctgtgggccgtgggaagcgctgcctaccagaccgagggcggctggcaacagcacggcaagggcgccagcatctgggacaccttcacccaccatcctctggctcctcccggagacagcagaaacgccagcctgcctctgggagcccccagccccctgcagcccgccactggagacgtggccagcgactcctacaacaacgtgttccgcgacaccgaggccctgcgcgagctgggcgtgacccactaccgctttagcatcagctgggccagagtgctgcccaacggcagcgccggcgtgcccaaccgggaaggcctgagatactatcgccgcctgctggagaggctgagagagttgggcgtgcagcccgtggtgaccctgtaccactgggacctgccccagcgcctgcaggacgcctacggcggctgggccaacagggcactcgccgaccacttccgcgactacgccgagctgtgcttccgccacttcggcgggcaggtgaagtactggatcaccatcgacaacccctacgtggtggcctggcacggctacgctacaggaaggctggcccccgggatccgcggcagccccaggctgggctacctggtggcccacaacctgctgctggcacacgccaaagtgtggcacctgtataacaccagctttcgccccacccagggtggacaggtgagcattgccctgagttctcattggatcaaccccaggcgcatgaccgatcacagcatcaaggaatgccagaagagcctggacttcgtgctgggctggttcgccaagcccgtgtttatcgacggcgactaccccgagtctatgaagaacaacctcagcagcatcctgcctgacgtcaccgagagcgagaagaagttcatcaagggcaccgccgacttcttcgccctgagcttcggccccaccctgagcttccagctgctggatccccatatgaagttcagacaactcgagagtcctaacctgcgccagctgctgagctggatcgacctggaattcaaccacccacagatcttcatcgtggagaacggctggtttgtgagcggcaccactaagcgcgacgacgcaaagtatatgtattatctgaagaaattcatcatggaaaccctgaaggccatcaagctggacggcgtggacgtgatcggatacaccgcatggagcctgatggacggcttcgagtggcaccgcggttacagcatccgccggggcctgttctacgttgacttcctgagccaggacaagatgttgctgcccaagagctccgccctgttctaccagaagttgatcgagaagaacggcttcccaccactccccgagaaccagcccctggagggcaccttcccctgcgatttcgcctggggcgtggtggacaactacatccaggtgagccagctgacaaaacctatcagcagcctgacaaagccttaccat

SEQ ID NO: 40 - RNA, 1548 nt, synthetic construct
  source 1..1548: mol_type = other RNA
gagcctggagatggagcccaaacatgggccagattcagcagacctcccgctcctgaagccgccggcttgtttcagggaacctttcctgacggtttcctgtgggctgtgggcagcgccgcctatcagaccgagggcggctggcaacagcacggaaaaggagccagcatctgggataccttcacccaccaccccctggccccccccggcgattcccgcaatgccagcctccctctgggagcccctagccccctgcaacctgccacaggagacgtggcctcagacagctataacaacgtgttccgcgacaccgaggcactgcgcgagctgggcgtgacccattaccgctttagcatcagctgggccagagtgctgcccaatggctctgccggcgtgcccaaccgggagggcctgaggtactaccgccgcctgctggagaggctgcgggagctgggcgtgcagcccgtggtaaccctgtaccactgggacctgccccagcgcctgcaggacgcttacggcggctgggccaaccgcgctctcgcagaccacttccgcgactacgccgagctgtgctttcgccactttggcggccaggtgaagtattggatcaccatcgataacccttacgtggtggcctggcacggatacgctacaggccgcctggcccccggcatccgcggcagccccagactgggctacctggtggcccacaacctgctgctggcccacgccaaggtgtggcacctgtacaacaccagcttccgccccacccagggtggacaggtctctattgccctgagctctcactggattaaccccaggaggatgaccgatcacagcatcaaggaatgccagaagagcctggacttcgttctgggctggttcgccaagcccgtgtttatcgacggcgactaccccgagagcatgaagaacaacctgtctagcatcctgcccgacgtcaccgagagcgaaaaaaaattcatcaagggcaccgccgatttcttcgccctgagcttcggcccaaccctgagcttccaactgctggatccccacatgaagttcagacaactcgagagtcccaacctgcgccagctgctgagctggatcgatctggaattcaaccacccccagatattcatagtggagaacggctggtttgtaagcggcactactaagcgcgatgatgcaaagtacatgtactatctgaagaagttcatcatggaaaccctgaaggccatcaagctggatggcgtggacgtgatcggatacaccgcatggagcctgatggacggcttcgagtggcaccgcggttactcaatccgcagggggttgttctacgtcgacttcctgagtcaggacaagatgttgctgccaaagagtagcgcccttttctaccagaagttgattgagaagaacggcttcccaccactccccgagaaccagcccctggagggcacctttccctgcgatttcgcttggggcgtggtggataattatattcaggtgagccagctgacaaaacctatcagcagcctgacaaagccttaccat

SEQ ID NO: 41 - RNA, 1650 nt, synthetic construct
  source 1..1650: mol_type = other RNA
atgcccgctagcgccccaccgagaagaccgcggccgccaccgccatcgctgtcgctgctgctggtgctgctgggactgggcggaagaagactgcgtgcggagcctggcgacggggcccagacctgggccagattcagcagaccccccgcacccgaggccgccggcctgttccagggcaccttccccgacggatttctgtgggccgtgggaagcgctgcctaccagaccgagggcggctggcaacagcacggcaagggcgccagcatctgggacaccttcacccaccatcctctggctcctcccggagacagcagaaacgccagcctgcctctgggagcccccagccccctgcagcccgccactggagacgtggccagcgactcctacaacaacgtgttccgcgacaccgaggccctgcgcgagctgggcgtgacccactaccgctttagcatcagctgggccagagtgctgcccaacggcagcgccggcgtgcccaaccgggaaggcctgagatactatcgccgcctgctggagaggctgagagagttgggcgtgcagcccgtggtgaccctgtaccactgggacctgccccagcgcctgcaggacgcctacggcggctgggccaacagggcactcgccgaccacttccgcgactacgccgagctgtgcttccgccacttcggcgggcaggtgaagtactggatcaccatcgacaacccctacgtggtggcctggcacggctacgctacaggaaggctggcccccgggatccgcggcagccccaggctgggctacctggtggcccacaacctgctgctggcacacgccaaagtgtggcacctgtataacaccagctttcgccccacccagggtggacaggtgagcattgccctgagttctcattggatcaaccccaggcgcatgaccgatcacagcatcaaggaatgccagaagagcctggacttcgtgctgggctggttcgccaagcccgtgtttatcgacggcgactaccccgagtctatgaagaacaacctcagcagcatcctgcctgacttcaccgagagcgagaagaagttcatcaagggcaccgccgacttcttcgccctgtgcttcggccccaccctgagcttccagctgctggatccccatatgaagttcagacaactcgagagtcctaacctgcgccagctgctgagctggatcgacctggaattcaaccacccacagatcttcatcgtggagaacggctggtttgtgagcggcaccactaagcgcgacgacgcaaagtatatgtattatctgaagaaattcatcatggaaaccctgaaggccatcaagctggacggcgtggacgtgatcggatacaccgcatggagcctgatggacggcttcgagtggcaccgcggttacagcatccgccggggcctgttctacgttgacttcctgagccaggacaagatgttgctgcccaagagctccgccctgttctaccagaagttgatcgagaagaacggcttcccaccactccccgagaaccagcccctggagggcaccttcccctgcgatttcgcctggggcgtggtggacaactacatccaggtgagccagctgacaaaacctatcagcagcctgacaaagccttaccattga

SEQ ID NO: 42 - RNA, 1650 nt, synthetic construct
  source 1..1650: mol_type = other RNA
atgcccgctagcgccccaccgagaagaccgcggccgccaccgccatcgctgtcgctgctgctggtgctgctgggactgggcggaagaagactgcgtgcggagcctggagatggagcccaaacatgggccagattcagcagacctcccgctcctgaagccgccggcttgtttcagggaacctttcctgacggtttcctgtgggctgtgggcagcgccgcctatcagaccgagggcggctggcaacagcacggaaaaggagccagcatctgggataccttcacccaccaccccctggccccccccggcgattcccgcaatgccagcctccctctgggagcccctagccccctgcaacctgccacaggagacgtggcctcagacagctataacaacgtgttccgcgacaccgaggcactgcgcgagctgggcgtgacccattaccgctttagcatcagctgggccagagtgctgcccaatggctctgccggcgtgcccaaccgggagggcctgaggtactaccgccgcctgctggagaggctgcgggagctgggcgtgcagcccgtggtaaccctgtaccactgggacctgccccagcgcctgcaggacgcttacggcggctgggccaaccgcgctctcgcagaccacttccgcgactacgccgagctgtgctttcgccactttggcggccaggtgaagtattggatcaccatcgataacccttacgtggtggcctggcacggatacgctacaggccgcctggcccccggcatccgcggcagccccagactgggctacctggtggcccacaacctgctgctggcccacgccaaggtgtggcacctgtacaacaccagcttccgccccacccagggtggacaggtctctattgccctgagctctcactggattaaccccaggaggatgaccgatcacagcatcaaggaatgccagaagagcctggacttcgttctgggctggttcgccaagcccgtgtttatcgacggcgactaccccgagagcatgaagaacaacctgtctagcatcctgcccgacttcaccgagagcgaaaaaaaattcatcaagggcaccgccgatttcttcgccctgtgtttcggcccaaccctgagcttccaactgctggatccccacatgaagttcagacaactcgagagtcccaacctgcgccagctgctgagctggatcgatctggaattcaaccacccccagatattcatagtggagaacggctggtttgtaagcggcactactaagcgcgatgatgcaaagtacatgtactatctgaagaagttcatcatggaaaccctgaaggccatcaagctggatggcgtggacgtgatcggatacaccgcatggagcctgatggacggcttcgagtggcaccgcggttactcaatccgcagggggttgttctacgtcgacttcctgagtcaggacaagatgttgctgccaaagagtagcgcccttttctaccagaagttgattgagaagaacggcttcccaccactccccgagaaccagcccctggagggcacctttccctgcgatttcgcttggggcgtggtggataattatattcaggtgagccagctgacaaaacctatcagcagcctgacaaagccttaccattga

SEQ ID NO: 43 - RNA, 1650 nt, synthetic construct
  source 1..1650: mol_type = other RNA
atgcccgctagcgccccaccgagaagaccgcggccgccaccgccatcgctgtcgctgctgctggtgctgctgggactgggcggaagaagactgcgtgcggagcctggcgacggggcccagacctgggccagattcagcagaccccccgcacccgaggccgccggcctgttccagggcaccttccccgacggatttctgtgggccgtgggaagcgctgcctaccagaccgagggcggctggcaacagcacggcaagggcgccagcatctgggacaccttcacccaccatcctctggctcctcccggagacagcagaaacgccagcctgcctctgggagcccccagccccctgcagcccgccactggagacgtggccagcgactcctacaacaacgtgttccgcgacaccgaggccctgcgcgagctgggcgtgacccactaccgctttagcatcagctgggccagagtgctgcccaacggcagcgccggcgtgcccaaccgggaaggcctgagatactatcgccgcctgctggagaggctgagagagttgggcgtgcagcccgtggtgaccctgtaccactgggacctgccccagcgcctgcaggacgcctacggcggctgggccaacagggcactcgccgaccacttccgcgactacgccgagctgtgcttccgccacttcggcgggcaggtgaagtactggatcaccatcgacaacccctacgtggtggcctggcacggctacgctacaggaaggctggcccccgggatccgcggcagccccaggctgggctacctggtggcccacaacctgctgctggcacacgccaaagtgtggcacctgtataacaccagctttcgccccacccagggtggacaggtgagcattgccctgagttctcattggatcaaccccaggcgcatgaccgatcacagcatcaaggaatgccagaagagcctggacttcgtgctgggctggttcgccaagcccgtgtttatcgacggcgactaccccgagtctatgaagaacaacctcagcagcatcctgcctgacgtcaccgagagcgagaagaagttcatcaagggcaccgccgacttcttcgccctgagcttcggccccaccctgagcttccagctgctggatccccatatgaagttcagacaactcgagagtcctaacctgcgccagctgctgagctggatcgacctggaattcaaccacccacagatcttcatcgtggagaacggctggtttgtgagcggcaccactaagcgcgacgacgcaaagtatatgtattatctgaagaaattcatcatggaaaccctgaaggccatcaagctggacggcgtggacgtgatcggatacaccgcatggagcctgatggacggcttcgagtggcaccgcggttacagcatccgccggggcctgttctacgttgacttcctgagccaggacaagatgttgctgcccaagagctccgccctgttctaccagaagttgatcgagaagaacggcttcccaccactccccgagaaccagcccctggagggcaccttcccctgcgatttcgcctggggcgtggtggacaactacatccaggtgagccagctgacaaaacctatcagcagcctgacaaagccttaccattga

SEQ ID NO: 44 - RNA, 1650 nt, synthetic construct
  source 1..1650: mol_type = other RNA
atgcccgctagcgccccaccgagaagaccgcggccgccaccgccatcgctgtcgctgctgctggtgctgctgggactgggcggaagaagactgcgtgcggagcctggagatggagcccaaacatgggccagattcagcagacctcccgctcctgaagccgccggcttgtttcagggaacctttcctgacggtttcctgtgggctgtgggcagcgccgcctatcagaccgagggcggctggcaacagcacggaaaaggagccagcatctgggataccttcacccaccaccccctggccccccccggcgattcccgcaatgccagcctccctctgggagcccctagccccctgcaacctgccacaggagacgtggcctcagacagctataacaacgtgttccgcgacaccgaggcactgcgcgagctgggcgtgacccattaccgctttagcatcagctgggccagagtgctgcccaatggctctgccggcgtgcccaaccgggagggcctgaggtactaccgccgcctgctggagaggctgcgggagctgggcgtgcagcccgtggtaaccctgtaccactgggacctgccccagcgcctgcaggacgcttacggcggctgggccaaccgcgctctcgcagaccacttccgcgactacgccgagctgtgctttcgccactttggcggccaggtgaagtattggatcaccatcgataacccttacgtggtggcctggcacggatacgctacaggccgcctggcccccggcatccgcggcagccccagactgggctacctggtggcccacaacctgctgctggcccacgccaaggtgtggcacctgtacaacaccagcttccgccccacccagggtggacaggtctctattgccctgagctctcactggattaaccccaggaggatgaccgatcacagcatcaaggaatgccagaagagcctggacttcgttctgggctggttcgccaagcccgtgtttatcgacggcgactaccccgagagcatgaagaacaacctgtctagcatcctgcccgacgtcaccgagagcgaaaaaaaattcatcaagggcaccgccgatttcttcgccctgagcttcggcccaaccctgagcttccaactgctggatccccacatgaagttcagacaactcgagagtcccaacctgcgccagctgctgagctggatcgatctggaattcaaccacccccagatattcatagtggagaacggctggtttgtaagcggcactactaagcgcgatgatgcaaagtacatgtactatctgaagaagttcatcatggaaaccctgaaggccatcaagctggatggcgtggacgtgatcggatacaccgcatggagcctgatggacggcttcgagtggcaccgcggttactcaatccgcagggggttgttctacgtcgacttcctgagtcaggacaagatgttgctgccaaagagtagcgcccttttctaccagaagttgattgagaagaacggcttcccaccactccccgagaaccagcccctggagggcacctttccctgcgatttcgcttggggcgtggtggataattatattcaggtgagccagctgacaaaacctatcagcagcctgacaaagccttaccattga

SEQ ID NO: 45 - RNA, 1953 nt, synthetic construct
  source 1..1953: mol_type = other RNA
gggagacataaaccctggcgcgctcgcggcccggcactcttctggtccccacagactcagagagaacccaccatgcccgctagcgccccaccgagaagaccgcggccgccaccgccatcgctgtcgctgctgctggtgctgctgggactgggcggaagaagactgcgtgcggagcctggcgacggggcccagacctgggccagattcagcagaccccccgcacccgaggccgccggcctgttccagggcaccttccccgacggatttctgtgggccgtgggaagcgctgcctaccagaccgagggcggctggcaacagcacggcaagggcgccagcatctgggacaccttcacccaccatcctctggctcctcccggagacagcagaaacgccagcctgcctctgggagcccccagccccctgcagcccgccactggagacgtggccagcgactcctacaacaacgtgttccgcgacaccgaggccctgcgcgagctgggcgtgacccactaccgctttagcatcagctgggccagagtgctgcccaacggcagcgccggcgtgcccaaccgggaaggcctgagatactatcgccgcctgctggagaggctgagagagttgggcgtgcagcccgtggtgaccctgtaccactgggacctgccccagcgcctgcaggacgcctacggcggctgggccaacagggcactcgccgaccacttccgcgactacgccgagctgtgcttccgccacttcggcgggcaggtgaagtactggatcaccatcgacaacccctacgtggtggcctggcacggctacgctacaggaaggctggcccccgggatccgcggcagccccaggctgggctacctggtggcccacaacctgctgctggcacacgccaaagtgtggcacctgtataacaccagctttcgccccacccagggtggacaggtgagcattgccctgagttctcattggatcaaccccaggcgcatgaccgatcacagcatcaaggaatgccagaagagcctggacttcgtgctgggctggttcgccaagcccgtgtttatcgacggcgactaccccgagtctatgaagaacaacctcagcagcatcctgcctgacttcaccgagagcgagaagaagttcatcaagggcaccgccgacttcttcgccctgtgcttcggccccaccctgagcttccagctgctggatccccatatgaagttcagacaactcgagagtcctaacctgcgccagctgctgagctggatcgacctggaattcaaccacccacagatcttcatcgtggagaacggctggtttgtgagcggcaccactaagcgcgacgacgcaaagtatatgtattatctgaagaaattcatcatggaaaccctgaaggccatcaagctggacggcgtggacgtgatcggatacaccgcatggagcctgatggacggcttcgagtggcaccgcggttacagcatccgccggggcctgttctacgttgacttcctgagccaggacaagatgttgctgcccaagagctccgccctgttctaccagaagttgatcgagaagaacggcttcccaccactccccgagaaccagcccctggagggcaccttcccctgcgatttcgcctggggcgtggtggacaactacatccaggtgagccagctgacaaaacctatcagcagcctgacaaagccttaccattgagctggagcctcggtggccatgcttcttgccccttgggcctccccccagcccctcctccccttcctgcacccgtacccccgtggtctttgaataaagtctgagtgggcggcaaaaaaaaaaaaaaaaaaaaaaaaaaaaaaaaaaaaaaaaaaaaaaaaaaaaaaaaaaaaaaaaaaaaaaaaaaaaaaaaaaaaaaaaaaaaaaaaaaaaaaaaaaaaaaaaaaaaaaaaa

SEQ ID NO: 46 - RNA, 1953 nt, synthetic construct
  source 1..1953: mol_type = other RNA
gggagacataaaccctggcgcgctcgcggcccggcactcttctggtccccacagactcagagagaacccaccatgcccgctagcgccccaccgagaagaccgcggccgccaccgccatcgctgtcgctgctgctggtgctgctgggactgggcggaagaagactgcgtgcggagcctggagatggagcccaaacatgggccagattcagcagacctcccgctcctgaagccgccggcttgtttcagggaacctttcctgacggtttcctgtgggctgtgggcagcgccgcctatcagaccgagggcggctggcaacagcacggaaaaggagccagcatctgggataccttcacccaccaccccctggccccccccggcgattcccgcaatgccagcctccctctgggagcccctagccccctgcaacctgccacaggagacgtggcctcagacagctataacaacgtgttccgcgacaccgaggcactgcgcgagctgggcgtgacccattaccgctttagcatcagctgggccagagtgctgcccaatggctctgccggcgtgcccaaccgggagggcctgaggtactaccgccgcctgctggagaggctgcgggagctgggcgtgcagcccgtggtaaccctgtaccactgggacctgccccagcgcctgcaggacgcttacggcggctgggccaaccgcgctctcgcagaccacttccgcgactacgccgagctgtgctttcgccactttggcggccaggtgaagtattggatcaccatcgataacccttacgtggtggcctggcacggatacgctacaggccgcctggcccccggcatccgcggcagccccagactgggctacctggtggcccacaacctgctgctggcccacgccaaggtgtggcacctgtacaacaccagcttccgccccacccagggtggacaggtctctattgccctgagctctcactggattaaccccaggaggatgaccgatcacagcatcaaggaatgccagaagagcctggacttcgttctgggctggttcgccaagcccgtgtttatcgacggcgactaccccgagagcatgaagaacaacctgtctagcatcctgcccgacttcaccgagagcgaaaaaaaattcatcaagggcaccgccgatttcttcgccctgtgtttcggcccaaccctgagcttccaactgctggatccccacatgaagttcagacaactcgagagtcccaacctgcgccagctgctgagctggatcgatctggaattcaaccacccccagatattcatagtggagaacggctggtttgtaagcggcactactaagcgcgatgatgcaaagtacatgtactatctgaagaagttcatcatggaaaccctgaaggccatcaagctggatggcgtggacgtgatcggatacaccgcatggagcctgatggacggcttcgagtggcaccgcggttactcaatccgcagggggttgttctacgtcgacttcctgagtcaggacaagatgttgctgccaaagagtagcgcccttttctaccagaagttgattgagaagaacggcttcccaccactccccgagaaccagcccctggagggcacctttccctgcgatttcgcttggggcgtggtggataattatattcaggtgagccagctgacaaaacctatcagcagcctgacaaagccttaccattgagctggagcctcggtggccatgcttcttgccccttgggcctccccccagcccctcctccccttcctgcacccgtacccccgtggtctttgaataaagtctgagtgggcggcaaaaaaaaaaaaaaaaaaaaaaaaaaaaaaaaaaaaaaaaaaaaaaaaaaaaaaaaaaaaaaaaaaaaaaaaaaaaaaaaaaaaaaaaaaaaaaaaaaaaaaaaaaaaaaaaaaaaaaaaa

SEQ ID NO: 47 - RNA, 1953 nt, synthetic construct
  source 1..1953: mol_type = other RNA
gggagacataaaccctggcgcgctcgcggcccggcactcttctggtccccacagactcagagagaacccaccatgcccgctagcgccccaccgagaagaccgcggccgccaccgccatcgctgtcgctgctgctggtgctgctgggactgggcggaagaagactgcgtgcggagcctggcgacggggcccagacctgggccagattcagcagaccccccgcacccgaggccgccggcctgttccagggcaccttccccgacggatttctgtgggccgtgggaagcgctgcctaccagaccgagggcggctggcaacagcacggcaagggcgccagcatctgggacaccttcacccaccatcctctggctcctcccggagacagcagaaacgccagcctgcctctgggagcccccagccccctgcagcccgccactggagacgtggccagcgactcctacaacaacgtgttccgcgacaccgaggccctgcgcgagctgggcgtgacccactaccgctttagcatcagctgggccagagtgctgcccaacggcagcgccggcgtgcccaaccgggaaggcctgagatactatcgccgcctgctggagaggctgagagagttgggcgtgcagcccgtggtgaccctgtaccactgggacctgccccagcgcctgcaggacgcctacggcggctgggccaacagggcactcgccgaccacttccgcgactacgccgagctgtgcttccgccacttcggcgggcaggtgaagtactggatcaccatcgacaacccctacgtggtggcctggcacggctacgctacaggaaggctggcccccgggatccgcggcagccccaggctgggctacctggtggcccacaacctgctgctggcacacgccaaagtgtggcacctgtataacaccagctttcgccccacccagggtggacaggtgagcattgccctgagttctcattggatcaaccccaggcgcatgaccgatcacagcatcaaggaatgccagaagagcctggacttcgtgctgggctggttcgccaagcccgtgtttatcgacggcgactaccccgagtctatgaagaacaacctcagcagcatcctgcctgacgtcaccgagagcgagaagaagttcatcaagggcaccgccgacttcttcgccctgagcttcggccccaccctgagcttccagctgctggatccccatatgaagttcagacaactcgagagtcctaacctgcgccagctgctgagctggatcgacctggaattcaaccacccacagatcttcatcgtggagaacggctggtttgtgagcggcaccactaagcgcgacgacgcaaagtatatgtattatctgaagaaattcatcatggaaaccctgaaggccatcaagctggacggcgtggacgtgatcggatacaccgcatggagcctgatggacggcttcgagtggcaccgcggttacagcatccgccggggcctgttctacgttgacttcctgagccaggacaagatgttgctgcccaagagctccgccctgttctaccagaagttgatcgagaagaacggcttcccaccactccccgagaaccagcccctggagggcaccttcccctgcgatttcgcctggggcgtggtggacaactacatccaggtgagccagctgacaaaacctatcagcagcctgacaaagccttaccattgagctggagcctcggtggccatgcttcttgccccttgggcctccccccagcccctcctccccttcctgcacccgtacccccgtggtctttgaataaagtctgagtgggcggcaaaaaaaaaaaaaaaaaaaaaaaaaaaaaaaaaaaaaaaaaaaaaaaaaaaaaaaaaaaaaaaaaaaaaaaaaaaaaaaaaaaaaaaaaaaaaaaaaaaaaaaaaaaaaaaaaaaaaaaaa

SEQ ID NO: 48 - RNA, 1953 nt, synthetic construct
  source 1..1953: mol_type = other RNA
gggagacataaaccctggcgcgctcgcggcccggcactcttctggtccccacagactcagagagaacccaccatgcccgctagcgccccaccgagaagaccgcggccgccaccgccatcgctgtcgctgctgctggtgctgctgggactgggcggaagaagactgcgtgcggagcctggagatggagcccaaacatgggccagattcagcagacctcccgctcctgaagccgccggcttgtttcagggaacctttcctgacggtttcctgtgggctgtgggcagcgccgcctatcagaccgagggcggctggcaacagcacggaaaaggagccagcatctgggataccttcacccaccaccccctggccccccccggcgattcccgcaatgccagcctccctctgggagcccctagccccctgcaacctgccacaggagacgtggcctcagacagctataacaacgtgttccgcgacaccgaggcactgcgcgagctgggcgtgacccattaccgctttagcatcagctgggccagagtgctgcccaatggctctgccggcgtgcccaaccgggagggcctgaggtactaccgccgcctgctggagaggctgcgggagctgggcgtgcagcccgtggtaaccctgtaccactgggacctgccccagcgcctgcaggacgcttacggcggctgggccaaccgcgctctcgcagaccacttccgcgactacgccgagctgtgctttcgccactttggcggccaggtgaagtattggatcaccatcgataacccttacgtggtggcctggcacggatacgctacaggccgcctggcccccggcatccgcggcagccccagactgggctacctggtggcccacaacctgctgctggcccacgccaaggtgtggcacctgtacaacaccagcttccgccccacccagggtggacaggtctctattgccctgagctctcactggattaaccccaggaggatgaccgatcacagcatcaaggaatgccagaagagcctggacttcgttctgggctggttcgccaagcccgtgtttatcgacggcgactaccccgagagcatgaagaacaacctgtctagcatcctgcccgacgtcaccgagagcgaaaaaaaattcatcaagggcaccgccgatttcttcgccctgagcttcggcccaaccctgagcttccaactgctggatccccacatgaagttcagacaactcgagagtcccaacctgcgccagctgctgagctggatcgatctggaattcaaccacccccagatattcatagtggagaacggctggtttgtaagcggcactactaagcgcgatgatgcaaagtacatgtactatctgaagaagttcatcatggaaaccctgaaggccatcaagctggatggcgtggacgtgatcggatacaccgcatggagcctgatggacggcttcgagtggcaccgcggttactcaatccgcagggggttgttctacgtcgacttcctgagtcaggacaagatgttgctgccaaagagtagcgcccttttctaccagaagttgattgagaagaacggcttcccaccactccccgagaaccagcccctggagggcacctttccctgcgatttcgcttggggcgtggtggataattatattcaggtgagccagctgacaaaacctatcagcagcctgacaaagccttaccattgagctggagcctcggtggccatgcttcttgccccttgggcctccccccagcccctcctccccttcctgcacccgtacccccgtggtctttgaataaagtctgagtgggcggcaaaaaaaaaaaaaaaaaaaaaaaaaaaaaaaaaaaaaaaaaaaaaaaaaaaaaaaaaaaaaaaaaaaaaaaaaaaaaaaaaaaaaaaaaaaaaaaaaaaaaaaaaaaaaaaaaaaaaaaaa

SEQ ID NO: 49 - protein, 1012 aa, Homo sapiens
MPASAPPRRPRPPPPSLSLLLVLLGLGGRRLRAEPGDGAQTWARFSRPPAPEAAGLFQGTFPDGFLWAVGSAAYQTEGGWQQHGKGASIWDTFTHHPLAPPGDSRNASLPLGAPSPLQPATGDVASDSYNNVFRDTEALRELGVTHYRFSISWARVLPNGSAGVPNREGLRYYRRLLERLRELGVQPVVTLYHWDLPQRLQDAYGGWANRALADHFRDYAELCFRHFGGQVKYWITIDNPYVVAWHGYATGRLAPGIRGSPRLGYLVAHNLLLAHAKVWHLYNTSFRPTQGGQVSIALSSHWINPRRMTDHSIKECQKSLDFVLGWFAKPVFIDGDYPESMKNNLSSILPDFTESEKKFIKGTADFFALCFGPTLSFQLLDPHMKFRQLESPNLRQLLSWIDLEFNHPQIFIVENGWFVSGTTKRDDAKYMYYLKKFIMETLKAIKLDGVDVIGYTAWSLMDGFEWHRGYSIRRGLFYVDFLSQDKMLLPKSSALFYQKLIEKNGFPPLPENQPLEGTFPCDFAWGVVDNYIQVDTTLSQFTDLNVYLWDVHHSKRLIKVDGVVTKKRKSYCVDFAAIQPQIALLQEMHVTHFRFSLDWALILPLGNQSQVNHTILQYYRCMASELVRVNITPVVALWQPMAPNQGLPRLLARQGAWENPYTALAFAEYARLCFQELGHHVKLWITMNEPYTRNMTYSAGHNLLKAHALAWHVYNEKFRHAQNGKISIALQADWIEPACPFSQKDKEVAERVLEFDIGWLAEPIFGSGDYPWVMRDWLNQRNNFLLPYFTEDEKKLIQGTFDFLALSHYTTILVDSEKEDPIKYNDYLEVQEMTDITWLNSPSQVAVVPWGLRKVLNWLKFKYGDLPMYIISNGIDDGLHAEDDQLRVYYMQNYINEALKAHILDGINLCGYFAYSFNDRTAPRFGLYRYAADQFEPKASMKHYRKIIDSNGFPGPETLERFCPEEFTVCTECSFFHTRKSLLAFIAFLFFASIISLSLIFYYSKKGRRSYK

SEQ ID NO: 50 - protein, 549 aa, Homo sapiens
MPASAPPRRPRPPPPSLSLLLVLLGLGGRRLRAEPGDGAQTWARFSRPPAPEAAGLFQGTFPDGFLWAVGSAAYQTEGGWQQHGKGASIWDTFTHHPLAPPGDSRNASLPLGAPSPLQPATGDVASDSYNNVFRDTEALRELGVTHYRFSISWARVLPNGSAGVPNREGLRYYRRLLERLRELGVQPVVTLYHWDLPQRLQDAYGGWANRALADHFRDYAELCFRHFGGQVKYWITIDNPYVVAWHGYATGRLAPGIRGSPRLGYLVAHNLLLAHAKVWHLYNTSFRPTQGGQVSIALSSHWINPRRMTDHSIKECQKSLDFVLGWFAKPVFIDGDYPESMKNNLSSILPDFTESEKKFIKGTADFFALCFGPTLSFQLLDPHMKFRQLESPNLRQLLSWIDLEFNHPQIFIVENGWFVSGTTKRDDAKYMYYLKKFIMETLKAIKLDGVDVIGYTAWSLMDGFEWHRGYSIRRGLFYVDFLSQDKMLLPKSSALFYQKLIEKNGFPPLPENQPLEGTFPCDFAWGVVDNYIQVSQLTKPISSLTKPYH

SEQ ID NO: 51 - protein, 33 aa, Homo sapiens
MPASAPPRRPRPPPPSLSLLLVLLGLGGRRLRA

SEQ ID NO: 52 - protein, 451 aa, Homo sapiens
LFQGTFPDGFLWAVGSAAYQTEGGWQQHGKGASIWDTFTHHPLAPPGDSRNASLPLGAPSPLQPATGDVASDSYNNVFRDTEALRELGVTHYRFSISWARVLPNGSAGVPNREGLRYYRRLLERLRELGVQPVVTLYHWDLPQRLQDAYGGWANRALADHFRDYAELCFRHFGGQVKYWITIDNPYVVAWHGYATGRLAPGIRGSPRLGYLVAHNLLLAHAKVWHLYNTSFRPTQGGQVSIALSSHWINPRRMTDHSIKECQKSLDFVLGWFAKPVFIDGDYPESMKNNLSSILPDFTESEKKFIKGTADFFALCFGPTLSFQLLDPHMKFRQLESPNLRQLLSWIDLEFNHPQIFIVENGWFVSGTTKRDDAKYMYYLKKFIMETLKAIKLDGVDVIGYTAWSLMDGFEWHRGYSIRRGLFYVDFLSQDKMLLPKSSALFYQKLIEKNGF

SEQ ID NO: 53 - protein, 451 aa, synthetic construct
LFQGTFPDGFLWAVGSAAYQTEGGWQQHGKGASIWDTFTHHPLAPPGDSRNASLPLGAPSPLQPATGDVASDSYNNVFRDTEALRELGVTHYRFSISWARVLPNGSAGVPNREGLRYYRRLLERLRELGVQPVVTLYHWDLPQRLQDAYGGWANRALADHFRDYAELCFRHFGGQVKYWITIDNPYVVAWHGYATGRLAPGIRGSPRLGYLVAHNLLLAHAKVWHLYNTSFRPTQGGQVSIALSSHWINPRRMTDHSIKECQKSLDFVLGWFAKPVFIDGDYPESMKNNLSSILPDVTESEKKFIKGTADFFALSFGPTLSFQLLDPHMKFRQLESPNLRQLLSWIDLEFNHPQIFIVENGWFVSGTTKRDDAKYMYYLKKFIMETLKAIKLDGVDVIGYTAWSLMDGFEWHRGYSIRRGLFYVDFLSQDKMLLPKSSALFYQKLIEKNGF

SEQ ID NO: 54 - protein, 897 aa, Homo sapiens
LFQGTFPDGFLWAVGSAAYQTEGGWQQHGKGASIWDTFTHHPLAPPGDSRNASLPLGAPSPLQPATGDVASDSYNNVFRDTEALRELGVTHYRFSISWARVLPNGSAGVPNREGLRYYRRLLERLRELGVQPVVTLYHWDLPQRLQDAYGGWANRALADHFRDYAELCFRHFGGQVKYWITIDNPYVVAWHGYATGRLAPGIRGSPRLGYLVAHNLLLAHAKVWHLYNTSFRPTQGGQVSIALSSHWINPRRMTDHSIKECQKSLDFVLGWFAKPVFIDGDYPESMKNNLSSILPDFTESEKKFIKGTADFFALCFGPTLSFQLLDPHMKFRQLESPNLRQLLSWIDLEFNHPQIFIVENGWFVSGTTKRDDAKYMYYLKKFIMETLKAIKLDGVDVIGYTAWSLMDGFEWHRGYSIRRGLFYVDFLSQDKMLLPKSSALFYQKLIEKNGFPPLPENQPLEGTFPCDFAWGVVDNYIQVDTTLSQFTDLNVYLWDVHHSKRLIKVDGVVTKKRKSYCVDFAAIQPQIALLQEMHVTHFRFSLDWALILPLGNQSQVNHTILQYYRCMASELVRVNITPVVALWQPMAPNQGLPRLLARQGAWENPYTALAFAEYARLCFQELGHHVKLWITMNEPYTRNMTYSAGHNLLKAHALAWHVYNEKFRHAQNGKISIALQADWIEPACPFSQKDKEVAERVLEFDIGWLAEPIFGSGDYPWVMRDWLNQRNNFLLPYFTEDEKKLIQGTFDFLALSHYTTILVDSEKEDPIKYNDYLEVQEMTDITWLNSPSQVAVVPWGLRKVLNWLKFKYGDLPMYIISNGIDDGLHAEDDQLRVYYMQNYINEALKAHILDGINLCGYFAYSFNDRTAPRFGLYRYAADQFEPKASMKHYRKIIDSNG

SEQ ID NO: 55 - protein, 506 aa, Homo sapiens
MPASAPPRRPRPPPPSLSLLLVLLGLGGRRLRAEPGDGAQTWARFSRPPAPEAAGLFQGTFPDGFLWAVGSAAYQTEGGWQQHGKGASIWDTFTHHPLAPPGDSRNASLPLGAPSPLQPATGDVASDSYNNVFRDTEALRELGVTHYRFSISWARVLPNGSAGVPNREGLRYYRRLLERLRELGVQPVVTLYHWDLPQRLQDAYGGWANRALADHFRDYAELCFRHFGGQVKYWITIDNPYVVAWHGYATGRLAPGIRGSPRLGYLVAHNLLLAHAKVWHLYNTSFRPTQGGQVSIALSSHWINPRRMTDHSIKECQKSLDFVLGWFAKPVFIDGDYPESMKNNLSSILPDFTESEKKFIKGTADFFALCFGPTLSFQLLDPHMKFRQLESPNLRQLLSWIDLEFNHPQIFIVENGWFVSGTTKRDDAKYMYYLKKFIMETLKAIKLDGVDVIGYTAWSLMDGFEWHRGYSIRRGLFYVDFLSQDKMLLPKSSALFYQKLIEKNGF

SEQ ID NO: 56 - protein, 506 aa, synthetic construct
MPASAPPRRPRPPPPSLSLLLVLLGLGGRRLRAEPGDGAQTWARFSRPPAPEAAGLFQGTFPDGFLWAVGSAAYQTEGGWQQHGKGASIWDTFTHHPLAPPGDSRNASLPLGAPSPLQPATGDVASDSYNNVFRDTEALRELGVTHYRFSISWARVLPNGSAGVPNREGLRYYRRLLERLRELGVQPVVTLYHWDLPQRLQDAYGGWANRALADHFRDYAELCFRHFGGQVKYWITIDNPYVVAWHGYATGRLAPGIRGSPRLGYLVAHNLLLAHAKVWHLYNTSFRPTQGGQVSIALSSHWINPRRMTDHSIKECQKSLDFVLGWFAKPVFIDGDYPESMKNNLSSILPDVTESEKKFIKGTADFFALSFGPTLSFQLLDPHMKFRQLESPNLRQLLSWIDLEFNHPQIFIVENGWFVSGTTKRDDAKYMYYLKKFIMETLKAIKLDGVDVIGYTAWSLMDGFEWHRGYSIRRGLFYVDFLSQDKMLLPKSSALFYQKLIEKNGF

SEQ ID NO: 57 - protein, 981 aa, Homo sapiens
MPASAPPRRPRPPPPSLSLLLVLLGLGGRRLRAEPGDGAQTWARFSRPPAPEAAGLFQGTFPDGFLWAVGSAAYQTEGGWQQHGKGASIWDTFTHHPLAPPGDSRNASLPLGAPSPLQPATGDVASDSYNNVFRDTEALRELGVTHYRFSISWARVLPNGSAGVPNREGLRYYRRLLERLRELGVQPVVTLYHWDLPQRLQDAYGGWANRALADHFRDYAELCFRHFGGQVKYWITIDNPYVVAWHGYATGRLAPGIRGSPRLGYLVAHNLLLAHAKVWHLYNTSFRPTQGGQVSIALSSHWINPRRMTDHSIKECQKSLDFVLGWFAKPVFIDGDYPESMKNNLSSILPDFTESEKKFIKGTADFFALCFGPTLSFQLLDPHMKFRQLESPNLRQLLSWIDLEFNHPQIFIVENGWFVSGTTKRDDAKYMYYLKKFIMETLKAIKLDGVDVIGYTAWSLMDGFEWHRGYSIRRGLFYVDFLSQDKMLLPKSSALFYQKLIEKNGFPPLPENQPLEGTFPCDFAWGVVDNYIQVDTTLSQFTDLNVYLWDVHHSKRLIKVDGVVTKKRKSYCVDFAAIQPQIALLQEMHVTHFRFSLDWALILPLGNQSQVNHTILQYYRCMASELVRVNITPVVALWQPMAPNQGLPRLLARQGAWENPYTALAFAEYARLCFQELGHHVKLWITMNEPYTRNMTYSAGHNLLKAHALAWHVYNEKFRHAQNGKISIALQADWIEPACPFSQKDKEVAERVLEFDIGWLAEPIFGSGDYPWVMRDWLNQRNNFLLPYFTEDEKKLIQGTFDFLALSHYTTILVDSEKEDPIKYNDYLEVQEMTDITWLNSPSQVAVVPWGLRKVLNWLKFKYGDLPMYIISNGIDDGLHAEDDQLRVYYMQNYINEALKAHILDGINLCGYFAYSFNDRTAPRFGLYRYAADQFEPKASMKHYRKIIDSNGFPGPETLERFCPEEFTVCTECSFFHTRKS

SEQ ID NO: 58 - protein, 981 aa, synthetic construct
MPASAPPRRPRPPPPSLSLLLVLLGLGGRRLRAEPGDGAQTWARFSRPPAPEAAGLFQGTFPDGFLWAVGSAAYQTEGGWQQHGKGASIWDTFTHHPLAPPGDSRNASLPLGAPSPLQPATGDVASDSYNNVFRDTEALRELGVTHYRFSISWARVLPNGSAGVPNREGLRYYRRLLERLRELGVQPVVTLYHWDLPQRLQDAYGGWANRALADHFRDYAELCFRHFGGQVKYWITIDNPYVVAWHGYATGRLAPGIRGSPRLGYLVAHNLLLAHAKVWHLYNTSFRPTQGGQVSIALSSHWINPRRMTDHSIKECQKSLDFVLGWFAKPVFIDGDYPESMKNNLSSILPDVTESEKKFIKGTADFFALSFGPTLSFQLLDPHMKFRQLESPNLRQLLSWIDLEFNHPQIFIVENGWFVSGTTKRDDAKYMYYLKKFIMETLKAIKLDGVDVIGYTAWSLMDGFEWHRGYSIRRGLFYVDFLSQDKMLLPKSSALFYQKLIEKNGFPPLPENQPLEGTFPCDFAWGVVDNYIQVDTTLSQFTDLNVYLWDVHHSKRLIKVDGVVTKKRKSYCVDFAAIQPQIALLQEMHVTHFRFSLDWALILPLGNQSQVNHTILQYYRCMASELVRVNITPVVALWQPMAPNQGLPRLLARQGAWENPYTALAFAEYARLCFQELGHHVKLWITMNEPYTRNMTYSAGHNLLKAHALAWHVYNEKFRHAQNGKISIALQADWIEPACPFSQKDKEVAERVLEFDIGWLAEPIFGSGDYPWVMRDWLNQRNNFLLPYFTEDEKKLIQGTFDFLALSHYTTILVDSEKEDPIKYNDYLEVQEMTDITWLNSPSQVAVVPWGLRKVLNWLKFKYGDLPMYIISNGIDDGLHAEDDQLRVYYMQNYINEALKAHILDGINLCGYFAYSFNDRTAPRFGLYRYAADQFEPKASMKHYRKIIDSNGFPGPETLERFCPEEFTVCTECSFFHTRKS

SEQ ID NO: 59 - protein, 549 aa, Homo sapiens; identical to SEQ ID NO: 50

SEQ ID NO: 60 - protein, 549 aa, synthetic construct
MPASAPPRRPRPPPPSLSLLLVLLGLGGRRLRAEPGDGAQTWARFSRPPAPEAAGLFQGTFPDGFLWAVGSAAYQTEGGWQQHGKGASIWDTFTHHPLAPPGDSRNASLPLGAPSPLQPATGDVASDSYNNVFRDTEALRELGVTHYRFSISWARVLPNGSAGVPNREGLRYYRRLLERLRELGVQPVVTLYHWDLPQRLQDAYGGWANRALADHFRDYAELCFRHFGGQVKYWITIDNPYVVAWHGYATGRLAPGIRGSPRLGYLVAHNLLLAHAKVWHLYNTSFRPTQGGQVSIALSSHWINPRRMTDHSIKECQKSLDFVLGWFAKPVFIDGDYPESMKNNLSSILPDVTESEKKFIKGTADFFALSFGPTLSFQLLDPHMKFRQLESPNLRQLLSWIDLEFNHPQIFIVENGWFVSGTTKRDDAKYMYYLKKFIMETLKAIKLDGVDVIGYTAWSLMDGFEWHRGYSIRRGLFYVDFLSQDKMLLPKSSALFYQKLIEKNGFPPLPENQPLEGTFPCDFAWGVVDNYIQVSQLTKPISSLTKPYH

SEQ ID NO: 61 - RNA, 72 nt, synthetic construct
  source 1..72: mol_type = other RNA
gggagacataaaccctggcgcgctcgcggcccggcactcttctggtccccacagactcagagagaacccacc

SEQ ID NO: 62 - RNA, 111 nt, synthetic construct
  source 1..111: mol_type = other RNA
gctggagcctcggtggccatgcttcttgccccttgggcctccccccagcccctcctccccttcctgcacccgtacccccgtggtctttgaataaagtctgagtgggcggca

SEQ ID NO: 63 - RNA, 15 nt, synthetic construct
  source 1..15: mol_type = other RNA
  misc_feature 5: note = any 0 to 10 nucleotides
  misc_feature 10: note = any 0 to 10 pyrimidine (y) nucleotides
yccancccwntcycc

SEQ ID NO: 64 - RNA, 2937 nt, synthetic construct
  source 1..2937: mol_type = other RNA
gagcctggcgacggggcccagacctgggccagattcagcagaccccccgcacccgaggccgccggcctgttccagggcaccttccccgacggatttctgtgggccgtgggaagcgctgcctaccagaccgagggcggctggcaacagcacggcaagggcgccagcatctgggacaccttcacccaccatcctctggctcctcccggagacagcagaaacgccagcctgcctctgggagcccccagccccctgcagcccgccactggagacgtggccagcgactcctacaacaacgtgttccgcgacaccgaggccctgcgcgagctgggcgtgacccactaccgctttagcatcagctgggccagagtgctgcccaacggcagcgccggcgtgcccaaccgggaaggcctgagatactatcgccgcctgctggagaggctgagagagttgggcgtgcagcccgtggtgaccctgtaccactgggacctgccccagcgcctgcaggacgcctacggcggctgggccaacagggcactcgccgaccacttccgcgactacgccgagctgtgcttccgccacttcggcgggcaggtgaagtactggatcaccatcgacaacccctacgtggtggcctggcacggctacgctacaggaaggctggcccccgggatccgcggcagccccaggctgggctacctggtggcccacaacctgctgctggcacacgccaaagtgtggcacctgtataacaccagctttcgccccacccagggtggacaggtgagcattgccctgagttctcattggatcaaccccaggcgcatgaccgatcacagcatcaaggaatgccagaagagcctggacttcgtgctgggctggttcgccaagcccgtgtttatcgacggcgactaccccgagtctatgaagaacaacctcagcagcatcctgcctgacttcaccgagagcgagaagaagttcatcaagggcaccgccgacttcttcgccctgtgcttcggccccaccctgagcttccagctgctggatccccatatgaagttcagacaactcgagagtcctaacctgcgccagctgctgagctggatcgacctggaattcaaccacccacagatcttcatcgtggagaacggctggtttgtgagcggcaccactaagcgcgacgacgcaaagtatatgtattatctgaagaaattcatcatggaaaccctgaaggccatcaagctggacggcgtggacgtgatcggatacaccgcatggagcctgatggacggcttcgagtggcaccgcggttacagcatccgccggggcctgttctacgttgacttcctgagccaggacaagatgttgctgcccaagagctccgccctgttctaccagaagttgatcgagaagaacggcttcccaccactccccgagaaccagcccctggagggcaccttcccctgcgatttcgcctggggcgtggtggacaactacatccaggtggacaccaccctgagtcagttcactgacctgaacgtgtacctttgggacgtgcaccacagcaagcgcctgataaaggtcgacggcgtggtgaccaagaagcgcaaaagctactgcgtggactttgccgccatccagccccagatcgccctgctgcaggagatgcacgtgactcacttccgcttcagcctcgactgggccctgattctgcccctgggcaaccagtcacaagtgaaccacaccattctgcagtactaccgctgtatggccagcgagctggtacgcgtgaacatcacccccgttgtggccctttggcagcccatggcccccaaccagggcctgcctcgcctgctggcccgccagggagcctgggagaatccctacaccgcactggccttcgctgaatacgcccgcctgtgcttccaggagctggggcaccacgtgaaactctggatcaccatgaacgagccctacaccagaaacatgacctacagcgccggacacaatctgctgaaggcccacgctctggcctggcacgtgtacaacgagaagtttcgccacgcccagaacggcaagatcagcatcgccctgcaggccgattggatcgagcccgcctgccccttcagccagaaggacaaggaggtggctgagcgggtgctggagttcgacatcgggtggctggctgagcctatcttcggcagcggagactacccctgggtgatgcgcgattggcttaaccagaggaacaatttcctgctgccctacttcaccgaggacgagaagaagctgatccagggcacctttgacttcctggctttgagccactataccactatcctggtggacagcgagaaggaggaccccatcaagtacaacgactacttggaggtgcaggagatgaccgacatcacctggctgaacagccctagccaggtggctgtggtgccttggggcctgcgcaaggtgctgaactggctgaagttcaagtacggcgacctgcccatgtatatcatcagcaacggcatcgacgacggcctgcacgccgaggacgaccagctgagagtgtactacatgcagaactacatcaacgaggccctcaaggcccacatcctggacggcatcaacctgtgtggctactttgcctacagcttcaacgacagaaccgccccccgcttcggcctgtacaggtacgccgccgaccagttcgaacccaaggccagcatgaagcactaccgcaaaatcatcgacagcaacggattccctggacccgagacactggagcgcttctgcccagaggagttcaccgtgtgcaccgagtgcagtttcttccacacccgcaagagcctgctggctttcattgcttttctgttttttgcttccattatttctctctccctcatcttttactacagcaagaaaggaagaagaagctacaaa

SEQ ID NO: 65 - RNA, 2937 nt, synthetic construct
  source 1..2937: mol_type = other RNA
gagcctggagatggagcccaaacatgggccagattcagcagacctcccgctcctgaagccgccggcttgtttcagggaacctttcctgacggtttcctgtgggctgtgggcagcgccgcctatcagaccgagggcggctggcaacagcacggaaaaggagccagcatctgggataccttcacccaccaccccctggccccccccggcgattcccgcaatgccagcctccctctgggagcccctagccccctgcaacctgccacaggagacgtggcctcagacagctataacaacgtgttccgcgacaccgaggcactgcgcgagctgggcgtgacccattaccgctttagcatcagctgggccagagtgctgcccaatggctctgccggcgtgcccaaccgggagggcctgaggtactaccgccgcctgctggagaggctgcgggagctgggcgtgcagcccgtggtaaccctgtaccactgggacctgccccagcgcctgcaggacgcttacggcggctgggccaaccgcgctctcgcagaccacttccgcgactacgccgagctgtgctttcgccactttggcggccaggtgaagtattggatcaccatcgataacccttacgtggtggcctggcacggatacgctacaggccgcctggcccccggcatccgcggcagccccagactgggctacctggtggcccacaacctgctgctggcccacgccaaggtgtggcacctgtacaacaccagcttccgccccacccagggtggacaggtctctattgccctgagctctcactggattaaccccaggaggatgaccgatcacagcatcaaggaatgccagaagagcctggacttcgttctgggctggttcgccaagcccgtgtttatcgacggcgactaccccgagagcatgaagaacaacctgtctagcatcctgcccgacttcaccgagagcgaaaaaaaattcatcaagggcaccgccgatttcttcgccctgtgtttcggcccaaccctgagcttccaactgctggatccccacatgaagttcagacaactcgagagtcccaacctgcgccagctgctgagctggatcgatctggaattcaaccacccccagatattcatagtggagaacggctggtttgtaagcggcactactaagcgcgatgatgcaaagtacatgtactatctgaagaagttcatcatggaaaccctgaaggccatcaagctggatggcgtggacgtgatcggatacaccgcatggagcctgatggacggcttcgagtggcaccgcggttactcaatccgcagggggttgttctacgtcgacttcctgagtcaggacaagatgttgctgccaaagagtagcgcccttttctaccagaagttgattgagaagaacggcttcccaccactccccgagaaccagcccctggagggcacctttccctgcgatttcgcttggggcgtggtggataattatattcaggtggacaccaccctgtcacagttcactgacctgaacgtgtacctgtgggacgtgcaccattccaagcgcctgatcaaggtggacggcgtggtgaccaagaagcgcaaatcctactgcgttgactttgccgccattcagccacagatcgccctgctgcaggagatgcacgtcacccacttccgcttcagcctggactgggccctcatcctgccactgggcaaccagtcccaggtgaaccacaccattctgcagtactaccgctgtatggccagcgagctggtacgcgtgaacatcacccccgtggtggccctgtggcagcccatggcccccaaccagggcctgccacgcctgctggccaggcagggggcctgggagaacccctacaccgcactcgctttcgccgaatatgccaggctgtgcttccaggagctggggcaccacgtgaagctctggatcaccatgaacgaaccctacaccagaaacatgacctactctgccggacacaatctgctgaaggcccacgccctggcctggcacgtctacaacgagaagttccgccacgcccaaaatggaaagatctctatagccctgcaggccgattggatcgagcccgcctgccccttctcacagaaggacaaggaggtggccgagcgcgtgctggagttcgacatcggctggctggccgagcccatcttcggcagcggagactacccctgggtgatgcgcgattggcttaaccagcgcaacaactttctgctgccctacttcaccgaggacgagaagaagctgatccagggcaccttcgacttcctggccctgagccactatactaccatcctggtcgacagcgagaaggaggacccaatcaagtacaacgactacctggaggtgcaggagatgaccgacatcacctggctgaacagccctagccaggtcgccgtggtgccttggggcctgcgcaaggtgctgaactggctgaagttcaagtatggcgacctgccaatgtacatcatcagcaacggcattgatgacggcctgcacgccgaggacgatcagctgagagtgtactatatgcagaactacatcaacgaggcactgaaggcccacatcctggacggcatcaacctgtgtggctactttgcatactccttcaacgacagaaccgccccccgcttcggcctgtacaggtacgctgccgatcagttcgagcccaaggccagcatgaagcactacagaaaaatcattgatagcaacgggttcccaggccccgagaccctggagcgcttctgccccgaggagttcaccgtgtgcaccgagtgcagttttttccacacccgcaagagcctgctggctttcattgcttttctgttttttgcttccattatttctctctccctcatcttttactacagcaagaaaggaagaagaagctacaaa

SEQ ID NO: 66 - RNA, 2937 nt, synthetic construct
  source 1..2937: mol_type = other RNA
gagcctggcgacggggcccagacctgggccagattcagcagaccccccgcacccgaggccgccggcctgttccagggcaccttccccgacggatttctgtgggccgtgggaagcgctgcctaccagaccgagggcggctggcaacagcacggcaagggcgccagcatctgggacaccttcacccaccatcctctggctcctcccggagacagcagaaacgccagcctgcctctgggagcccccagccccctgcagcccgccactggagacgtggccagcgactcctacaacaacgtgttccgcgacaccgaggccctgcgcgagctgggcgtgacccactaccgctttagcatcagctgggccagagtgctgcccaacggcagcgccggcgtgcccaaccgggaaggcctgagatactatcgccgcctgctggagaggctgagagagttgggcgtgcagcccgtggtgaccctgtaccactgggacctgccccagcgcctgcaggacgcctacggcggctgggccaacagggcactcgccgaccacttccgcgactacgccgagctgtgcttccgccacttcggcgggcaggtgaagtactggatcaccatcgacaacccctacgtggtggcctggcacggctacgctacaggaaggctggcccccgggatccgcggcagccccaggctgggctacctggtggcccacaacctgctgctggcacacgccaaagtgtggcacctgtataacaccagctttcgccccacccagggtggacaggtgagcattgccctgagttctcattggatcaaccccaggcgcatgaccgatcacagcatcaaggaatgccagaagagcctggacttcgtgctgggctggttcgccaagcccgtgtttatcgacggcgactaccccgagtctatgaagaacaacctcagcagcatcctgcctgacgtcaccgagagcgagaagaagttcatcaagggcaccgccgacttcttcgccctgagcttcggccccaccctgagcttccagctgctggatccccatatgaagttcagacaactcgagagtcctaacctgcgccagctgctgagctggatcgacctggaattcaaccacccacagatcttcatcgtggagaacggctggtttgtgagcggcaccactaagcgcgacgacgcaaagtatatgtattatctgaagaaattcatcatggaaaccctgaaggccatcaagctggacggcgtggacgtgatcggatacaccgcatggagcctgatggacggcttcgagtggcaccgcggttacagcatccgccggggcctgttctacgttgacttcctgagccaggacaagatgttgctgcccaagagctccgccctgttctaccagaagttgatcgagaagaacggcttcccaccactccccgagaaccagcccctggagggcaccttcccctgcgatttcgcctggggcgtggtggacaactacatccaggtggacaccaccctgagtcagttcactgacctgaacgtgtacctttgggacgtgcaccacagcaagcgcctgataaaggtcgacggcgtggtgaccaagaagcgcaaaagctactgcgtggactttgccgccatccagccccagatcgccctgctgcaggagatgcacgtgactcacttccgcttcagcctcgactgggccctgattctgcccctgggcaaccagtcacaagtgaaccacaccattctgcagtactaccgctgtatggccagcgagctggtacgcgtgaacatcacccccgttgtggccctttggcagcccatggcccccaaccagggcctgcctcgcctgctggcccgccagggagcctgggagaatccctacaccgcactggccttcgctgaatacgcccgcctgtgcttccaggagctggggcaccacgtgaaactctggatcaccatgaacgagccctacaccagaaacatgacctacagcgccggacacaatctgctgaaggcccacgctctggcctggcacgtgtacaacgagaagtttcgccacgcccagaacggcaagatcagcatcgccctgcaggccgattggatcgagcccgcctgccccttcagccagaaggacaaggaggtggctgagcgggtgctggagttcgacatcgggtggctggctgagcctatcttcggcagcggagactacccctgggtgatgcgcgattggcttaaccagaggaacaatttcctgctgccctacttcaccgaggacgagaagaagctgatccagggcacctttgacttcctggctttgagccactataccactatcctggtggacagcgagaaggaggaccccatcaagtacaacgactacttggaggtgcaggagatgaccgacatcacctggctgaacagccctagccaggtggctgtggtgccttggggcctgcgcaaggtgctgaactggctgaagttcaagtacggcgacctgcccatgtatatcatcagcaacggcatcgacgacggcctgcacgccgaggacgaccagctgagagtgtactacatgcagaactacatcaacgaggccctcaaggcccacatcctggacggcatcaacctgtgtggctactttgcctacagcttcaacgacagaaccgccccccgcttcggcctgtacaggtacgccgccgaccagttcgaacccaaggccagcatgaagcactaccgcaaaatcatcgacagcaacggattccctggacccgagacactggagcgcttctgcccagaggagttcaccgtgtgcaccgagtgcagtttcttccacacccgcaagagcctgctggctttcattgcttttctgttttttgcttccattatttctctctccctcatcttttactacagcaagaaaggaagaagaagctacaaa

SEQ ID NO: 67 - RNA, 2937 nt, synthetic construct
  source 1..2937: mol_type = other RNA
gagcctggagatggagcccaaacatgggccagattcagcagacctcccgctcctgaagccgccggcttgtttcagggaacctttcctgacggtttcctgtgggctgtgggcagcgccgcctatcagaccgagggcggctggcaacagcacggaaaaggagccagcatctgggataccttcacccaccaccccctggccccccccggcgattcccgcaatgccagcctccctctgggagcccctagccccctgcaacctgccacaggagacgtggcctcagacagctataacaacgtgttccgcgacaccgaggcactgcgcgagctgggcgtgacccattaccgctttagcatcagctgggccagagtgctgcccaatggctctgccggcgtgcccaaccgggagggcctgaggtactaccgccgcctgctggagaggctgcgggagctgggcgtgcagcccgtggtaaccctgtaccactgggacctgccccagcgcctgcaggacgcttacggcggctgggccaaccgcgctctcgcagaccacttccgcgactacgccgagctgtgctttcgccactttggcggccaggtgaagtattggatcaccatcgataacccttacgtggtggcctggcacggatacgctacaggccgcctggcccccggcatccgcggcagccccagactgggctacctggtggcccacaacctgctgctggcccacgccaaggtgtggcacctgtacaacaccagcttccgccccacccagggtggacaggtctctattgccctgagctctcactggattaaccccaggaggatgaccgatcacagcatcaaggaatgccagaagagcctggacttcgttctgggctggttcgccaagcccgtgtttatcgacggcgactaccccgagagcatgaagaacaacctgtctagcatcctgcccgacgtcaccgagagcgaaaaaaaattcatcaagggcaccgccgatttcttcgccctgagcttcggcccaaccctgagcttccaactgctggatccccacatgaagttcagacaactcgagagtcccaacctgcgccagctgctgagctggatcgatctggaattcaaccacccccagatattcatagtggagaacggctggtttgtaagcggcactactaagcgcgatgatgcaaagtacatgtactatctgaagaagttcatcatggaaaccctgaaggccatcaagctggatggcgtggacgtgatcggatacaccgcatggagcctgatggacggcttcgagtggcaccgcggttactcaatccgcagggggttgttctacgtcgacttcctgagtcaggacaagatgttgctgccaaagagtagcgcccttttctaccagaagttgattgagaagaacggcttcccaccactccccgagaaccagcccctggagggcacctttccctgcgatttcgcttggggcgtggtggataattatattcaggtggacaccaccctgtcacagttcactgacctgaacgtgtacctgtgggacgtgcaccattccaagcgcctgatcaaggtggacggcgtggtgaccaagaagcgcaaatcctactgcgttgactttgccgccattcagccacagatcgccctgctgcaggagatgcacgtcacccacttccgcttcagcctggactgggccctcatcctgccactgggcaaccagtcccaggtgaaccacaccattctgcagtactaccgctgtatggccagcgagctggtacgcgtgaacatcacccccgtggtggccctgtggcagcccatggcccccaaccagggcctgccacgcctgctggccaggcagggggcctgggagaacccctacaccgcactcgctttcgccgaatatgccaggctgtgcttccaggagctggggcaccacgtgaagctctggatcaccatgaacgaaccctacaccagaaacatgacctactctgccggacacaatctgctgaaggcccacgccctggcctggcacgtctacaacgagaagttccgccacgcccaaaatggaaagatctctatagccctgcaggccgattggatcgagcccgcctgccccttctcacagaaggacaaggaggtggccgagcgcgtgctggagttcgacatcggctggctggccgagcccatcttcggcagcggagactacccctgggtgatgcgcgattggcttaaccagcgcaacaactttctgctgccctacttcaccgaggacgagaagaagctgatccagggcaccttcgacttcctggccctgagccactatactaccatcctggtcgacagcgagaaggaggacccaatcaagtacaacgactacctggaggtgcaggagatgaccgacatcacctggctgaacagccctagccaggtcgccgtggtgccttggggcctgcgcaaggtgctgaactggctgaagttcaagtatggcgacctgccaatgtacatcatcagcaacggcattgatgacggcctgcacgccgaggacgatcagctgagagtgtactatatgcagaactacatcaacgaggcactgaaggcccacatcctggacggcatcaacctgtgtggctactttgcatactccttcaacgacagaaccgccccccgcttcggcctgtacaggtacgctgccgatcagttcgagcccaaggccagcatgaagcactacagaaaaatcattgatagcaacgggttcccaggccccgagaccctggagcgcttctgccccgaggagttcaccgtgtgcaccgagtgcagttttttccacacccgcaagagcctgctggctttcattgcttttctgttttttgcttccattatttctctctccctcatcttttactacagcaagaaaggaagaagaagctacaaa

SEQ ID NO: 68 - RNA, 3039 nt, synthetic construct
  source 1..3039: mol_type = other RNA
atgcccgctagcgccccaccgagaagaccgcggccgccaccgccatcgctgtcgctgctgctggtgctgctgggactgggcggaagaagactgcgtgcggagcctggcgacggggcccagacctgggccagattcagcagaccccccgcacccgaggccgccggcctgttccagggcaccttccccgacggatttctgtgggccgtgggaagcgctgcctaccagaccgagggcggctggcaacagcacggcaagggcgccagcatctgggacaccttcacccaccatcctctggctcctcccggagacagcagaaacgccagcctgcctctgggagcccccagccccctgcagcccgccactggagacgtggccagcgactcctacaacaacgtgttccgcgacaccgaggccctgcgcgagctgggcgtgacccactaccgctttagcatcagctgggccagagtgctgcccaacggcagcgccggcgtgcccaaccgggaaggcctgagatactatcgccgcctgctggagaggctgagagagttgggcgtgcagcccgtggtgaccctgtaccactgggacctgccccagcgcctgcaggacgcctacggcggctgggccaacagggcactcgccgaccacttccgcgactacgccgagctgtgcttccgccacttcggcgggcaggtgaagtactggatcaccatcgacaacccctacgtggtggcctggcacggctacgctacaggaaggctggcccccgggatccgcggcagccccaggctgggctacctggtggcccacaacctgctgctggcacacgccaaagtgtggcacctgtataacaccagctttcgccccacccagggtggacaggtgagcattgccctgagttctcattggatcaaccccaggcgcatgaccgatcacagcatcaaggaatgccagaagagcctggacttcgtgctgggctggttcgccaagcccgtgtttatcgacggcgactaccccgagtctatgaagaacaacctcagcagcatcctgcctgacttcaccgagagcgagaagaagttcatcaagggcaccgccgacttcttcgccctgtgcttcggccccaccctgagcttccagctgctggatccccatatgaagttcagacaactcgagagtcctaacctgcgccagctgctgagctggatcgacctggaattcaaccacccacagatcttcatcgtggagaacggctggtttgtgagcggcaccactaagcgcgacgacgcaaagtatatgtattatctgaagaaattcatcatggaaaccctgaaggccatcaagctggacggcgtggacgtgatcggatacaccgcatggagcctgatggacggcttcgagtggcaccgcggttacagcatccgccggggcctgttctacgttgacttcctgagccaggacaagatgttgctgcccaagagctccgccctgttctaccagaagttgatcgagaagaacggcttcccaccactccccgagaaccagcccctggagggcaccttcccctgcgatttcgcctggggcgtggtggacaactacatccaggtggacaccaccctgagtcagttcactgacctgaacgtgtacctttgggacgtgcaccacagcaagcgcctgataaaggtcgacggcgtggtgaccaagaagcgcaaaagctactgcgtggactttgccgccatccagccccagatcgccctgctgcaggagatgcacgtgactcacttccgcttcagcctcgactgggccctgattctgcccctgggcaaccagtcacaagtgaaccacaccattctgcagtactaccgctgtatggccagcgagctggtacgcgtgaacatcacccccgttgtggccctttggcagcccatggcccccaaccagggcctgcctcgcctgctggcccgccagggagcctgggagaatccctacaccgcactggccttcgctgaatacgcccgcctgtgcttccaggagctggggcaccacgtgaaactctggatcaccatgaacgagccctacaccagaaacatgacctacagcgccggacacaatctgctgaaggcccacgctctggcctggcacgtgtacaacgagaagtttcgccacgcccagaacggcaagatcagcatcgccctgcaggccgattggatcgagcccgcctgccccttcagccagaaggacaaggaggtggctgagcgggtgctggagttcgacatcgggtggctggctgagcctatcttcggcagcggagactacccctgggtgatgcgcgattggcttaaccagaggaacaatttcctgctgccctacttcaccgaggacgagaagaagctgatccagggcacctttgacttcctggctttgagccactataccactatcctggtggacagcgagaaggaggaccccatcaagtacaacgactacttggaggtgcaggagatgaccgacatcacctggctgaacagccctagccaggtggctgtggtgccttggggcctgcgcaaggtgctgaactggctgaagttcaagtacggcgacctgcccatgtatatcatcagcaacggcatcgacgacggcctgcacgccgaggacgaccagctgagagtgtactacatgcagaactacatcaacgaggccctcaaggcccacatcctggacggcatcaacctgtgtggctactttgcctacagcttcaacgacagaaccgccccccgcttcggcctgtacaggtacgccgccgaccagttcgaacccaaggccagcatgaagcactaccgcaaaatcatcgacagcaacggattccctggacccgagacactggagcgcttctgcccagaggagttcaccgtgtgcaccgagtgcagtttcttccacacccgcaagagcctgctggctttcattgcttttctgttttttgcttccattatttctctctccctcatcttttactacagcaagaaaggaagaagaagctacaaatga

SEQ ID NO: 69 - RNA, 3039 nt, synthetic construct
  source 1..3039: mol_type = other RNA
atgcccgctagcgccccaccgagaagaccgcggccgccaccgccatcgctgtcgctgctgctggtgctgctgggactgggcggaagaagactgcgtgcggagcctggagatggagcccaaacatgggccagattcagcagacctcccgctcctgaagccgccggcttgtttcagggaacctttcctgacggtttcctgtgggctgtgggcagcgccgcctatcagaccgagggcggctggcaacagcacggaaaaggagccagcatctgggataccttcacccaccaccccctggccccccccggcgattcccgcaatgccagcctccctctgggagcccctagccccctgcaacctgccacaggagacgtggcctcagacagctataacaacgtgttccgcgacaccgaggcactgcgcgagctgggcgtgacccattaccgctttagcatcagctgggccagagtgctgcccaatggctctgccggcgtgcccaaccgggagggcctgaggtactaccgccgcctgctggagaggctgcgggagctgggcgtgcagcccgtggtaaccctgtaccactgggacctgccccagcgcctgcaggacgcttacggcggctgggccaaccgcgctctcgcagaccacttccgcgactacgccgagctgtgctttcgccactttggcggccaggtgaagtattggatcaccatcgataacccttacgtggtggcctggcacggatacgctacaggccgcctggcccccggcatccgcggcagccccagactgggctacctggtggcccacaacctgctgctggcccacgccaaggtgtggcacctgtacaacaccagcttccgccccacccagggtggacaggtctctattgccctgagctctcactggattaaccccaggaggatgaccgatcacagcatcaaggaatgccagaagagcctggacttcgttctgggctggttcgccaagcccgtgtttatcgacggcgactaccccgagagcatgaagaacaacctgtctagcatcctgcccgacttcaccgagagcgaaaaaaaattcatcaagggcaccgccgatttcttcgccctgtgtttcggcccaaccctgagcttccaactgctggatccccacatgaagttcagacaactcgagagtcccaacctgcgccagctgctgagctggatcgatctggaattcaaccacccccagatattcatagtggagaacggctggtttgtaagcggcactactaagcgcgatgatgcaaagtacatgtactatctgaagaagttcatcatggaaaccctgaaggccatcaagctggatggcgtggacgtgatcggatacaccgcatggagcctgatggacggcttcgagtggcaccgcggttactcaatccgcagggggttgttctacgtcgacttcctgagtcaggacaagatgttgctgccaaagagtagcgcccttttctaccagaagttgattgagaagaacggcttcccaccactccccgagaaccagcccctggagggcacctttccctgcgatttcgcttggggcgtggtggataattatattcaggtggacaccaccctgtcacagttcactgacctgaacgtgtacctgtgggacgtgcaccattccaagcgcctgatcaaggtggacggcgtggtgaccaagaagcgcaaatcctactgcgttgactttgccgccattcagccacagatcgccctgctgcaggagatgcacgtcacccacttccgcttcagcctggactgggccctcatcctgccactgggcaaccagtcccaggtgaaccacaccattctgcagtactaccgctgtatggccagcgagctggtacgcgtgaacatcacccccgtggtggccctgtggcagcccatggcccccaaccagggcctgccacgcctgctggccaggcagggggcctgggagaacccctacaccgcactcgctttcgccgaatatgccaggctgtgcttccaggagctggggcaccacgtgaagctctggatcaccatgaacgaaccctacaccagaaacatgacctactctgccggacacaatctgctgaaggcccacgccctggcctggcacgtctacaacgagaagttccgccacgcccaaaatggaaagatctctatagccctgcaggccgattggatcgagcccgcctgccccttctcacagaaggacaaggaggtggccgagcgcgtgctggagttcgacatcggctggctggccgagcccatcttcggcagcggagactacccctgggtgatgcgcgattggcttaaccagcgcaacaactttctgctgccctacttcaccgaggacgagaagaagctgatccagggcaccttcgacttcctggccctgagccactatactaccatcctggtcgacagcgagaaggaggacccaatcaagtacaacgactacctggaggtgcaggagatgaccgacatcacctggctgaacagccctagccaggtcgccgtggtgccttggggcctgcgcaaggtgctgaactggctgaagttcaagtatggcgacctgccaatgtacatcatcagcaacggcattgatgacggcctgcacgccgaggacgatcagctgagagtgtactatatgcagaactacatcaacgaggcactgaaggcccacatcctggacggcatcaacctgtgtggctactttgcatactccttcaacgacagaaccgccccccgcttcggcctgtacaggtacgctgccgatcagttcgagcccaaggccagcatgaagcactacagaaaaatcattgatagcaacgggttcccaggccccgagaccctggagcgcttctgccccgaggagttcaccgtgtgcaccgagtgcagttttttccacacccgcaagagcctgctggctttcattgcttttctgttttttgcttccattatttctctctccctcatcttttactacagcaagaaaggaagaagaagctacaaatga

SEQ ID NO: 70 - RNA, 3039 nt, synthetic construct
  source 1..3039: mol_type = other RNA
atgcccgctagcgccccaccgagaagaccgcggccgccaccgccatcgctgtcgctgctgctggtgctgctgggactgggcggaagaagactgcgtgcggagcctggcgacggggcccagacctgggccagattcagcagaccccccgcacccgaggccgccggcctgttccagggcaccttccccgacggatttctgtgggccgtgggaagcgctgcctaccagaccgagggcggctggcaacagcacggcaagggcgccagcatctgggacaccttcacccaccatcctctggctcctcccggagacagcagaaacgccagcctgcctctgggagcccccagccccctgcagcccgccactggagacgtggccagcgactcctacaacaacgtgttccgcgacaccgaggccctgcgcgagctgggcgtgacccactaccgctttagcatcagctgggccagagtgctgcccaacggcagcgccggcgtgcccaaccgggaaggcctgagatactatcgccgcctgctggagaggctgagagagttgggcgtgcagcccgtggtgaccctgtaccactgggacctgccccagcgcctgcaggacgcctacggcggctgggccaacagggcactcgccgaccacttccgcgactacgccgagctgtgcttccgccacttcggcgggcaggtgaagtactggatcaccatcgacaacccctacgtggtggcctggcacggctacgctacaggaaggctggcccccgggatccgcggcagccccaggctgggctacctggtggcccacaacctgctgctggcacacgccaaagtgtggcacctgtataacaccagctttcgccccacccagggtggacaggtgagcattgccctgagttctcattggatcaaccccaggcgcatgaccgatcacagcatcaaggaatgccagaagagcctggacttcgtgctgggctggttcgccaagcccgtgtttatcgacggcgactaccccgagtctatgaagaacaacctcagcagcatcctgcctgacgtcaccgagagcgagaagaagttcatcaagggcaccgccgacttcttcgccctgagcttcggccccaccctgagcttccagctgctggatccccatatgaagttcagacaactcgagagtcctaacctgcgccagctgctgagctggatcgacctggaattcaaccacccacagatcttcatcgtggagaacggctggtttgtgagcggcaccactaagcgcgacgacgcaaagtatatgtattatctgaagaaattcatcatggaaaccctgaaggccatcaagctggacggcgtggacgtgatcggatacaccgcatggagcctgatggacggcttcgagtggcaccgcggttacagcatccgccggggcctgttctacgttgacttcctgagccaggacaagatgttgctgcccaagagctccgccctgttctaccagaagttgatcgagaagaacggcttcccaccactccccgagaaccagcccctggagggcaccttcccctgcgatttcgcctggggcgtggtggacaactacatccaggtggacaccaccctgagtcagttcactgacctgaacgtgtacctttgggacgtgcaccacagcaagcgcctgataaaggtcgacggcgtggtgaccaagaagcgcaaaagctactgcgtggactttgccgccatccagccccagatcgccctgctgcaggagatgcacgtgactcacttccgcttcagcctcgactgggccctgattctgcccctgggcaaccagtcacaagtgaaccacaccattctgcagtactaccgctgtatggccagcgagctggtacgcgtgaacatcacccccgttgtggccctttggcagcccatggcccccaaccagggcctgcctcgcctgctggcccgccagggagcctgggagaatccctacaccgcactggccttcgctgaatacgcccgcctgtgcttccaggagctggggcaccacgtgaaactctggatcaccatgaacgagccctacaccagaaacatgacctacagcgccggacacaatctgctgaaggcccacgctctggcctggcacgtgtacaacgagaagtttcgccacgcccagaacggcaagatcagcatcgccctgcaggccgattggatcgagcccgcctgccccttcagccagaaggacaaggaggtggctgagcgggtgctggagttcgacatcgggtggctggctgagcctatcttcggcagcggagactacccctgggtgatgcgcgattggcttaaccagaggaacaatttcctgctgccctacttcaccgaggacgagaagaagctgatccagggcacctttgacttcctggctttgagccactataccactatcctggtggacagcgagaaggaggaccccatcaagtacaacgactacttggaggtgcaggagatgaccgacatcacctggctgaacagccctagccaggtggctgtggtgccttggggcctgcgcaaggtgctgaactggctgaagttcaagtacggcgacctgcccatgtatatcatcagcaacggcatcgacgacggcctgcacgccgaggacgaccagctgagagtgtactacatgcagaactacatcaacgaggccctcaaggcccacatcctggacggcatcaacctgtgtggctactttgcctacagcttcaacgacagaaccgccccccgcttcggcctgtacaggtacgccgccgaccagttcgaacccaaggccagcatgaagcactaccgcaaaatcatcgacagcaacggattccctggacccgagacactggagcgcttctgcccagaggagttcaccgtgtgcaccgagtgcagtttcttccacacccgcaagagcctgctggctttcattgcttttctgttttttgcttccattatttctctctccctcatcttttactacagcaagaaaggaagaagaagctacaaatga

SEQ ID NO: 71 - RNA, 3039 nt, synthetic construct
  source 1..3039: mol_type = other RNA
atgcccgctagcgccccaccgagaagaccgcggccgccaccgccatcgctgtcgctgctgctggtgctgctgggactgggcggaagaagactgcgtgcggagcctggagatggagcccaaacatgggccagattcagcagacctcccgctcctgaagccgccggcttgtttcagggaacctttcctgacggtttcctgtgggctgtgggcagcgccgcctatcagaccgagggcggctggcaacagcacggaaaaggagccagcatctgggataccttcacccaccaccccctggccccccccggcgattcccgcaatgccagcctccctctgggagcccctagccccctgcaacctgccacaggagacgtggcctcagacagctataacaacgtgttccgcgacaccgaggcactgcgcgagctgggcgtgacccattaccgctttagcatcagctgggccagagtgctgcccaatggctctgccggcgtgcccaaccgggagggcctgaggtactaccgccgcctgctggagaggctgcgggagctgggcgtgcagcccgtggtaaccctgtaccactgggacctgccccagcgcctgcaggacgcttacggcggctgggccaaccgcgctctcgcagaccacttccgcgactacgccgagctgtgctttcgccactttggcggccaggtgaagtattggatcaccatcgataacccttacgtggtggcctggcacggatacgctacaggccgcctggcccccggcatccgcggcagccccagactgggctacctggtggcccacaacctgctgctggcccacgccaaggtgtggcacctgtacaacaccagcttccgccccacccagggtggacaggtctctattgccctgagctctcactggattaaccccaggaggatgaccgatcacagcatcaaggaatgccagaagagcctggacttcgttctgggctggttcgccaagcccgtgtttatcgacggcgactaccccgagagcatgaagaacaacctgtctagcatcctgcccgacgtcaccgagagcgaaaaaaaattcatcaagggcaccgccgatttcttcgccctgagcttcggcccaaccctgagcttccaactgctggatccccacatgaagttcagacaactcgagagtcccaacctgcgccagctgctgagctggatcgatctggaattcaaccacccccagatattcatagtggagaacggctggtttgtaagcggcactactaagcgcgatgatgcaaagtacatgtactatctgaagaagttcatcatggaaaccctgaaggccatcaagctggatggcgtggacgtgatcggatacaccgcatggagcctgatggacggcttcgagtggcaccgcggttactcaatccgcagggggttgttctacgtcgacttcctgagtcaggacaagatgttgctgccaaagagtagcgcccttttctaccagaagttgattgagaagaacggcttcccaccactccccgagaaccagcccctggagggcacctttccctgcgatttcgcttggggcgtggtggataattatattcaggtggacaccaccctgtcacagttcactgacctgaacgtgtacctgtgggacgtgcaccattccaagcgcctgatcaaggtggacggcgtggtgaccaagaagcgcaaatcctactgcgttgactttgccgccattcagccacagatcgccctgctgcaggagatgcacgtcacccacttccgcttcagcctggactgggccctcatcctgccactgggcaaccagtcccaggtgaaccacaccattctgcagtactaccgctgtatggccagcgagctggtacgcgtgaacatcacccccgtggtggccctgtggcagcccatggcccccaaccagggcctgccacgcctgctggccaggcagggggcctgggagaacccctacaccgcactcgctttcgccgaatatgccaggctgtgcttccaggagctggggcaccacgtgaagctctggatcaccatgaacgaaccctacaccagaaacatgacctactctgccggacacaatctgctgaaggcccacgccctggcctggcacgtctacaacgagaagttccgccacgcccaaaatggaaagatctctatagccctgcaggccgattggatcgagcccgcctgccccttctcacagaaggacaaggaggtggccgagcgcgtgctggagttcgacatcggctggctggccgagcccatcttcggcagcggagactacccctgggtgatgcgcgattggcttaaccagcgcaacaactttctgctgccctacttcaccgaggacgagaagaagctgatccagggcaccttcgacttcctggccctgagccactatactaccatcctggtcgacagcgagaaggaggacccaatcaagtacaacgactacctggaggtgcaggagatgaccgacatcacctggctgaacagccctagccaggtcgccgtggtgccttggggcctgcgcaaggtgctgaactggctgaagttcaagtatggcgacctgccaatgtacatcatcagcaacggcattgatgacggcctgcacgccgaggacgatcagctgagagtgtactatatgcagaactacatcaacgaggcactgaaggcccacatcctggacggcatcaacctgtgtggctactttgcatactccttcaacgacagaaccgccccccgcttcggcctgtacaggtacgctgccgatcagttcgagcccaaggccagcatgaagcactacagaaaaatcattgatagcaacgggttcccaggccccgagaccctggagcgcttctgccccgaggagttcaccgtgtgcaccgagtgcagttttttccacacccgcaagagcctgctggctttcattgcttttctgttttttgcttccattatttctctctccctcatcttttactacagcaagaaaggaagaagaagctacaaatga

SEQ ID NO: 72 - RNA, 3342 nt, synthetic construct
  source 1..3342: mol_type = other RNA
gggagacataaaccctggcgcgctcgcggcccggcactcttctggtccccacagactcagagagaacccaccatgcccgctagcgccccaccgagaagaccgcggccgccaccgccatcgctgtcgctgctgctggtgctgctgggactgggcggaagaagactgcgtgcggagcctggcgacggggcccagacctgggccagattcagcagaccccccgcacccgaggccgccggcctgttccagggcaccttccccgacggatttctgtgggccgtgggaagcgctgcctaccagaccgagggcggctggcaacagcacggcaagggcgccagcatctgggacaccttcacccaccatcctctggctcctcccggagacagcagaaacgccagcctgcctctgggagcccccagccccctgcagcccgccactggagacgtggccagcgactcctacaacaacgtgttccgcgacaccgaggccctgcgcgagctgggcgtgacccactaccgctttagcatcagctgggccagagtgctgcccaacggcagcgccggcgtgcccaaccgggaaggcctgagatactatcgccgcctgctggagaggctgagagagttgggcgtgcagcccgtggtgaccctgtaccactgggacctgccccagcgcctgcaggacgcctacggcggctgggccaacagggcactcgccgaccacttccgcgactacgccgagctgtgcttccgccacttcggcgggcaggtgaagtactggatcaccatcgacaacccctacgtggtggcctggcacggctacgctacaggaaggctggcccccgggatccgcggcagccccaggctgggctacctggtggcccacaacctgctgctggcacacgccaaagtgtggcacctgtataacaccagctttcgccccacccagggtggacaggtgagcattgccctgagttctcattggatcaaccccaggcgcatgaccgatcacagcatcaaggaatgccagaagagcctggacttcgtgctgggctggttcgccaagcccgtgtttatcgacggcgactaccccgagtctatgaagaacaacctcagcagcatcctgcctgacttcaccgagagcgagaagaagttcatcaagggcaccgccgacttcttcgccctgtgcttcggccccaccctgagcttccagctgctggatccccatatgaagttcagacaactcgagagtcctaacctgcgccagctgctgagctggatcgacctggaattcaaccacccacagatcttcatcgtggagaacggctggtttgtgagcggcaccactaagcgcgacgacgcaaagtatatgtattatctgaagaaattcatcatggaaaccctgaaggccatcaagctggacggcgtggacgtgatcggatacaccgcatggagcctgatggacggcttcgagtggcaccgcggttacagcatccgccggggcctgttctacgttgacttcctgagccaggacaagatgttgctgcccaagagctccgccctgttctaccagaagttgatcgagaagaacggcttcccaccactccccgagaaccagcccctggagggcaccttcccctgcgatttcgcctggggcgtggtggacaactacatccaggtggacaccaccctgagtcagttcactgacctgaacgtgtacctttgggacgtgcaccacagcaagcgcctgataaaggtcgacggcgtggtgaccaagaagcgcaaaagctactgcgtggactttgccgccatccagccccagatcgccctgctgcaggagatgcacgtgactcacttccgcttcagcctcgactgggccctgattctgcccctgggcaaccagtcacaagtgaaccacaccattctgcagtactaccgctgtatggccagcgagctggtacgcgtgaacatcacccccgttgtggccctttggcagcccatggcccccaaccagggcctgcctcgcctgctggcccgccagggagcctgggagaatccctacaccgcactggccttcgctgaatacgcccgcctgtgcttccaggagctggggcaccacgtgaaactctggatcaccatgaacgagccctacaccagaaacatgacctacagcgccggacacaatctgctgaaggcccacgctctggcctggcacgtgtacaacgagaagtttcgccacgcccagaacggcaagatcagcatcgccctgcaggccgattggatcgagcccgcctgccccttcagccagaaggacaaggaggtggctgagcgggtgctggagttcgacatcgggtggctggctgagcctatcttcggcagcggagactacccctgggtgatgcgcgattggcttaaccagaggaacaatttcctgctgccctacttcaccgaggacgagaagaagctgatccagggcacctttgacttcctggctttgagccactataccactatcctggtggacagcgagaaggaggaccccatcaagtacaacgactacttggaggtgcaggagatgaccgacatcacctggctgaacagccctagccaggtggctgtggtgccttggggcctgcgcaaggtgctgaactggctgaagttcaagtacggcgacctgcccatgtatatcatcagcaacggcatcgacgacggcctgcacgccgaggacgaccagctgagagtgtactacatgcagaactacatcaacgaggccctcaaggcccacatcctggacggcatcaacctgtgtggctactttgcctacagcttcaacgacagaaccgccccccgcttcggcctgtacaggtacgccgccgaccagttcgaacccaaggccagcatgaagcactaccgcaaaatcatcgacagcaacggattccctggacccgagacactggagcgcttctgcccagaggagttcaccgtgtgcaccgagtgcagtttcttccacacccgcaagagcctgctggctttcattgcttttctgttttttgcttccattatttctctctccctcatcttttactacagcaagaaaggaagaagaagctacaaatgagctggagcctcggtggccatgcttcttgccccttgggcctccccccagcccctcctccccttcctgcacccgtacccccgtggtctttgaataaagtctgagtgggcggcaaaaaaaaaaaaaaaaaaaaaaaaaaaaaaaaaaaaaaaaaaaaaaaaaaaaaaaaaaaaaaaaaaaaaaaaaaaaaaaaaaaaaaaaaaaaaaaaaaaaaaaaaaaaaaaaaaaaaaaaa

SEQ ID NO: 73 - RNA, 3342 nt, synthetic construct
  source 1..3342: mol_type = other RNA
gggagacataaaccctggcgcgctcgcggcccggcactcttctggtccccacagactcagagagaacccaccatgcccgctagcgccccaccgagaagaccgcggccgccaccgccatcgctgtcgctgctgctggtgctgctgggactgggcggaagaagactgcgtgcggagcctggagatggagcccaaacatgggccagattcagcagacctcccgctcctgaagccgccggcttgtttcagggaacctttcctgacggtttcctgtgggctgtgggcagcgccgcctatcagaccgagggcggctggcaacagcacggaaaaggagccagcatctgggataccttcacccaccaccccctggccccccccggcgattcccgcaatgccagcctccctctgggagcccctagccccctgcaacctgccacaggagacgtggcctcagacagctataacaacgtgttccgcgacaccgaggcactgcgcgagctgggcgtgacccattaccgctttagcatcagctgggccagagtgctgcccaatggctctgccggcgtgcccaaccgggagggcctgaggtactaccgccgcctgctggagaggctgcgggagctgggcgtgcagcccgtggtaaccctgtaccactgggacctgccccagcgcctgcaggacgcttacggcggctgggccaaccgcgctctcgcagaccacttccgcgactacgccgagctgtgctttcgccactttggcggccaggtgaagtattggatcaccatcgataacccttacgtggtggcctggcacggatacgctacaggccgcctggcccccggcatccgcggcagccccagactgggctacctggtggcccacaacctgctgctggcccacgccaaggtgtggcacctgtacaacaccagcttccgccccacccagggtggacaggtctctattgccctgagctctcactggattaaccccaggaggatgaccgatcacagcatcaaggaatgccagaagagcctggacttcgttctgggctggttcgccaagcccgtgtttatcgacggcgactaccccgagagcatgaagaacaacctgtctagcatcctgcccgacttcaccgagagcgaaaaaaaattcatcaagggcaccgccgatttcttcgccctgtgtttcggcccaaccctgagcttccaactgctggatccccacatgaagttcagacaactcgagagtcccaacctgcgccagctgctgagctggatcgatctggaattcaaccacccccagatattcatagtggagaacggctggtttgtaagcggcactactaagcgcgatgatgcaaagtacatgtactatctgaagaagttcatcatggaaaccctgaaggccatcaagctggatggcgtggacgtgatcggatacaccgcatggagcctgatggacggcttcgagtggcaccgcggttactcaatccgcagggggttgttctacgtcgacttcctgagtcaggacaagatgttgctgccaaagagtagcgcccttttctaccagaagttgattgagaagaacggcttcccaccactccccgagaaccagcccctggagggcacctttccctgcgatttcgcttggggcgtggtggataattatattcaggtggacaccaccctgtcacagttcactgacctgaacgtgtacctgtgggacgtgcaccattccaagcgcctgatcaaggtggacggcgtggtgaccaagaagcgcaaatcctactgcgttgactttgccgccattcagccacagatcgccctgctgcaggagatgcacgtcacccacttccgcttcagcctggactgggccctcatcctgccactgggcaaccagtcccaggtgaaccacaccattctgcagtactaccgctgtatggccagcgagctggtacgcgtgaacatcacccccgtggtggccctgtggcagcccatggcccccaaccagggcctgccacgcctgctggccaggcagggggcctgggagaacccctacaccgcactcgctttcgccgaatatgccaggctgtgcttccaggagctggggcaccacgtgaagctctggatcaccatgaacgaaccctacaccagaaacatgacctactctgccggacacaatctgctgaaggcccacgccctggcctggcacgtctacaacgagaagttccgccacgcccaaaatggaaagatctctatagccctgcaggccgattggatcgagcccgcctgccccttctcacagaaggacaaggaggtggccgagcgcgtgctggagttcgacatcggctggctggccgagcccatcttcggcagcggagactacccctgggtgatgcgcgattggcttaaccagcgcaacaactttctgctgccctacttcaccgaggacgagaagaagctgatccagggcaccttcgacttcctggccctgagccactatactaccatcctggtcgacagcgagaaggaggacccaatcaagtacaacgactacctggaggtgcaggagatgaccgacatcacctggctgaacagccctagccaggtcgccgtggtgccttggggcctgcgcaaggtgctgaactggctgaagttcaagtatggcgacctgccaatgtacatcatcagcaacggcattgatgacggcctgcacgccgaggacgatcagctgagagtgtactatatgcagaactacatcaacgaggcactgaaggcccacatcctggacggcatcaacctgtgtggctactttgcatactccttcaacgacagaaccgccccccgcttcggcctgtacaggtacgctgccgatcagttcgagcccaaggccagcatgaagcactacagaaaaatcattgatagcaacgggttcccaggccccgagaccctggagcgcttctgccccgaggagttcaccgtgtgcaccgagtgcagttttttccacacccgcaagagcctgctggctttcattgcttttctgttttttgcttccattatttctctctccctcatcttttactacagcaagaaaggaagaagaagctacaaatgagctggagcctcggtggccatgcttcttgccccttgggcctccccccagcccctcctccccttcctgcacccgtacccccgtggtctttgaataaagtctgagtgggcggcaaaaaaaaaaaaaaaaaaaaaaaaaaaaaaaaaaaaaaaaaaaaaaaaaaaaaaaaaaaaaaaaaaaaaaaaaaaaaaaaaaaaaaaaaaaaaaaaaaaaaaaaaaaaaaaaaaaaaaaaa

SEQ ID NO: 74 - RNA, 3342 nt, synthetic construct
  source 1..3342: mol_type = other RNA
gggagacataaaccctggcgcgctcgcggcccggcactcttctggtccccacagactcagagagaacccaccatgcccgctagcgccccaccgagaagaccgcggccgccaccgccatcgctgtcgctgctgctggtgctgctgggactgggcggaagaagactgcgtgcggagcctggcgacggggcccagacctgggccagattcagcagaccccccgcacccgaggccgccggcctgttccagggcaccttccccgacggatttctgtgggccgtgggaagcgctgcctaccagaccgagggcggctggcaacagcacggcaagggcgccagcatctgggacaccttcacccaccatcctctggctcctcccggagacagcagaaacgccagcctgcctctgggagcccccagccccctgcagcccgccactggagacgtggccagcgactcctacaacaacgtgttccgcgacaccgaggccctgcgcgagctgggcgtgacccactaccgctttagcatcagctgggccagagtgctgcccaacggcagcgccggcgtgcccaaccgggaaggcctgagatactatcgccgcctgctggagaggctgagagagttgggcgtgcagcccgtggtgaccctgtaccactgggacctgccccagcgcctgcaggacgcctacggcggctgggccaacagggcactcgccgaccacttccgcgactacgccgagctgtgcttccgccacttcggcgggcaggtgaagtactggatcaccatcgacaacccctacgtggtggcctggcacggctacgctacaggaaggctggcccccgggatccgcggcagccccaggctgggctacctggtggcccacaacctgctgctggcacacgccaaagtgtggcacctgtataacaccagctttcgccccacccagggtggacaggtgagcattgccctgagttctcattggatcaaccccaggcgcatgaccgatcacagcatcaaggaatgccagaagagcctggacttcgtgctgggctggttcgccaagcccgtgtttatcgacggcgactaccccgagtctatgaagaacaacctcagcagcatcctgcctgacgtcaccgagagcgagaagaagttcatcaagggcaccgccgacttcttcgccctgagcttcggccccaccctgagcttccagctgctggatccccatatgaagttcagacaactcgagagtcctaacctgcgccagctgctgagctggatcgacctggaattcaaccacccacagatcttcatcgtggagaacggctggtttgtgagcggcaccactaagcgcgacgacgcaaagtatatgtattatctgaagaaattcatcatggaaaccctgaaggccatcaagctggacggcgtggacgtgatcggatacaccgcatggagcctgatggacggcttcgagtggcaccgcggttacagcatccgccggggcctgttctacgttgacttcctgagccaggacaagatgttgctgcccaagagctccgccctgttctaccagaagttgatcgagaagaacggcttcccaccactccccgagaaccagcccctggagggcaccttcccctgcgatttcgcctggggcgtggtggacaactacatccaggtggacaccaccctgagtcagttcactgacctgaacgtgtacctttgggacgtgcaccacagcaagcgcctgataaaggtcgacggcgtggtgaccaagaagcgcaaaagctactgcgtggactttgccgccatccagccccagatcgccctgctgcaggagatgcacgtgactcacttccgcttcagcctcgactgggccctgattctgcccctgggcaaccagtcacaagtgaaccacaccattctgcagtactaccgctgtatggccagcgagctggtacgcgtgaacatcacccccgttgtggccctttggcagcccatggcccccaaccagggcctgcctcgcctgctggcccgccagggagcctgggagaatccctacaccgcactggccttcgctgaatacgcccgcctgtgcttccaggagctggggcaccacgtgaaactctggatcaccatgaacgagccctacaccagaaacatgacctacagcgccggacacaatctgctgaaggcccacgctctggcctggcacgtgtacaacgagaagtttcgccacgcccagaacggcaagatcagcatcgccctgcaggccgattggatcgagcccgcctgccccttcagccagaaggacaaggaggtggctgagcgggtgctggagttcgacatcgggtggctggctgagcctatcttcggcagcggagactacccctgggtgatgcgcgattggcttaaccagaggaacaatttcctgctgccctacttcaccgaggacgagaagaagctgatccagggcacctttgacttcctggctttgagccactataccactatcctggtggacagcgagaaggaggaccccatcaagtacaacgactacttggaggtgcaggagatgaccgacatcacctggctgaacagccctagccaggtggctgtggtgccttggggcctgcgcaaggtgctgaactggctgaagttcaagtacggcgacctgcccatgtatatcatcagcaacggcatcgacgacggcctgcacgccgaggacgaccagctgagagtgtactacatgcagaactacatcaacgaggccctcaaggcccacatcctggacggcatcaacctgtgtggctactttgcctacagcttcaacgacagaaccgccccccgcttcggcctgtacaggtacgccgccgaccagttcgaacccaaggccagcatgaagcactaccgcaaaatcatcgacagcaacggattccctggacccgagacactggagcgcttctgcccagaggagttcaccgtgtgcaccgagtgcagtttcttccacacccgcaagagcctgctggctttcattgcttttctgttttttgcttccattatttctctctccctcatcttttactacagcaagaaaggaagaagaagctacaaatgagctggagcctcggtggccatgcttcttgccccttgggcctccccccagcccctcctccccttcctgcacccgtacccccgtggtctttgaataaagtctgagtgggcggcaaaaaaaaaaaaaaaaaaaaaaaaaaaaaaaaaaaaaaaaaaaaaaaaaaaaaaaaaaaaaaaaaaaaaaaaaaaaaaaaaaaaaaaaaaaaaaaaaaaaaaaaaaaaaaaaaaaaaaaaa

SEQ ID NO: 75 - RNA, 3342 nt, synthetic construct
  source 1..3342: mol_type = other RNA
gggagacataaaccctggcgcgctcgcggcccggcactcttctggtccccacagactcagagagaacccaccatgcccgctagcgccccaccgagaagaccgcggccgccaccgccatcgctgtcgctgctgctggtgctgctgggactgggcggaagaagactgcgtgcggagcctggagatggagcccaaacatgggccagattcagcagacctcccgctcctgaagccgccggcttgtttcagggaacctttcctgacggtttcctgtgggctgtgggcagcgccgcctatcagaccgagggcggctggcaacagcacggaaaaggagccagcatctgggataccttcacccaccaccccctggccccccccggcgattcccgcaatgccagcctccctctgggagcccctagccccctgcaacctgccacaggagacgtggcctcagacagctataacaacgtgttccgcgacaccgaggcactgcgcgagctgggcgtgacccattaccgctttagcatcagctgggccagagtgctgcccaatggctctgccggcgtgcccaaccgggagggcctgaggtactaccgccgcctgctggagaggctgcgggagctgggcgtgcagcccgtggtaaccctgtaccactgggacctgccccagcgcctgcaggacgcttacggcggctgggccaaccgcgctctcgcagaccacttccgcgactacgccgagctgtgctttcgccactttggcggccaggtgaagtattggatcaccatcgataacccttacgtggtggcctggcacggatacgctacaggccgcctggcccccggcatccgcggcagccccagactgggctacctggtggcccacaacctgctgctggcccacgccaaggtgtggcacctgtacaacaccagcttccgccccacccagggtggacaggtctctattgccctgagctctcactggattaaccccaggaggatgaccgatcacagcatcaaggaatgccagaagagcctggacttcgttctgggctggttcgccaagcccgtgtttatcgacggcgactaccccgagagcatgaagaacaacctgtctagcatcctgcccgacgtcaccgagagcgaaaaaaaattcatcaagggcaccgccgatttcttcgccctgagcttcggcccaaccctgagcttccaactgctggatccccacatgaagttcagacaactcgagagtcccaacctgcgccagctgctgagctggatcgatctggaattcaaccacccccagatattcatagtggagaacggctggtttgtaagcggcactactaagcgcgatgatgcaaagtacatgtactatctgaagaagttcatcatggaaaccctgaaggccatcaagctggatggcgtggacgtgatcggatacaccgcatggagcctgatggacggcttcgagtggcaccgcggttactcaatccgcagggggttgttctacgtcgacttcctgagtcaggacaagatgttgctgccaaagagtagcgcccttttctaccagaagttgattgagaagaacggcttcccaccactccccgagaaccagcccctggagggcacctttccctgcgatttcgcttggggcgtggtggataattatattcaggtggacaccaccctgtcacagttcactgacctgaacgtgtacctgtgggacgtgcaccattccaagcgcctgatcaaggtggacggcgtggtgaccaagaagcgcaaatcctactgcgttgactttgccgccattcagccacagatcgccctgctgcaggagatgcacgtcacccacttccgcttcagcctggactgggccctcatcctgccactgggcaaccagtcccaggtgaaccacaccattctgcagtactaccgctgtatggccagcgagctggtacgcgtgaacatcacccccgtggtggccctgtggcagcccatggcccccaaccagggcctgccacgcctgctggccaggcagggggcctgggagaacccctacaccgcactcgctttcgccgaatatgccaggctgtgcttccaggagctggggcaccacgtgaagctctggatcaccatgaacgaaccctacaccagaaacatgacctactctgccggacacaatctgctgaaggcccacgccctggcctggcacgtctacaacgagaagttccgccacgcccaaaatggaaagatctctatagccctgcaggccgattggatcgagcccgcctgccccttctcacagaaggacaaggaggtggccgagcgcgtgctggagttcgacatcggctggctggccgagcccatcttcggcagcggagactacccctgggtgatgcgcgattggcttaaccagcgcaacaactttctgctgccctacttcaccgaggacgagaagaagctgatccagggcaccttcgacttcctggccctgagccactatactaccatcctggtcgacagcgagaaggaggacccaatcaagtacaacgactacctggaggtgcaggagatgaccgacatcacctggctgaacagccctagccaggtcgccgtggtgccttggggcctgcgcaaggtgctgaactggctgaagttcaagtatggcgacctgccaatgtacatcatcagcaacggcattgatgacggcctgcacgccgaggacgatcagctgagagtgtactatatgcagaactacatcaacgaggcactgaaggcccacatcctggacggcatcaacctgtgtggctactttgcatactccttcaacgacagaaccgccccccgcttcggcctgtacaggtacgctgccgatcagttcgagcccaaggccagcatgaagcactacagaaaaatcattgatagcaacgggttcccaggccccgagaccctggagcgcttctgccccgaggagttcaccgtgtgcaccgagtgcagttttttccacacccgcaagagcctgctggctttcattgcttttctgttttttgcttccattatttctctctccctcatcttttactacagcaagaaaggaagaagaagctacaaatgagctggagcctcggtggccatgcttcttgccccttgggcctccccccagcccctcctccccttcctgcacccgtacccccgtggtctttgaataaagtctgagtgggcggcaaaaaaaaaaaaaaaaaaaaaaaaaaaaaaaaaaaaaaaaaaaaaaaaaaaaaaaaaaaaaaaaaaaaaaaaaaaaaaaaaaaaaaaaaaaaaaaaaaaaaaaaaaaaaaaaaaaaaaaaa

SEQ ID NO: 76 - protein, 1012 aa, synthetic construct
MPASAPPRRPRPPPPSLSLLLVLLGLGGRRLRAEPGDGAQTWARFSRPPAPEAAGLFQGTFPDGFLWAVGSAAYQTEGGWQQHGKGASIWDTFTHHPLAPPGDSRNASLPLGAPSPLQPATGDVASDSYNNVFRDTEALRELGVTHYRFSISWARVLPNGSAGVPNREGLRYYRRLLERLRELGVQPVVTLYHWDLPQRLQDAYGGWANRALADHFRDYAELCFRHFGGQVKYWITIDNPYVVAWHGYATGRLAPGIRGSPRLGYLVAHNLLLAHAKVWHLYNTSFRPTQGGQVSIALSSHWINPRRMTDHSIKECQKSLDFVLGWFAKPVFIDGDYPESMKNNLSSILPDVTESEKKFIKGTADFFALSFGPTLSFQLLDPHMKFRQLESPNLRQLLSWIDLEFNHPQIFIVENGWFVSGTTKRDDAKYMYYLKKFIMETLKAIKLDGVDVIGYTAWSLMDGFEWHRGYSIRRGLFYVDFLSQDKMLLPKSSALFYQKLIEKNGFPPLPENQPLEGTFPCDFAWGVVDNYIQVDTTLSQFTDLNVYLWDVHHSKRLIKVDGVVTKKRKSYCVDFAAIQPQIALLQEMHVTHFRFSLDWALILPLGNQSQVNHTILQYYRCMASELVRVNITPVVALWQPMAPNQGLPRLLARQGAWENPYTALAFAEYARLCFQELGHHVKLWITMNEPYTRNMTYSAGHNLLKAHALAWHVYNEKFRHAQNGKISIALQADWIEPACPFSQKDKEVAERVLEFDIGWLAEPIFGSGDYPWVMRDWLNQRNNFLLPYFTEDEKKLIQGTFDFLALSHYTTILVDSEKEDPIKYNDYLEVQEMTDITWLNSPSQVAVVPWGLRKVLNWLKFKYGDLPMYIISNGIDDGLHAEDDQLRVYYMQNYINEALKAHILDGINLCGYFAYSFNDRTAPRFGLYRYAADQFEPKASMKHYRKIIDSNGFPGPETLERFCPEEFTVCTECSFFHTRKSLLAFIAFLFFASIISLSLIFYYSKKGRRSYK

SEQ ID NO: 77 - DNA, 28 bp, synthetic construct
  source 1..28: mol_type = other DNA
tgctgccgtaatacgactcactataagg

SEQ ID NO: 78 - DNA, 143 bp, synthetic construct
  source 1..143: mol_type = other DNA
tttttttttttttttttttttttttttttttttttttttttttttttttttttttttttttttttttttttttttttttttttttttttttttttttttttttttttttttttttttttttgccgcccactcagactttattc